European Patent Application EP 4 653 010 A1, published November 26, 2025. Title: ACTIVIN RECEPTOR TYPE IIB VARIANTS AND USES THEREOF. Applicant: 35Pharma Inc. Application US. The sequence listing filed with the application follows.

SEQUENCE LISTING (377 sequences)

SEQ ID NO: 1 - protein, 19 aa, Homo sapiens
MDWTWRILFLVAAATGTHA

SEQ ID NO: 2 - protein, 107 aa, Homo sapiens
ETRECIYYNANWELERTNQSGLERCEGEQDKRLHCYASWRNSSGTIELVKKGCWLDDFNCYDRQECVATEENPQVYFCCCEGNFCNERFTHLPEAGGPEVTYEPPPT

SEQ ID NO: 3 - protein, 116 aa, Homo sapiens
ILGRSETQECLFFNANWEKDRTNQTGVEPCYGDKDKRRHCFATWKNISGSIEIVKQGCWLDDINCYDRTDCVEKKDSPEVYFCCCEGNMCNEKFSYFPEMEVTQPTSNPVTPKPPT

SEQ ID NO: 4 - protein, 107 aa, synthetic construct
ETRECIYYNANWELERTNQSGLERCEEEQDKRLHCYASWRNSSGTIELVKKGCWLDDFNCYDRQECVATEENPQVYFCCCEGNFCNERFTHLPEAGGPEVTYEPPPT

SEQ ID NO: 5 - protein, 107 aa, synthetic construct
ETRECIYYNANWELERTNQSGLERCENEQDKRLHCYASWRNSSGTIELVKKGCWLDDFNCYDRQECVATEENPQVYFCCCEGNFCNERFTHLPEAGGPEVTYEPPPT

SEQ ID NO: 6 - protein, 107 aa, synthetic construct
ETRECIYYNANWELERTNQSGLERCEQEQDKRLHCYASWRNSSGTIELVKKGCWLDDFNCYDRQECVATEENPQVYFCCCEGNFCNERFTHLPEAGGPEVTYEPPPT

SEQ ID NO: 7 - protein, 107 aa, synthetic construct
ETRECIYYNANWELERTNQSGLERCEKEQDKRLHCYASWRNSSGTIELVKKGCWLDDFNCYDRQECVATEENPQVYFCCCEGNFCNERFTHLPEAGGPEVTYEPPPT

SEQ ID NO: 8 - protein, 107 aa, synthetic construct
ETRECIYYNANWELERTNQSGLERCETEQDKRLHCYASWRNSSGTIELVKKGCWLDDFNCYDRQECVATEENPQVYFCCCEGNFCNERFTHLPEAGGPEVTYEPPPT

SEQ ID NO: 9 - protein, 107 aa, synthetic construct
ETRECIYYNANWELERTNQSGLERCEMEQDKRLHCYASWRNSSGTIELVKKGCWLDDFNCYDRQECVATEENPQVYFCCCEGNFCNERFTHLPEAGGPEVTYEPPPT

SEQ ID NO: 10 - protein, 107 aa, synthetic construct
ETRECIYYNANWELERTNQSGLERCEGEQDKRFHCYASWRNSSGTIELVKKGCWLDDFNCYDRQECVATEENPQVYFCCCEGNFCNERFTHLPEAGGPEVTYEPPPT

SEQ ID NO: 11 - protein, 107 aa, synthetic construct
ETRECIYYNANWELERTNQSGLERCEGEQDKRQHCYASWRNSSGTIELVKKGCWLDDFNCYDRQECVATEENPQVYFCCCEGNFCNERFTHLPEAGGPEVTYEPPPT

SEQ ID NO: 12 - protein, 107 aa, synthetic construct
ETRECIYYNANWELERTNQSGLERCEGEQDKRYHCYASWRNSSGTIELVKKGCWLDDFNCYDRQECVATEENPQVYFCCCEGNFCNERFTHLPEAGGPEVTYEPPPT

SEQ ID NO: 13 - protein, 107 aa, synthetic construct
ETRECIYYNANWELERTNQSGLERCEGEQDKRWHCYASWRNSSGTIELVKKGCWLDDFNCYDRQECVATEENPQVYFCCCEGNFCNERFTHLPEAGGPEVTYEPPPT

SEQ ID NO: 14 - protein, 107 aa, synthetic construct
ETRECIYYNANWELERTNQSGLERCEGEQDKRHHCYASWRNSSGTIELVKKGCWLDDFNCYDRQECVATEENPQVYFCCCEGNFCNERFTHLPEAGGPEVTYEPPPT

SEQ ID NO: 15 - protein, 107 aa, synthetic construct
ETRECIYYNANWELERTNQSGLERCEGEQDKRRHCYASWRNSSGTIELVKKGCWLDDFNCYDRQECVATEENPQVYFCCCEGNFCNERFTHLPEAGGPEVTYEPPPT

SEQ ID NO: 16 - protein, 107 aa, synthetic construct
ETRECIYYNANWELERTNQSGLERCEGEQDKREHCYASWRNSSGTIELVKKGCWLDDFNCYDRQECVATEENPQVYFCCCEGNFCNERFTHLPEAGGPEVTYEPPPT

SEQ ID NO: 17 - protein, 107 aa, synthetic construct
ETRECIYYNANWELERTNQSGLERCEGEQDKRKHCYASWRNSSGTIELVKKGCWLDDFNCYDRQECVATEENPQVYFCCCEGNFCNERFTHLPEAGGPEVTYEPPPT

SEQ ID NO: 18 - protein, 107 aa, synthetic construct
ETRECIYYNANWELERTNQSGLERCEGEQDKRMHCYASWRNSSGTIELVKKGCWLDDFNCYDRQECVATEENPQVYFCCCEGNFCNERFTHLPEAGGPEVTYEPPPT

SEQ ID NO: 19 - protein, 107 aa, synthetic construct
ETRECIYYNANWELERTNQSGLERCEGEQDKRLHCYASWRNSSGTIELVKKGCWLDDFNCYDRQECVAHEENPQVYFCCCEGNFCNERFTHLPEAGGPEVTYEPPPT

SEQ ID NO: 20 - protein, 107 aa, synthetic construct
ETRECIYYNANWELERTNQSGLERCEGEQDKRLHCYASWRNSSGTIELVKKGCWLDDFNCYDRQECVAQEENPQVYFCCCEGNFCNERFTHLPEAGGPEVTYEPPPT

SEQ ID NO: 21 - protein, 107 aa, synthetic construct
ETRECIYYNANWELERTNQSGLERCEGEQDKRLHCYASWRNSSGTIELVKKGCWLDDFNCYDRQECVAEEENPQVYFCCCEGNFCNERFTHLPEAGGPEVTYEPPPT

SEQ ID NO: 22 - protein, 107 aa, synthetic construct
ETRECIYYNANWELERTNQSGLERCEGEQDKRLHCYASWRNSSGTIELVKKGCWLDDFNCYDRQECVAREENPQVYFCCCEGNFCNERFTHLPEAGGPEVTYEPPPT

SEQ ID NO: 23 - protein, 107 aa, synthetic construct
ETRECIYYNANWELERTNQSGLERCEGEQDKRLHCYASWRNSSGTIELVKKGCWLDDFNCYDRQECVAYEENPQVYFCCCEGNFCNERFTHLPEAGGPEVTYEPPPT

SEQ ID NO: 24 - protein, 107 aa, synthetic construct
ETRECIYYNANWELERTNQSGLERCEGEQDKRLHCYASWRNSSGTIELVKKGCWLDDFNCYDRQECVAWEENPQVYFCCCEGNFCNERFTHLPEAGGPEVTYEPPPT

SEQ ID NO: 25 - protein, 107 aa, synthetic construct
ETRECIYYNANWELERTNQSGLERCEGEQDKRYHCYASWRNSSGTIELVKKGCWLDDFNCYDRQECVAREENPQVYFCCCEGNFCNERFTHLPEAGGPEVTYEPPPT

SEQ ID NO: 26 - protein, 107 aa, synthetic construct
ETRECIYYNANWELERTNQSGLERCEGEQDKRYHCYASWRNSSGTIELVKKGCWLDDFNCYDRQECVAYEENPQVYFCCCEGNFCNERFTHLPEAGGPEVTYEPPPT

SEQ ID NO: 27 - protein, 107 aa, synthetic construct
ETRECIYYNANWELERTNQSGLERCEGEQDKRYHCYASWRNSSGTIELVKKGCWLDDFNCYDRQECVAWEENPQVYFCCCEGNFCNERFTHLPEAGGPEVTYEPPPT

SEQ ID NO: 28 - protein, 107 aa, synthetic construct
ETRECIYYNANWELERTNQSGLERCEGEQDKRYHCYASWRNSSGTIELVKKGCWLDDFNCYDRQECVAHEENPQVYFCCCEGNFCNERFTHLPEAGGPEVTYEPPPT

SEQ ID NO: 29 - protein, 107 aa, synthetic construct
ETRECIYYNANWELERTNQSGLERCEGEQDKRYHCYASWRNSSGTIELVKKGCWLDDFNCYDRQECVAQEENPQVYFCCCEGNFCNERFTHLPEAGGPEVTYEPPPT

SEQ ID NO: 30 - protein, 107 aa, synthetic construct
ETRECIYYNANWELERTNQSGLERCEGEQDKRYHCYASWRNSSGTIELVKKGCWLDDFNCYDRQECVAEEENPQVYFCCCEGNFCNERFTHLPEAGGPEVTYEPPPT

SEQ ID NO: 31 - protein, 107 aa, synthetic construct
ETRECIYYNANWELERTNQSGLERCEGEQDKRFHCYASWRNSSGTIELVKKGCWLDDFNCYDRQECVAQEENPQVYFCCCEGNFCNERFTHLPEAGGPEVTYEPPPT

SEQ ID NO: 32 - protein, 107 aa, synthetic construct
ETRECIYYNANWELERTNQSGLERCEEEQDKRYHCYASWRNSSGTIELVKKGCWLDDFNCYDRQECVATEENPQVYFCCCEGNFCNERFTHLPEAGGPEVTYEPPPT

SEQ ID NO: 33 - protein, 107 aa, synthetic construct
ETRECIYYNANWELERTNQSGLERCEDEQDKRYHCYASWRNSSGTIELVKKGCWLDDFNCYDRQECVATEENPQVYFCCCEGNFCNERFTHLPEAGGPEVTYEPPPT

SEQ ID NO: 34 - protein, 107 aa, synthetic construct
ETRECIYYNANWELERTNQSGLERCENEQDKRYHCYASWRNSSGTIELVKKGCWLDDFNCYDRQECVATEENPQVYFCCCEGNFCNERFTHLPEAGGPEVTYEPPPT

SEQ ID NO: 35 - protein, 107 aa, synthetic construct
ETRECIYYNANWELERTNQSGLERCEQEQDKRYHCYASWRNSSGTIELVKKGCWLDDFNCYDRQECVATEENPQVYFCCCEGNFCNERFTHLPEAGGPEVTYEPPPT

SEQ ID NO: 36 - protein, 107 aa, synthetic construct
ETRECIYYNANWELERTNQSGLERCEKEQDKRYHCYASWRNSSGTIELVKKGCWLDDFNCYDRQECVATEENPQVYFCCCEGNFCNERFTHLPEAGGPEVTYEPPPT

SEQ ID NO: 37 - protein, 107 aa, synthetic construct
ETRECIYYNANWELERTNQSGLERCETEQDKRYHCYASWRNSSGTIELVKKGCWLDDFNCYDRQECVATEENPQVYFCCCEGNFCNERFTHLPEAGGPEVTYEPPPT

SEQ ID NO: 38 - protein, 107 aa, synthetic construct
ETRECIYYNANWELERTNQSGLERCEMEQDKRYHCYASWRNSSGTIELVKKGCWLDDFNCYDRQECVATEENPQVYFCCCEGNFCNERFTHLPEAGGPEVTYEPPPT

SEQ ID NO: 39 - protein, 107 aa, synthetic construct; identical to SEQ ID NO: 33

SEQ ID NO: 40 - protein, 107 aa, synthetic construct; identical to SEQ ID NO: 32

SEQ ID NO: 41 - protein, 107 aa, synthetic construct; identical to SEQ ID NO: 34

SEQ ID NO: 42 - protein, 107 aa, synthetic construct; identical to SEQ ID NO: 35

SEQ ID NO: 43 - protein, 107 aa, synthetic construct
ETRECIYYNANWELERTNQSGLERCEDEQDKRWHCYASWRNSSGTIELVKKGCWLDDFNCYDRQECVATEENPQVYFCCCEGNFCNERFTHLPEAGGPEVTYEPPPT

SEQ ID NO: 44 - protein, 107 aa, synthetic construct
ETRECIYYNANWELERTNQSGLERCEEEQDKRWHCYASWRNSSGTIELVKKGCWLDDFNCYDRQECVATEENPQVYFCCCEGNFCNERFTHLPEAGGPEVTYEPPPT

SEQ ID NO: 45 - protein, 107 aa, synthetic construct
ETRECIYYNANWELERTNQSGLERCENEQDKRWHCYASWRNSSGTIELVKKGCWLDDFNCYDRQECVATEENPQVYFCCCEGNFCNERFTHLPEAGGPEVTYEPPPT

SEQ ID NO: 46 - protein, 126 aa, synthetic construct
ETRECIYYNANWELERTNQSGLERCEQEQDKRWHCYASWRNSSGTIELVKKGCWLDDFNCYDRQECVATEENPQVYFCCCEGNFCNERFTHLPEAGGPEVTYEPPPTGGGGSGGGGSGGGGSGGGG

SEQ ID NO: 47 - protein, 107 aa, synthetic construct
ETRECIYYNANWELERTNQSGLERCETEQDKRWHCYASWRNSSGTIELVKKGCWLDDFNCYDRQECVATEENPQVYFCCCEGNFCNERFTHLPEAGGPEVTYEPPPT

SEQ ID NO: 48 - protein, 107 aa, synthetic construct
ETRECIYYNANWELERTNQSGLERCEMEQDKRWHCYASWRNSSGTIELVKKGCWLDDFNCYDRQECVATEENPQVYFCCCEGNFCNERFTHLPEAGGPEVTYEPPPT

SEQ ID NO: 49 - protein, 107 aa, synthetic construct
ETRECIYYNANWEQERTNQSGLERCEGEQDKRYHCYASWRNSSGTIELVKKGCWLDDFNCYDRQECVATEENPQVYFCCCEGNFCNERFTHLPEAGGPEVTYEPPPT

SEQ ID NO: 50 - protein, 107 aa, synthetic construct
ETRECIYYNANWEDERTNQSGLERCEGEQDKRYHCYASWRNSSGTIELVKKGCWLDDFNCYDRQECVATEENPQVYFCCCEGNFCNERFTHLPEAGGPEVTYEPPPT

SEQ ID NO: 51 - protein, 107 aa, synthetic construct
ETRECIYYNANWENERTNQSGLERCEGEQDKRYHCYASWRNSSGTIELVKKGCWLDDFNCYDRQECVATEENPQVYFCCCEGNFCNERFTHLPEAGGPEVTYEPPPT

SEQ ID NO: 52 - protein, 107 aa, synthetic construct
ETRECIYYNANWEEERTNQSGLERCEGEQDKRYHCYASWRNSSGTIELVKKGCWLDDFNCYDRQECVATEENPQVYFCCCEGNFCNERFTHLPEAGGPEVTYEPPPT

SEQ ID NO: 53 - protein, 107 aa, synthetic construct
ETRECIYYNANWEHERTNQSGLERCEGEQDKRYHCYASWRNSSGTIELVKKGCWLDDFNCYDRQECVATEENPQVYFCCCEGNFCNERFTHLPEAGGPEVTYEPPPT

SEQ ID NO: 54 - protein, 107 aa, synthetic construct
ETRECIYYNANWESERTNQSGLERCEGEQDKRYHCYASWRNSSGTIELVKKGCWLDDFNCYDRQECVATEENPQVYFCCCEGNFCNERFTHLPEAGGPEVTYEPPPT

SEQ ID NO: 55 - protein, 107 aa, synthetic construct
ETRECIYYNANWEEERTNQSGLERCEGEQDKRWHCYASWRNSSGTIELVKKGCWLDDFNCYDRQECVATEENPQVYFCCCEGNFCNERFTHLPEAGGPEVTYEPPPT

SEQ ID NO: 56 - protein, 107 aa, synthetic construct
ETRECIYYNANWEDERTNQSGLERCEGEQDKRWHCYASWRNSSGTIELVKKGCWLDDFNCYDRQECVATEENPQVYFCCCEGNFCNERFTHLPEAGGPEVTYEPPPT

SEQ ID NO: 57 - protein, 107 aa, synthetic construct
ETRECIYYNANWENERTNQSGLERCEGEQDKRWHCYASWRNSSGTIELVKKGCWLDDFNCYDRQECVATEENPQVYFCCCEGNFCNERFTHLPEAGGPEVTYEPPPT

SEQ ID NO: 58 - protein, 107 aa, synthetic construct
ETRECIYYNANWEQERTNQSGLERCEGEQDKRWHCYASWRNSSGTIELVKKGCWLDDFNCYDRQECVATEENPQVYFCCCEGNFCNERFTHLPEAGGPEVTYEPPPT

SEQ ID NO: 59 - protein, 107 aa, synthetic construct
ETRECIYYNANWELERTNQSGLERCEGEQDKRYHCYASWRNSSGTIELVKKGCWYDDFNCYDRQECVATEENPQVYFCCCEGNFCNERFTHLPEAGGPEVTYEPPPT

SEQ ID NO: 60 - protein, 107 aa, synthetic construct
ETRECIYYNANWELERTNQSGLERCEGEQDKRYHCYASWRNSSGTIELVKKGCWQDDFNCYDRQECVATEENPQVYFCCCEGNFCNERFTHLPEAGGPEVTYEPPPT

SEQ ID NO: 61 - protein, 107 aa, synthetic construct
ETRECIYYNANWELERTNQSGLERCEGEQDKRYHCYASWRNSSGTIELVKKGCWMDDFNCYDRQECVATEENPQVYFCCCEGNFCNERFTHLPEAGGPEVTYEPPPT

SEQ ID NO: 62 - protein, 107 aa, synthetic construct
ETRECIYYNANWELERTNQSGLERCEGEQDKRYHCYASWRNSSGTIELVKKGCWIDDFNCYDRQECVATEENPQVYFCCCEGNFCNERFTHLPEAGGPEVTYEPPPT

SEQ ID NO: 63 - protein, 5 aa, synthetic construct
GRGEA

SEQ ID NO: 64 - skipped

SEQ ID NO: 65 - protein, 115 aa, synthetic construct
GRGEAETRECIYYNANWELERTNQSGLERCEGEQDKRLHCYASWRNSSGTIELVKKGCWLDDFNCYDRQECVATEENPQVYFCCCEGNFCNERFTHLPEAGGPEVTYEPPPTAPT

SEQ ID NO: 66 - protein, 112 aa, synthetic construct
GRGEAETRECIYYNANWELERTNQSGLERCEGEQDKRLHCYASWRNSSGTIELVKKGCWLDDFNCYDRQECVATEENPQVYFCCCEGNFCNERFTHLPEAGGPEVTYEPPPT

SEQ ID NO: 67 - protein, 110 aa, synthetic construct
ETRECIYYNANWELERTNQSGLERCEGEQDKRLHCYASWRNSSGTIELVKKGCWLDDFNCYDRQECVATEENPQVYFCCCEGNFCNERFTHLPEAGGPEVTYEPPPTAPT

SEQ ID NO: 68 - protein, 40 aa, synthetic construct
GGGGSGGGGSGGGGSGGGGSGGGGSGGGGSGGGGSGGGGS

SEQ ID NO: 69 - protein, 39 aa, synthetic construct
GGGGSGGGGSGGGGSGGGGSGGGGSGGGGSGGGGSGGGG

SEQ ID NO: 70 - protein, 38 aa, synthetic construct
GGGGSGGGGSGGGGSGGGGSGGGGSGGGGSGGGGSGGG

SEQ ID NO: 71 - protein, 37 aa, synthetic construct
GGGGSGGGGSGGGGSGGGGSGGGGSGGGGSGGGGSGG

SEQ ID NO: 72 - protein, 36 aa, synthetic construct
GGGGSGGGGSGGGGSGGGGSGGGGSGGGGSGGGGSG

SEQ ID NO: 73 - protein, 35 aa, synthetic construct
GGGGSGGGGSGGGGSGGGGSGGGGSGGGGSGGGGS

SEQ ID NO: 74 - protein, 34 aa, synthetic construct
GGGGSGGGGSGGGGSGGGGSGGGGSGGGGSGGGG

SEQ ID NO: 75 - protein, 33 aa, synthetic construct
GGGGSGGGGSGGGGSGGGGSGGGGSGGGGSGGG

SEQ ID NO: 76 - protein, 32 aa, synthetic construct
GGGGSGGGGSGGGGSGGGGSGGGGSGGGGSGG

SEQ ID NO: 77 - protein, 31 aa, synthetic construct
GGGGSGGGGSGGGGSGGGGSGGGGSGGGGSG

SEQ ID NO: 78 - protein, 30 aa, synthetic construct
GGGGSGGGGSGGGGSGGGGSGGGGSGGGGS

SEQ ID NO: 79 - protein, 29 aa, synthetic construct
GGGGSGGGGSGGGGSGGGGSGGGGSGGGG

SEQ ID NO: 80 - protein, 28 aa, synthetic construct
GGGGSGGGGSGGGGSGGGGSGGGGSGGG

SEQ ID NO: 81 - protein, 27 aa, synthetic construct
GGGGSGGGGSGGGGSGGGGSGGGGSGG

SEQ ID NO: 82 - protein, 26 aa, synthetic construct
GGGGSGGGGSGGGGSGGGGSGGGGSG

SEQ ID NO: 83 - protein, 25 aa, synthetic construct
GGGGSGGGGSGGGGSGGGGSGGGGS

SEQ ID NO: 84 - protein, 24 aa, synthetic construct
GGGGSGGGGSGGGGSGGGGSGGGG

SEQ ID NO: 85 - protein, 23 aa, synthetic construct
GGGGSGGGGSGGGGSGGGGSGGG

SEQ ID NO: 86 - protein, 22 aa, synthetic construct
GGGGSGGGGSGGGGSGGGGSGG

SEQ ID NO: 87 - protein, 21 aa, synthetic construct
GGGGSGGGGSGGGGSGGGGSG

SEQ ID NO: 88 - protein, 20 aa, synthetic construct
GGGGSGGGGSGGGGSGGGGS

SEQ ID NO: 89 - protein, 19 aa, synthetic construct
GGGGSGGGGSGGGGSGGGG

SEQ ID NO: 90 - protein, 18 aa, synthetic construct
GGGGSGGGGSGGGGSGGG

SEQ ID NO: 91 - protein, 17 aa, synthetic construct
GGGGSGGGGSGGGGSGG

SEQ ID NO: 92 - protein, 16 aa, synthetic construct
GGGGSGGGGSGGGGSG

SEQ ID NO: 93 - protein, 15 aa, synthetic construct
GGGGSGGGGSGGGGS

SEQ ID NO: 94 - protein, 14 aa, synthetic construct
GGGGSGGGGSGGGG

SEQ ID NO: 95 - protein, 13 aa, synthetic construct
GGGGSGGGGSGGG

SEQ ID NO: 96 - protein, 12 aa, synthetic construct
GGGGSGGGGSGG

SEQ ID NO: 97 - protein, 11 aa, synthetic construct
GGGGSGGGGSG

SEQ ID NO: 98 - protein, 10 aa, synthetic construct
GGGGSGGGGS

SEQ ID NO: 99 - protein, 9 aa, synthetic construct
GGGGSGGGG

SEQ ID NO: 100 - protein, 8 aa, synthetic construct
GGGGSGGG

SEQ ID NO: 101 - protein, 7 aa, synthetic construct
GGGGSGG

SEQ ID NO: 102 - protein, 6 aa, synthetic construct
GGGGSG

SEQ ID NO: 103 - protein, 5 aa, synthetic construct
GGGGS

SEQ ID NO: 104 - protein, 4 aa, synthetic construct
GGGG

SEQ ID NO: 105-106 - skipped (2 entries)

SEQ ID NO: 107 - protein, 4 aa, synthetic construct
TGGG

SEQ ID NO: 108 - protein, 5 aa, synthetic construct
TGGGG

SEQ ID NO: 109 - protein, 5 aa, synthetic construct
SGGGG

SEQ ID NO: 110 - protein, 4 aa, synthetic construct
SGGG

SEQ ID NO: 111 - protein, 11 aa, synthetic construct
TGGGGSGGGGS

SEQ ID NO: 112 - protein, 16 aa, synthetic construct
TGGGGSGGGGSGGGGS

SEQ ID NO: 113 - protein, 21 aa, synthetic construct
TGGGGSGGGGSGGGGSGGGGS

SEQ ID NO: 114 - protein, 26 aa, synthetic construct
TGGGGSGGGGSGGGGSGGGGSGGGGS

SEQ ID NO: 115 - protein, 31 aa, synthetic construct
TGGGGSGGGGSGGGGSGGGGSGGGGSGGGGS

SEQ ID NO: 116 - protein, 36 aa, synthetic construct
TGGGGSGGGGSGGGGSGGGGSGGGGSGGGGSGGGGS

SEQ ID NO: 117 - protein, 10 aa, synthetic construct
TGGGPKSCDK

SEQ ID NO: 118-119 - skipped (2 entries)

SEQ ID NO: 120 - protein, 4 aa, synthetic construct
AGGG

SEQ ID NO: 121 - protein, 4 aa, synthetic construct
GGSG

SEQ ID NO: 122 - protein, 4 aa, synthetic construct
GGAG

SEQ ID NO: 123 - protein, 5 aa, synthetic construct
GGGGG

SEQ ID NO: 124 - protein, 5 aa, synthetic construct
GGGGA

SEQ ID NO: 125 - protein, 4 aa, synthetic construct
GGGS

SEQ ID NO: 126 - protein, 4 aa, synthetic construct
GGGA

SEQ ID NO: 127-128 - skipped (2 entries)

SEQ ID NO: 129 - protein, 4 aa, synthetic construct
GSGS

SEQ ID NO: 130 - protein, 6 aa, synthetic construct
GAGAGA

SEQ ID NO: 131 - protein, 6 aa, synthetic construct
GSGSGS

SEQ ID NO: 132 - protein, 8 aa, synthetic construct
GAGAGAGA

SEQ ID NO: 133 - protein, 8 aa, synthetic construct
GSGSGSGS

SEQ ID NO: 134 - protein, 10 aa, synthetic construct
GAGAGAGAGA

SEQ ID NO: 135 - protein, 10 aa, synthetic construct
GSGSGSGSGS

SEQ ID NO: 136 - protein, 12 aa, synthetic construct
GAGAGAGAGAGA

SEQ ID NO: 137 - protein, 4 aa, synthetic construct
GAGA

SEQ ID NO: 138 - protein, 12 aa, synthetic construct
GSGSGSGSGSGS

SEQ ID NO: 139 - protein, 6 aa, synthetic construct
GGAGGA

SEQ ID NO: 140 - protein, 6 aa, synthetic construct
GGSGGS

SEQ ID NO: 141 - protein, 9 aa, synthetic construct
GGAGGAGGA

SEQ ID NO: 142 - protein, 9 aa, synthetic construct
GGSGGSGGS

SEQ ID NO: 143 - protein, 12 aa, synthetic construct
GGAGGAGGAGGA

SEQ ID NO: 144 - protein, 12 aa, synthetic construct
GGSGGSGGSGGS

SEQ ID NO: 145 - protein, 4 aa, synthetic construct
GGAG

SEQ ID NO: 146 - protein, 4 aa, synthetic construct
GGSG

SEQ ID NO: 147 - protein, 8 aa, synthetic construct
GGAGGGAG

SEQ ID NO: 148 - protein, 8 aa, synthetic construct
GGSGGGSG

SEQ ID NO: 149 - protein, 12 aa, synthetic construct
GGAGGGAGGGAG

SEQ ID NO: 150 - protein, 12 aa, synthetic construct
GGSGGGSGGGSG

SEQ ID NO: 151 - protein, 15 aa, synthetic construct
GGGGAGGGGAGGGGA

SEQ ID NO: 152 - protein, 4 aa, synthetic construct
AAAL

SEQ ID NO: 153 - protein, 4 aa, synthetic construct
AAAK

SEQ ID NO: 154 - protein, 4 aa, synthetic construct
AAAR

SEQ ID NO: 155 - protein, 14 aa, synthetic construct
EGKSSGSGSESKST

SEQ ID NO: 156 - protein, 12 aa, synthetic construct
GSAGSAAGSGEF

SEQ ID NO: 157 - protein, 12 aa, synthetic construct
AEAAAKEAAAKA

SEQ ID NO: 158 - protein, 18 aa, synthetic construct
KESGSVSSEQLAQFRSLD

SEQ ID NO: 159 - protein, 10 aa, synthetic construct
GENLYFQSGG

SEQ ID NO: 160 - protein, 8 aa, synthetic construct
SACYCELS

SEQ ID NO: 161 - protein, 5 aa, synthetic construct
RSIAT

SEQ ID NO: 162 - protein, 17 aa, synthetic construct
RPACKIPNDLKQKVMNH

SEQ ID NO: 163 - protein, 36 aa, synthetic construct
GGSAGGSGSGSSGGSSGASGTGTAGGTGSGSGTGSG

SEQ ID NO: 164 - protein, 17 aa, synthetic construct
AAANSSIDLISVPVDSR

SEQ ID NO: 165 - protein, 36 aa, synthetic construct
GGSGGGSEGGGSEGGGSEGGGSEGGGSEGGGSGGGS

SEQ ID NO: 166 - protein, 5 aa, synthetic construct
EAAAK

SEQ ID NO: 167 - protein, 5 aa, synthetic construct
PAPAP

SEQ ID NO: 168 - protein, 5 aa, synthetic construct
GGGAG

SEQ ID NO: 169 - protein, 6 aa, synthetic construct
GGGAGG

SEQ ID NO: 170 - protein, 7 aa, synthetic construct
GGGAGGG

SEQ ID NO: 171 - protein, 334 aa, synthetic construct
ETRECIYYNANWELERTNQSGLERCEGEQDKRLHCYASWRNSSGTIELVKKGCWLDDFNCYDRQECVATEENPQVYFCCCEGNFCNERFTHLPEAGGPEVTYEPPPTGGGTHTCPPCPAPELLGGPSVFLFPPKPKDTLMISRTPEVTCVVVDVSHEDPEVKFNWYVDGVEVHNAKTKPREEQYNSTYRVVSVLTVLHQDWLNGKEYKCKVSNKALPAPIEKTISKAKGQPREPQVYTLPPSRDELTKNQVSLTCLVKGFYPSDIAVEWESNGQPENNYKTTPPVLDSDGSFFLYSKLTVDKSRWQQGNVFSCSVMHEALHNHYTQKSLSLSPG

SEQ ID NO: 172 - protein, 345 aa, synthetic construct
ETRECIYYNANWELERTNQSGLERCEGEQDKRLHCYASWRNSSGTIELVKKGCWLDDFNCYDRQECVATEENPQVYFCCCEGNFCNERFTHLPEAGGPEVTYEPPPTGGGGSGGGGSGGGGTHTCPPCPAPELLGGPSVFLFPPKPKDTLMISRTPEVTCVVVDVSHEDPEVKFNWYVDGVEVHNAKTKPREEQYNSTYRVVSVLTVLHQDWLNGKEYKCKVSNKALPAPIEKTISKAKGQPREPQVYTLPPSRDELTKNQVSLTCLVKGFYPSDIAVEWESNGQPENNYKTTPPVLDSDGSFFLYSKLTVDKSRWQQGNVFSCSVMHEALHNHYTQKSLSLSPG

SEQ ID NO: 173 - protein, 343 aa, synthetic construct
ILGRSETQECLFFNANWEKDRTNQTGVEPCYGDKDKRRHCFATWKNISGSIEIVKQGCWLDDINCYDRTDCVEKKDSPEVYFCCCEGNMCNEKFSYFPEMEVTQPTSNPVTPKPPTGGGTHTCPPCPAPELLGGPSVFLFPPKPKDTLMISRTPEVTCVVVDVSHEDPEVKFNWYVDGVEVHNAKTKPREEQYNSTYRVVSVLTVLHQDWLNGKEYKCKVSNKALPVPIEKTISKAKGQPREPQVYTLPPSREEMTKNQVSLTCLVKGFYPSDIAVEWESNGQPENNYKTTPPVLDSDGSFFLYSKLTVDKSRWQQGNVFSCSVMHEALHNHYTQKSLSLSPG

SEQ ID NO: 174 - protein, 345 aa, synthetic construct
ETRECIYYNANWELERTNQSGLERCEEEQDKRLHCYASWRNSSGTIELVKKGCWLDDFNCYDRQECVATEENPQVYFCCCEGNFCNERFTHLPEAGGPEVTYEPPPTGGGGSGGGGSGGGGTHTCPPCPAPELLGGPSVFLFPPKPKDTLMISRTPEVTCVVVDVSHEDPEVKFNWYVDGVEVHNAKTKPREEQYNSTYRVVSVLTVLHQDWLNGKEYKCKVSNKALPAPIEKTISKAKGQPREPQVYTLPPSRDELTKNQVSLTCLVKGFYPSDIAVEWESNGQPENNYKTTPPVLDSDGSFFLYSKLTVDKSRWQQGNVFSCSVMHEALHNHYTQKSLSLSPG

SEQ ID NO: 175 - protein, 345 aa, synthetic construct
ETRECIYYNANWELERTNQSGLERCEGEQDKRRHCYASWRNSSGTIELVKKGCWLDDFNCYDRQECVATEENPQVYFCCCEGNFCNERFTHLPEAGGPEVTYEPPPTGGGGSGGGGSGGGGTHTCPPCPAPELLGGPSVFLFPPKPKDTLMISRTPEVTCVVVDVSHEDPEVKFNWYVDGVEVHNAKTKPREEQYNSTYRVVSVLTVLHQDWLNGKEYKCKVSNKALPAPIEKTISKAKGQPREPQVYTLPPSRDELTKNQVSLTCLVKGFYPSDIAVEWESNGQPENNYKTTPPVLDSDGSFFLYSKLTVDKSRWQQGNVFSCSVMHEALHNHYTQKSLSLSPG

SEQ ID NO: 176 - protein, 345 aa, synthetic construct
ETRECIYYNANWELERTNQSGLERCEGEQDKRYHCYASWRNSSGTIELVKKGCWLDDFNCYDRQECVATEENPQVYFCCCEGNFCNERFTHLPEAGGPEVTYEPPPTGGGGSGGGGSGGGGTHTCPPCPAPELLGGPSVFLFPPKPKDTLMISRTPEVTCVVVDVSHEDPEVKFNWYVDGVEVHNAKTKPREEQYNSTYRVVSVLTVLHQDWLNGKEYKCKVSNKALPAPIEKTISKAKGQPREPQVYTLPPSRDELTKNQVSLTCLVKGFYPSDIAVEWESNGQPENNYKTTPPVLDSDGSFFLYSKLTVDKSRWQQGNVFSCSVMHEALHNHYTQKSLSLSPG

SEQ ID NO: 177 - protein, 345 aa, synthetic construct
ETRECIYYNANWELERTNQSGLERCEGEQDKRLHCYASWRNSSGTIELVKKGCWLDDFNCYDRQECVAHEENPQVYFCCCEGNFCNERFTHLPEAGGPEVTYEPPPTGGGGSGGGGSGGGGTHTCPPCPAPELLGGPSVFLFPPKPKDTLMISRTPEVTCVVVDVSHEDPEVKFNWYVDGVEVHNAKTKPREEQYNSTYRVVSVLTVLHQDWLNGKEYKCKVSNKALPAPIEKTISKAKGQPREPQVYTLPPSRDELTKNQVSLTCLVKGFYPSDIAVEWESNGQPENNYKTTPPVLDSDGSFFLYSKLTVDKSRWQQGNVFSCSVMHEALHNHYTQKSLSLSPG

SEQ ID NO: 178 - protein, 345 aa, synthetic construct
ETRECIYYNANWELERTNQSGLERCEGEQDKRLHCYASWRNSSGTIELVKKGCWLDDFNCYDRQECVAQEENPQVYFCCCEGNFCNERFTHLPEAGGPEVTYEPPPTGGGGSGGGGSGGGGTHTCPPCPAPELLGGPSVFLFPPKPKDTLMISRTPEVTCVVVDVSHEDPEVKFNWYVDGVEVHNAKTKPREEQYNSTYRVVSVLTVLHQDWLNGKEYKCKVSNKALPAPIEKTISKAKGQPREPQVYTLPPSRDELTKNQVSLTCLVKGFYPSDIAVEWESNGQPENNYKTTPPVLDSDGSFFLYSKLTVDKSRWQQGNVFSCSVMHEALHNHYTQKSLSLSPG

SEQ ID NO: 179 - protein, 334 aa, synthetic construct
ETRECIYYNANWELERTNQSGLERCEEEQDKRLHCYASWRNSSGTIELVKKGCWLDDFNCYDRQECVATEENPQVYFCCCEGNFCNERFTHLPEAGGPEVTYEPPPTGGGTHTCPPCPAPELLGGPSVFLFPPKPKDTLMISRTPEVTCVVVDVSHEDPEVKFNWYVDGVEVHNAKTKPREEQYNSTYRVVSVLTVLHQDWLNGKEYKCKVSNKALPAPIEKTISKAKGQPREPQVYTLPPSRDELTKNQVSLTCLVKGFYPSDIAVEWESNGQPENNYKTTPPVLDSDGSFFLYSKLTVDKSRWQQGNVFSCSVMHEALHNHYTQKSLSLSPG

SEQ ID NO: 180 - protein, 334 aa, synthetic construct
ETRECIYYNANWELERTNQSGLERCEGEQDKRYHCYASWRNSSGTIELVKKGCWLDDFNCYDRQECVATEENPQVYFCCCEGNFCNERFTHLPEAGGPEVTYEPPPTGGGTHTCPPCPAPELLGGPSVFLFPPKPKDTLMISRTPEVTCVVVDVSHEDPEVKFNWYVDGVEVHNAKTKPREEQYNSTYRVVSVLTVLHQDWLNGKEYKCKVSNKALPAPIEKTISKAKGQPREPQVYTLPPSRDELTKNQVSLTCLVKGFYPSDIAVEWESNGQPENNYKTTPPVLDSDGSFFLYSKLTVDKSRWQQGNVFSCSVMHEALHNHYTQKSLSLSPG

SEQ ID NO: 181 - protein, 334 aa, synthetic construct
ETRECIYYNANWELERTNQSGLERCEGEQDKRLHCYASWRNSSGTIELVKKGCWLDDFNCYDRQECVAHEENPQVYFCCCEGNFCNERFTHLPEAGGPEVTYEPPPTGGGTHTCPPCPAPELLGGPSVFLFPPKPKDTLMISRTPEVTCVVVDVSHEDPEVKFNWYVDGVEVHNAKTKPREEQYNSTYRVVSVLTVLHQDWLNGKEYKCKVSNKALPAPIEKTISKAKGQPREPQVYTLPPSRDELTKNQVSLTCLVKGFYPSDIAVEWESNGQPENNYKTTPPVLDSDGSFFLYSKLTVDKSRWQQGNVFSCSVMHEALHNHYTQKSLSLSPG

SEQ ID NO: 182 - protein, 334 aa, synthetic construct
ETRECIYYNANWELERTNQSGLERCEGEQDKRLHCYASWRNSSGTIELVKKGCWLDDFNCYDRQECVAQEENPQVYFCCCEGNFCNERFTHLPEAGGPEVTYEPPPTGGGTHTCPPCPAPELLGGPSVFLFPPKPKDTLMISRTPEVTCVVVDVSHEDPEVKFNWYVDGVEVHNAKTKPREEQYNSTYRVVSVLTVLHQDWLNGKEYKCKVSNKALPAPIEKTISKAKGQPREPQVYTLPPSRDELTKNQVSLTCLVKGFYPSDIAVEWESNGQPENNYKTTPPVLDSDGSFFLYSKLTVDKSRWQQGNVFSCSVMHEALHNHYTQKSLSLSPG

SEQ ID NO: 183 - protein, 334 aa, synthetic construct
ETRECIYYNANWELERTNQSGLERCEGEQDKRYHCYASWRNSSGTIELVKKGCWLDDFNCYDRQECVAHEENPQVYFCCCEGNFCNERFTHLPEAGGPEVTYEPPPTGGGTHTCPPCPAPELLGGPSVFLFPPKPKDTLMISRTPEVTCVVVDVSHEDPEVKFNWYVDGVEVHNAKTKPREEQYNSTYRVVSVLTVLHQDWLNGKEYKCKVSNKALPAPIEKTISKAKGQPREPQVYTLPPSRDELTKNQVSLTCLVKGFYPSDIAVEWESNGQPENNYKTTPPVLDSDGSFFLYSKLTVDKSRWQQGNVFSCSVMHEALHNHYTQKSLSLSPG

SEQ ID NO: 184 - protein, 341 aa, synthetic construct
ETRECIYYNANWELERTNQSGLERCEGEQDKRYHCYASWRNSSGTIELVKKGCWLDDFNCYDRQECVAHEENPQVYFCCCEGNFCNERFTHLPEAGGPEVTYEPPPTGGGGSGGGGSTHTCPPCPAPELLGGPSVFLFPPKPKDTLMISRTPEVTCVVVDVSHEDPEVKFNWYVDGVEVHNAKTKPREEQYNSTYRVVSVLTVLHQDWLNGKEYKCKVSNKALPAPIEKTISKAKGQPREPQVYTLPPSRDELTKNQVSLTCLVKGFYPSDIAVEWESNGQPENNYKTTPPVLDSDGSFFLYSKLTVDKSRWQQGNVFSCSVMHEALHNHYTQKSLSLSPG

SEQ ID NO: 185 - protein, 345 aa, synthetic construct
ETRECIYYNANWELERTNQSGLERCEGEQDKRYHCYASWRNSSGTIELVKKGCWLDDFNCYDRQECVAHEENPQVYFCCCEGNFCNERFTHLPEAGGPEVTYEPPPTGGGGSGGGGSGGGGTHTCPPCPAPELLGGPSVFLFPPKPKDTLMISRTPEVTCVVVDVSHEDPEVKFNWYVDGVEVHNAKTKPREEQYNSTYRVVSVLTVLHQDWLNGKEYKCKVSNKALPAPIEKTISKAKGQPREPQVYTLPPSRDELTKNQVSLTCLVKGFYPSDIAVEWESNGQPENNYKTTPPVLDSDGSFFLYSKLTVDKSRWQQGNVFSCSVMHEALHNHYTQKSLSLSPG

SEQ ID NO: 186 - protein, 334 aa, synthetic construct
ETRECIYYNANWELERTNQSGLERCEGEQDKRYHCYASWRNSSGTIELVKKGCWLDDFNCYDRQECVAQEENPQVYFCCCEGNFCNERFTHLPEAGGPEVTYEPPPTGGGTHTCPPCPAPELLGGPSVFLFPPKPKDTLMISRTPEVTCVVVDVSHEDPEVKFNWYVDGVEVHNAKTKPREEQYNSTYRVVSVLTVLHQDWLNGKEYKCKVSNKALPAPIEKTISKAKGQPREPQVYTLPPSRDELTKNQVSLTCLVKGFYPSDIAVEWESNGQPENNYKTTPPVLDSDGSFFLYSKLTVDKSRWQQGNVFSCSVMHEALHNHYTQKSLSLSPG

SEQ ID NO: 187 - protein, 341 aa, synthetic construct
ETRECIYYNANWELERTNQSGLERCEGEQDKRYHCYASWRNSSGTIELVKKGCWLDDFNCYDRQECVAQEENPQVYFCCCEGNFCNERFTHLPEAGGPEVTYEPPPTGGGGSGGGGSTHTCPPCPAPELLGGPSVFLFPPKPKDTLMISRTPEVTCVVVDVSHEDPEVKFNWYVDGVEVHNAKTKPREEQYNSTYRVVSVLTVLHQDWLNGKEYKCKVSNKALPAPIEKTISKAKGQPREPQVYTLPPSRDELTKNQVSLTCLVKGFYPSDIAVEWESNGQPENNYKTTPPVLDSDGSFFLYSKLTVDKSRWQQGNVFSCSVMHEALHNHYTQKSLSLSPG

SEQ ID NO: 188 - protein, 345 aa, synthetic construct
ETRECIYYNANWELERTNQSGLERCEGEQDKRYHCYASWRNSSGTIELVKKGCWLDDFNCYDRQECVAQEENPQVYFCCCEGNFCNERFTHLPEAGGPEVTYEPPPTGGGGSGGGGSGGGGTHTCPPCPAPELLGGPSVFLFPPKPKDTLMISRTPEVTCVVVDVSHEDPEVKFNWYVDGVEVHNAKTKPREEQYNSTYRVVSVLTVLHQDWLNGKEYKCKVSNKALPAPIEKTISKAKGQPREPQVYTLPPSRDELTKNQVSLTCLVKGFYPSDIAVEWESNGQPENNYKTTPPVLDSDGSFFLYSKLTVDKSRWQQGNVFSCSVMHEALHNHYTQKSLSLSPG

SEQ ID NO: 189 - protein, 334 aa, synthetic construct
ETRECIYYNANWELERTNQSGLERCEGEQDKRYHCYASWRNSSGTIELVKKGCWLDDFNCYDRQECVAEEENPQVYFCCCEGNFCNERFTHLPEAGGPEVTYEPPPTGGGTHTCPPCPAPELLGGPSVFLFPPKPKDTLMISRTPEVTCVVVDVSHEDPEVKFNWYVDGVEVHNAKTKPREEQYNSTYRVVSVLTVLHQDWLNGKEYKCKVSNKALPAPIEKTISKAKGQPREPQVYTLPPSRDELTKNQVSLTCLVKGFYPSDIAVEWESNGQPENNYKTTPPVLDSDGSFFLYSKLTVDKSRWQQGNVFSCSVMHEALHNHYTQKSLSLSPG

SEQ ID NO: 190 - protein, 341 aa, synthetic construct
ETRECIYYNANWELERTNQSGLERCEGEQDKRYHCYASWRNSSGTIELVKKGCWLDDFNCYDRQECVAEEENPQVYFCCCEGNFCNERFTHLPEAGGPEVTYEPPPTGGGGSGGGGSTHTCPPCPAPELLGGPSVFLFPPKPKDTLMISRTPEVTCVVVDVSHEDPEVKFNWYVDGVEVHNAKTKPREEQYNSTYRVVSVLTVLHQDWLNGKEYKCKVSNKALPAPIEKTISKAKGQPREPQVYTLPPSRDELTKNQVSLTCLVKGFYPSDIAVEWESNGQPENNYKTTPPVLDSDGSFFLYSKLTVDKSRWQQGNVFSCSVMHEALHNHYTQKSLSLSPG

SEQ ID NO: 191 - protein, 345 aa, synthetic construct
ETRECIYYNANWELERTNQSGLERCEGEQDKRYHCYASWRNSSGTIELVKKGCWLDDFNCYDRQECVAEEENPQVYFCCCEGNFCNERFTHLPEAGGPEVTYEPPPTGGGGSGGGGSGGGGTHTCPPCPAPELLGGPSVFLFPPKPKDTLMISRTPEVTCVVVDVSHEDPEVKFNWYVDGVEVHNAKTKPREEQYNSTYRVVSVLTVLHQDWLNGKEYKCKVSNKALPAPIEKTISKAKGQPREPQVYTLPPSRDELTKNQVSLTCLVKGFYPSDIAVEWESNGQPENNYKTTPPVLDSDGSFFLYSKLTVDKSRWQQGNVFSCSVMHEALHNHYTQKSLSLSPG

SEQ ID NO: 192 - protein, 334 aa, synthetic construct
ETRECIYYNANWELERTNQSGLERCEDEQDKRYHCYASWRNSSGTIELVKKGCWLDDFNCYDRQECVATEENPQVYFCCCEGNFCNERFTHLPEAGGPEVTYEPPPTGGGTHTCPPCPAPELLGGPSVFLFPPKPKDTLMISRTPEVTCVVVDVSHEDPEVKFNWYVDGVEVHNAKTKPREEQYNSTYRVVSVLTVLHQDWLNGKEYKCKVSNKALPAPIEKTISKAKGQPREPQVYTLPPSRDELTKNQVSLTCLVKGFYPSDIAVEWESNGQPENNYKTTPPVLDSDGSFFLYSKLTVDKSRWQQGNVFSCSVMHEALHNHYTQKSLSLSPG

SEQ ID NO: 193 - protein, 341 aa, synthetic construct
ETRECIYYNANWELERTNQSGLERCEDEQDKRYHCYASWRNSSGTIELVKKGCWLDDFNCYDRQECVATEENPQVYFCCCEGNFCNERFTHLPEAGGPEVTYEPPPTGGGGSGGGGSTHTCPPCPAPELLGGPSVFLFPPKPKDTLMISRTPEVTCVVVDVSHEDPEVKFNWYVDGVEVHNAKTKPREEQYNSTYRVVSVLTVLHQDWLNGKEYKCKVSNKALPAPIEKTISKAKGQPREPQVYTLPPSRDELTKNQVSLTCLVKGFYPSDIAVEWESNGQPENNYKTTPPVLDSDGSFFLYSKLTVDKSRWQQGNVFSCSVMHEALHNHYTQKSLSLSPG

SEQ ID NO: 194 - protein, 345 aa, synthetic construct
ETRECIYYNANWELERTNQSGLERCEDEQDKRYHCYASWRNSSGTIELVKKGCWLDDFNCYDRQECVATEENPQVYFCCCEGNFCNERFTHLPEAGGPEVTYEPPPTGGGGSGGGGSGGGGTHTCPPCPAPELLGGPSVFLFPPKPKDTLMISRTPEVTCVVVDVSHEDPEVKFNWYVDGVEVHNAKTKPREEQYNSTYRVVSVLTVLHQDWLNGKEYKCKVSNKALPAPIEKTISKAKGQPREPQVYTLPPSRDELTKNQVSLTCLVKGFYPSDIAVEWESNGQPENNYKTTPPVLDSDGSFFLYSKLTVDKSRWQQGNVFSCSVMHEALHNHYTQKSLSLSPG

SEQ ID NO: 195 - protein, 334 aa, synthetic construct
ETRECIYYNANWELERTNQSGLERCEEEQDKRYHCYASWRNSSGTIELVKKGCWLDDFNCYDRQECVATEENPQVYFCCCEGNFCNERFTHLPEAGGPEVTYEPPPTGGGTHTCPPCPAPELLGGPSVFLFPPKPKDTLMISRTPEVTCVVVDVSHEDPEVKFNWYVDGVEVHNAKTKPREEQYNSTYRVVSVLTVLHQDWLNGKEYKCKVSNKALPAPIEKTISKAKGQPREPQVYTLPPSRDELTKNQVSLTCLVKGFYPSDIAVEWESNGQPENNYKTTPPVLDSDGSFFLYSKLTVDKSRWQQGNVFSCSVMHEALHNHYTQKSLSLSPG

SEQ ID NO: 196 - protein, 341 aa, synthetic construct
ETRECIYYNANWELERTNQSGLERCEEEQDKRYHCYASWRNSSGTIELVKKGCWLDDFNCYDRQECVATEENPQVYFCCCEGNFCNERFTHLPEAGGPEVTYEPPPTGGGGSGGGGSTHTCPPCPAPELLGGPSVFLFPPKPKDTLMISRTPEVTCVVVDVSHEDPEVKFNWYVDGVEVHNAKTKPREEQYNSTYRVVSVLTVLHQDWLNGKEYKCKVSNKALPAPIEKTISKAKGQPREPQVYTLPPSRDELTKNQVSLTCLVKGFYPSDIAVEWESNGQPENNYKTTPPVLDSDGSFFLYSKLTVDKSRWQQGNVFSCSVMHEALHNHYTQKSLSLSPG

SEQ ID NO: 197 - protein, 345 aa, synthetic construct
ETRECIYYNANWELERTNQSGLERCEEEQDKRYHCYASWRNSSGTIELVKKGCWLDDFNCYDRQECVATEENPQVYFCCCEGNFCNERFTHLPEAGGPEVTYEPPPTGGGGSGGGGSGGGGTHTCPPCPAPELLGGPSVFLFPPKPKDTLMISRTPEVTCVVVDVSHEDPEVKFNWYVDGVEVHNAKTKPREEQYNSTYRVVSVLTVLHQDWLNGKEYKCKVSNKALPAPIEKTISKAKGQPREPQVYTLPPSRDELTKNQVSLTCLVKGFYPSDIAVEWESNGQPENNYKTTPPVLDSDGSFFLYSKLTVDKSRWQQGNVFSCSVMHEALHNHYTQKSLSLSPG

SEQ ID NO: 198 - protein, 334 aa, synthetic construct
ETRECIYYNANWELERTNQSGLERCEGEQDKRFHCYASWRNSSGTIELVKKGCWLDDFNCYDRQECVAQEENPQVYFCCCEGNFCNERFTHLPEAGGPEVTYEPPPTGGGTHTCPPCPAPELLGGPSVFLFPPKPKDTLMISRTPEVTCVVVDVSHEDPEVKFNWYVDGVEVHNAKTKPREEQYNSTYRVVSVLTVLHQDWLNGKEYKCKVSNKALPAPIEKTISKAKGQPREPQVYTLPPSRDELTKNQVSLTCLVKGFYPSDIAVEWESNGQPENNYKTTPPVLDSDGSFFLYSKLTVDKSRWQQGNVFSCSVMHEALHNHYTQKSLSLSPG

SEQ ID NO: 199 - protein, 341 aa, synthetic construct
ETRECIYYNANWELERTNQSGLERCEGEQDKRFHCYASWRNSSGTIELVKKGCWLDDFNCYDRQECVAQEENPQVYFCCCEGNFCNERFTHLPEAGGPEVTYEPPPTGGGGSGGGGSTHTCPPCPAPELLGGPSVFLFPPKPKDTLMISRTPEVTCVVVDVSHEDPEVKFNWYVDGVEVHNAKTKPREEQYNSTYRVVSVLTVLHQDWLNGKEYKCKVSNKALPAPIEKTISKAKGQPREPQVYTLPPSRDELTKNQVSLTCLVKGFYPSDIAVEWESNGQPENNYKTTPPVLDSDGSFFLYSKLTVDKSRWQQGNVFSCSVMHEALHNHYTQKSLSLSPG

SEQ ID NO: 200 - protein, 345 aa, synthetic construct
ETRECIYYNANWELERTNQSGLERCEGEQDKRFHCYASWRNSSGTIELVKKGCWLDDFNCYDRQECVAQEENPQVYFCCCEGNFCNERFTHLPEAGGPEVTYEPPPTGGGGSGGGGSGGGGTHTCPPCPAPELLGGPSVFLFPPKPKDTLMISRTPEVTCVVVDVSHEDPEVKFNWYVDGVEVHNAKTKPREEQYNSTYRVVSVLTVLHQDWLNGKEYKCKVSNKALPAPIEKTISKAKGQPREPQVYTLPPSRDELTKNQVSLTCLVKGFYPSDIAVEWESNGQPENNYKTTPPVLDSDGSFFLYSKLTVDKSRWQQGNVFSCSVMHEALHNHYTQKSLSLSPG

SEQ ID NO: 201 - protein, 334 aa, synthetic construct
ETRECIYYNANWELERTNQSGLERCEGEQDKRLHCYASWRNSSGTIELVKKGCWLDDFNCYDRQECVAEEENPQVYFCCCEGNFCNERFTHLPEAGGPEVTYEPPPTGGGTHTCPPCPAPELLGGPSVFLFPPKPKDTLMISRTPEVTCVVVDVSHEDPEVKFNWYVDGVEVHNAKTKPREEQYNSTYRVVSVLTVLHQDWLNGKEYKCKVSNKALPAPIEKTISKAKGQPREPQVYTLPPSRDELTKNQVSLTCLVKGFYPSDIAVEWESNGQPENNYKTTPPVLDSDGSFFLYSKLTVDKSRWQQGNVFSCSVMHEALHNHYTQKSLSLSPG

SEQ ID NO: 202 - protein, 341 aa, synthetic construct
ETRECIYYNANWELERTNQSGLERCEGEQDKRLHCYASWRNSSGTIELVKKGCWLDDFNCYDRQECVAEEENPQVYFCCCEGNFCNERFTHLPEAGGPEVTYEPPPTGGGGSGGGGSTHTCPPCPAPELLGGPSVFLFPPKPKDTLMISRTPEVTCVVVDVSHEDPEVKFNWYVDGVEVHNAKTKPREEQYNSTYRVVSVLTVLHQDWLNGKEYKCKVSNKALPAPIEKTISKAKGQPREPQVYTLPPSRDELTKNQVSLTCLVKGFYPSDIAVEWESNGQPENNYKTTPPVLDSDGSFFLYSKLTVDKSRWQQGNVFSCSVMHEALHNHYTQKSLSLSPG

SEQ ID NO: 203 - protein, 345 aa, synthetic construct
ETRECIYYNANWELERTNQSGLERCEGEQDKRLHCYASWRNSSGTIELVKKGCWLDDFNCYDRQECVAEEENPQVYFCCCEGNFCNERFTHLPEAGGPEVTYEPPPTGGGGSGGGGSGGGGTHTCPPCPAPELLGGPSVFLFPPKPKDTLMISRTPEVTCVVVDVSHEDPEVKFNWYVDGVEVHNAKTKPREEQYNSTYRVVSVLTVLHQDWLNGKEYKCKVSNKALPAPIEKTISKAKGQPREPQVYTLPPSRDELTKNQVSLTCLVKGFYPSDIAVEWESNGQPENNYKTTPPVLDSDGSFFLYSKLTVDKSRWQQGNVFSCSVMHEALHNHYTQKSLSLSPG

SEQ ID NO: 204 - protein, 334 aa, synthetic construct
ETRECIYYNANWELERTNQSGLERCEGEQDKRFHCYASWRNSSGTIELVKKGCWLDDFNCYDRQECVATEENPQVYFCCCEGNFCNERFTHLPEAGGPEVTYEPPPTGGGTHTCPPCPAPELLGGPSVFLFPPKPKDTLMISRTPEVTCVVVDVSHEDPEVKFNWYVDGVEVHNAKTKPREEQYNSTYRVVSVLTVLHQDWLNGKEYKCKVSNKALPAPIEKTISKAKGQPREPQVYTLPPSRDELTKNQVSLTCLVKGFYPSDIAVEWESNGQPENNYKTTPPVLDSDGSFFLYSKLTVDKSRWQQGNVFSCSVMHEALHNHYTQKSLSLSPG

SEQ ID NO: 205 - protein, 341 aa, synthetic construct
ETRECIYYNANWELERTNQSGLERCEGEQDKRFHCYASWRNSSGTIELVKKGCWLDDFNCYDRQECVATEENPQVYFCCCEGNFCNERFTHLPEAGGPEVTYEPPPTGGGGSGGGGSTHTCPPCPAPELLGGPSVFLFPPKPKDTLMISRTPEVTCVVVDVSHEDPEVKFNWYVDGVEVHNAKTKPREEQYNSTYRVVSVLTVLHQDWLNGKEYKCKVSNKALPAPIEKTISKAKGQPREPQVYTLPPSRDELTKNQVSLTCLVKGFYPSDIAVEWESNGQPENNYKTTPPVLDSDGSFFLYSKLTVDKSRWQQGNVFSCSVMHEALHNHYTQKSLSLSPG

SEQ ID NO: 206 - protein, 345 aa, synthetic construct
ETRECIYYNANWELERTNQSGLERCEGEQDKRFHCYASWRNSSGTIELVKKGCWLDDFNCYDRQECVATEENPQVYFCCCEGNFCNERFTHLPEAGGPEVTYEPPPTGGGGSGGGGSGGGGTHTCPPCPAPELLGGPSVFLFPPKPKDTLMISRTPEVTCVVVDVSHEDPEVKFNWYVDGVEVHNAKTKPREEQYNSTYRVVSVLTVLHQDWLNGKEYKCKVSNKALPAPIEKTISKAKGQPREPQVYTLPPSRDELTKNQVSLTCLVKGFYPSDIAVEWESNGQPENNYKTTPPVLDSDGSFFLYSKLTVDKSRWQQGNVFSCSVMHEALHNHYTQKSLSLSPG

SEQ ID NO: 207 - protein, 334 aa, synthetic construct
ETRECIYYNANWELERTNQSGLERCEGEQDKRQHCYASWRNSSGTIELVKKGCWLDDFNCYDRQECVATEENPQVYFCCCEGNFCNERFTHLPEAGGPEVTYEPPPTGGGTHTCPPCPAPELLGGPSVFLFPPKPKDTLMISRTPEVTCVVVDVSHEDPEVKFNWYVDGVEVHNAKTKPREEQYNSTYRVVSVLTVLHQDWLNGKEYKCKVSNKALPAPIEKTISKAKGQPREPQVYTLPPSRDELTKNQVSLTCLVKGFYPSDIAVEWESNGQPENNYKTTPPVLDSDGSFFLYSKLTVDKSRWQQGNVFSCSVMHEALHNHYTQKSLSLSPG

SEQ ID NO: 208 - protein, 341 aa, synthetic construct
ETRECIYYNANWELERTNQSGLERCEGEQDKRQHCYASWRNSSGTIELVKKGCWLDDFNCYDRQECVATEENPQVYFCCCEGNFCNERFTHLPEAGGPEVTYEPPPTGGGGSGGGGSTHTCPPCPAPELLGGPSVFLFPPKPKDTLMISRTPEVTCVVVDVSHEDPEVKFNWYVDGVEVHNAKTKPREEQYNSTYRVVSVLTVLHQDWLNGKEYKCKVSNKALPAPIEKTISKAKGQPREPQVYTLPPSRDELTKNQVSLTCLVKGFYPSDIAVEWESNGQPENNYKTTPPVLDSDGSFFLYSKLTVDKSRWQQGNVFSCSVMHEALHNHYTQKSLSLSPG

SEQ ID NO: 209 - protein, 345 aa, synthetic construct
ETRECIYYNANWELERTNQSGLERCEGEQDKRQHCYASWRNSSGTIELVKKGCWLDDFNCYDRQECVATEENPQVYFCCCEGNFCNERFTHLPEAGGPEVTYEPPPTGGGGSGGGGSGGGGTHTCPPCPAPELLGGPSVFLFPPKPKDTLMISRTPEVTCVVVDVSHEDPEVKFNWYVDGVEVHNAKTKPREEQYNSTYRVVSVLTVLHQDWLNGKEYKCKVSNKALPAPIEKTISKAKGQPREPQVYTLPPSRDELTKNQVSLTCLVKGFYPSDIAVEWESNGQPENNYKTTPPVLDSDGSFFLYSKLTVDKSRWQQGNVFSCSVMHEALHNHYTQKSLSLSPG

SEQ ID NO: 210 - protein, 341 aa, synthetic construct
ETRECIYYNANWELERTNQSGLERCEGEQDKRYHCYASWRNSSGTIELVKKGCWLDDFNCYDRQECVATEENPQVYFCCCEGNFCNERFTHLPEAGGPEVTYEPPPTGGGGSGGGGSTHTCPPCPAPELLGGPSVFLFPPKPKDTLMISRTPEVTCVVVDVSHEDPEVKFNWYVDGVEVHNAKTKPREEQYNSTYRVVSVLTVLHQDWLNGKEYKCKVSNKALPAPIEKTISKAKGQPREPQVYTLPPSRDELTKNQVSLTCLVKGFYPSDIAVEWESNGQPENNYKTTPPVLDSDGSFFLYSKLTVDKSRWQQGNVFSCSVMHEALHNHYTQKSLSLSPG

SEQ ID NO: 211 - protein, 345 aa, synthetic construct
ETRECIYYNANWELERTNQSGLERCEGEQDKRWHCYASWRNSSGTIELVKKGCWLDDFNCYDRQECVATEENPQVYFCCCEGNFCNERFTHLPEAGGPEVTYEPPPTGGGGSGGGGSGGGGTHTCPPCPAPELLGGPSVFLFPPKPKDTLMISRTPEVTCVVVDVSHEDPEVKFNWYVDGVEVHNAKTKPREEQYNSTYRVVSVLTVLHQDWLNGKEYKCKVSNKALPAPIEKTISKAKGQPREPQVYTLPPSRDELTKNQVSLTCLVKGFYPSDIAVEWESNGQPENNYKTTPPVLDSDGSFFLYSKLTVDKSRWQQGNVFSCSVMHEALHNHYTQKSLSLSPG

SEQ ID NO: 212 - protein, 345 aa, synthetic construct
ETRECIYYNANWELERTNQSGLERCEGEQDKREHCYASWRNSSGTIELVKKGCWLDDFNCYDRQECVATEENPQVYFCCCEGNFCNERFTHLPEAGGPEVTYEPPPTGGGGSGGGGSGGGGTHTCPPCPAPELLGGPSVFLFPPKPKDTLMISRTPEVTCVVVDVSHEDPEVKFNWYVDGVEVHNAKTKPREEQYNSTYRVVSVLTVLHQDWLNGKEYKCKVSNKALPAPIEKTISKAKGQPREPQVYTLPPSRDELTKNQVSLTCLVKGFYPSDIAVEWESNGQPENNYKTTPPVLDSDGSFFLYSKLTVDKSRWQQGNVFSCSVMHEALHNHYTQKSLSLSPG

SEQ ID NO: 213 - protein, 345 aa, synthetic construct
ETRECIYYNANWELERTNQSGLERCEGEQDKRKHCYASWRNSSGTIELVKKGCWLDDFNCYDRQECVATEENPQVYFCCCEGNFCNERFTHLPEAGGPEVTYEPPPTGGGGSGGGGSGGGGTHTCPPCPAPELLGGPSVFLFPPKPKDTLMISRTPEVTCVVVDVSHEDPEVKFNWYVDGVEVHNAKTKPREEQYNSTYRVVSVLTVLHQDWLNGKEYKCKVSNKALPAPIEKTISKAKGQPREPQVYTLPPSRDELTKNQVSLTCLVKGFYPSDIAVEWESNGQPENNYKTTPPVLDSDGSFFLYSKLTVDKSRWQQGNVFSCSVMHEALHNHYTQKSLSLSPG

SEQ ID NO: 214 - protein, 345 aa, synthetic construct
ETRECIYYNANWELERTNQSGLERCEGEQDKRMHCYASWRNSSGTIELVKKGCWLDDFNCYDRQECVATEENPQVYFCCCEGNFCNERFTHLPEAGGPEVTYEPPPTGGGGSGGGGSGGGGTHTCPPCPAPELLGGPSVFLFPPKPKDTLMISRTPEVTCVVVDVSHEDPEVKFNWYVDGVEVHNAKTKPREEQYNSTYRVVSVLTVLHQDWLNGKEYKCKVSNKALPAPIEKTISKAKGQPREPQVYTLPPSRDELTKNQVSLTCLVKGFYPSDIAVEWESNGQPENNYKTTPPVLDSDGSFFLYSKLTVDKSRWQQGNVFSCSVMHEALHNHYTQKSLSLSPG

SEQ ID NO: 215 - protein, 345 aa, synthetic construct
ETRECIYYNANWELERTNQSGLERCENEQDKRYHCYASWRNSSGTIELVKKGCWLDDFNCYDRQECVATEENPQVYFCCCEGNFCNERFTHLPEAGGPEVTYEPPPTGGGGSGGGGSGGGGTHTCPPCPAPELLGGPSVFLFPPKPKDTLMISRTPEVTCVVVDVSHEDPEVKFNWYVDGVEVHNAKTKPREEQYNSTYRVVSVLTVLHQDWLNGKEYKCKVSNKALPAPIEKTISKAKGQPREPQVYTLPPSRDELTKNQVSLTCLVKGFYPSDIAVEWESNGQPENNYKTTPPVLDSDGSFFLYSKLTVDKSRWQQGNVFSCSVMHEALHNHYTQKSLSLSPG

SEQ ID NO: 216 - protein, 345 aa, synthetic construct
ETRECIYYNANWELERTNQSGLERCEQEQDKRYHCYASWRNSSGTIELVKKGCWLDDFNCYDRQECVATEENPQVYFCCCEGNFCNERFTHLPEAGGPEVTYEPPPTGGGGSGGGGSGGGGTHTCPPCPAPELLGGPSVFLFPPKPKDTLMISRTPEVTCVVVDVSHEDPEVKFNWYVDGVEVHNAKTKPREEQYNSTYRVVSVLTVLHQDWLNGKEYKCKVSNKALPAPIEKTISKAKGQPREPQVYTLPPSRDELTKNQVSLTCLVKGFYPSDIAVEWESNGQPENNYKTTPPVLDSDGSFFLYSKLTVDKSRWQQGNVFSCSVMHEALHNHYTQKSLSLSPG

SEQ ID NO: 217 - protein, 345 aa, synthetic construct
ETRECIYYNANWELERTNQSGLERCEKEQDKRYHCYASWRNSSGTIELVKKGCWLDDFNCYDRQECVATEENPQVYFCCCEGNFCNERFTHLPEAGGPEVTYEPPPTGGGGSGGGGSGGGGTHTCPPCPAPELLGGPSVFLFPPKPKDTLMISRTPEVTCVVVDVSHEDPEVKFNWYVDGVEVHNAKTKPREEQYNSTYRVVSVLTVLHQDWLNGKEYKCKVSNKALPAPIEKTISKAKGQPREPQVYTLPPSRDELTKNQVSLTCLVKGFYPSDIAVEWESNGQPENNYKTTPPVLDSDGSFFLYSKLTVDKSRWQQGNVFSCSVMHEALHNHYTQKSLSLSPG

SEQ ID NO: 218 - protein, 345 aa, synthetic construct
ETRECIYYNANWELERTNQSGLERCETEQDKRYHCYASWRNSSGTIELVKKGCWLDDFNCYDRQECVATEENPQVYFCCCEGNFCNERFTHLPEAGGPEVTYEPPPTGGGGSGGGGSGGGGTHTCPPCPAPELLGGPSVFLFPPKPKDTLMISRTPEVTCVVVDVSHEDPEVKFNWYVDGVEVHNAKTKPREEQYNSTYRVVSVLTVLHQDWLNGKEYKCKVSNKALPAPIEKTISKAKGQPREPQVYTLPPSRDELTKNQVSLTCLVKGFYPSDIAVEWESNGQPENNYKTTPPVLDSDGSFFLYSKLTVDKSRWQQGNVFSCSVMHEALHNHYTQKSLSLSPG

SEQ ID NO: 219 - protein, 345 aa, synthetic construct
ETRECIYYNANWELERTNQSGLERCEMEQDKRYHCYASWRNSSGTIELVKKGCWLDDFNCYDRQECVATEENPQVYFCCCEGNFCNERFTHLPEAGGPEVTYEPPPTGGGGSGGGGSGGGGTHTCPPCPAPELLGGPSVFLFPPKPKDTLMISRTPEVTCVVVDVSHEDPEVKFNWYVDGVEVHNAKTKPREEQYNSTYRVVSVLTVLHQDWLNGKEYKCKVSNKALPAPIEKTISKAKGQPREPQVYTLPPSRDELTKNQVSLTCLVKGFYPSDIAVEWESNGQPENNYKTTPPVLDSDGSFFLYSKLTVDKSRWQQGNVFSCSVMHEALHNHYTQKSLSLSPG

SEQ ID NO: 220 - protein, 345 aa, synthetic construct
ETRECIYYNANWELERTNQSGLERCEGEQDKRYHCYASWRNSSGTIELVKKGCWLDDFNCYDRQECVAREENPQVYFCCCEGNFCNERFTHLPEAGGPEVTYEPPPTGGGGSGGGGSGGGGTHTCPPCPAPELLGGPSVFLFPPKPKDTLMISRTPEVTCVVVDVSHEDPEVKFNWYVDGVEVHNAKTKPREEQYNSTYRVVSVLTVLHQDWLNGKEYKCKVSNKALPAPIEKTISKAKGQPREPQVYTLPPSRDELTKNQVSLTCLVKGFYPSDIAVEWESNGQPENNYKTTPPVLDSDGSFFLYSKLTVDKSRWQQGNVFSCSVMHEALHNHYTQKSLSLSPG

SEQ ID NO: 221 - protein, 345 aa, synthetic construct
ETRECIYYNANWELERTNQSGLERCEGEQDKRYHCYASWRNSSGTIELVKKGCWLDDFNCYDRQECVAYEENPQVYFCCCEGNFCNERFTHLPEAGGPEVTYEPPPTGGGGSGGGGSGGGGTHTCPPCPAPELLGGPSVFLFPPKPKDTLMISRTPEVTCVVVDVSHEDPEVKFNWYVDGVEVHNAKTKPREEQYNSTYRVVSVLTVLHQDWLNGKEYKCKVSNKALPAPIEKTISKAKGQPREPQVYTLPPSRDELTKNQVSLTCLVKGFYPSDIAVEWESNGQPENNYKTTPPVLDSDGSFFLYSKLTVDKSRWQQGNVFSCSVMHEALHNHYTQKSLSLSPG

SEQ ID NO: 222 - protein, 345 aa, synthetic construct
ETRECIYYNANWELERTNQSGLERCEGEQDKRYHCYASWRNSSGTIELVKKGCWLDDFNCYDRQECVAWEENPQVYFCCCEGNFCNERFTHLPEAGGPEVTYEPPPTGGGGSGGGGSGGGGTHTCPPCPAPELLGGPSVFLFPPKPKDTLMISRTPEVTCVVVDVSHEDPEVKFNWYVDGVEVHNAKTKPREEQYNSTYRVVSVLTVLHQDWLNGKEYKCKVSNKALPAPIEKTISKAKGQPREPQVYTLPPSRDELTKNQVSLTCLVKGFYPSDIAVEWESNGQPENNYKTTPPVLDSDGSFFLYSKLTVDKSRWQQGNVFSCSVMHEALHNHYTQKSLSLSPG

SEQ ID NO: 223 - protein, 345 aa, synthetic construct
ETRECIYYNANWEEERTNQSGLERCEGEQDKRYHCYASWRNSSGTIELVKKGCWLDDFNCYDRQECVATEENPQVYFCCCEGNFCNERFTHLPEAGGPEVTYEPPPTGGGGSGGGGSGGGGTHTCPPCPAPELLGGPSVFLFPPKPKDTLMISRTPEVTCVVVDVSHEDPEVKFNWYVDGVEVHNAKTKPREEQYNSTYRVVSVLTVLHQDWLNGKEYKCKVSNKALPAPIEKTISKAKGQPREPQVYTLPPSRDELTKNQVSLTCLVKGFYPSDIAVEWESNGQPENNYKTTPPVLDSDGSFFLYSKLTVDKSRWQQGNVFSCSVMHEALHNHYTQKSLSLSPG

SEQ ID NO: 224 - protein, 345 aa, synthetic construct
ETRECIYYNANWEHERTNQSGLERCEGEQDKRYHCYASWRNSSGTIELVKKGCWLDDFNCYDRQECVATEENPQVYFCCCEGNFCNERFTHLPEAGGPEVTYEPPPTGGGGSGGGGSGGGGTHTCPPCPAPELLGGPSVFLFPPKPKDTLMISRTPEVTCVVVDVSHEDPEVKFNWYVDGVEVHNAKTKPREEQYNSTYRVVSVLTVLHQDWLNGKEYKCKVSNKALPAPIEKTISKAKGQPREPQVYTLPPSRDELTKNQVSLTCLVKGFYPSDIAVEWESNGQPENNYKTTPPVLDSDGSFFLYSKLTVDKSRWQQGNVFSCSVMHEALHNHYTQKSLSLSPG

SEQ ID NO: 225 - protein, 345 aa, synthetic construct
ETRECIYYNANWESERTNQSGLERCEGEQDKRYHCYASWRNSSGTIELVKKGCWLDDFNCYDRQECVATEENPQVYFCCCEGNFCNERFTHLPEAGGPEVTYEPPPTGGGGSGGGGSGGGGTHTCPPCPAPELLGGPSVFLFPPKPKDTLMISRTPEVTCVVVDVSHEDPEVKFNWYVDGVEVHNAKTKPREEQYNSTYRVVSVLTVLHQDWLNGKEYKCKVSNKALPAPIEKTISKAKGQPREPQVYTLPPSRDELTKNQVSLTCLVKGFYPSDIAVEWESNGQPENNYKTTPPVLDSDGSFFLYSKLTVDKSRWQQGNVFSCSVMHEALHNHYTQKSLSLSPG

SEQ ID NO: 226 - protein, 345 aa, synthetic construct
ETRECIYYNANWELERTNQSGLERCEGEQDKRYHCYASWRNSSGTIELVKKGCWYDDFNCYDRQECVATEENPQVYFCCCEGNFCNERFTHLPEAGGPEVTYEPPPTGGGGSGGGGSGGGGTHTCPPCPAPELLGGPSVFLFPPKPKDTLMISRTPEVTCVVVDVSHEDPEVKFNWYVDGVEVHNAKTKPREEQYNSTYRVVSVLTVLHQDWLNGKEYKCKVSNKALPAPIEKTISKAKGQPREPQVYTLPPSRDELTKNQVSLTCLVKGFYPSDIAVEWESNGQPENNYKTTPPVLDSDGSFFLYSKLTVDKSRWQQGNVFSCSVMHEALHNHYTQKSLSLSPG

SEQ ID NO: 227 - protein, 345 aa, synthetic construct
ETRECIYYNANWELERTNQSGLERCEGEQDKRYHCYASWRNSSGTIELVKKGCWQDDFNCYDRQECVATEENPQVYFCCCEGNFCNERFTHLPEAGGPEVTYEPPPTGGGGSGGGGSGGGGTHTCPPCPAPELLGGPSVFLFPPKPKDTLMISRTPEVTCVVVDVSHEDPEVKFNWYVDGVEVHNAKTKPREEQYNSTYRVVSVLTVLHQDWLNGKEYKCKVSNKALPAPIEKTISKAKGQPREPQVYTLPPSRDELTKNQVSLTCLVKGFYPSDIAVEWESNGQPENNYKTTPPVLDSDGSFFLYSKLTVDKSRWQQGNVFSCSVMHEALHNHYTQKSLSLSPG

SEQ ID NO: 228 - protein, 345 aa, synthetic construct
ETRECIYYNANWELERTNQSGLERCEGEQDKRYHCYASWRNSSGTIELVKKGCWMDDFNCYDRQECVATEENPQVYFCCCEGNFCNERFTHLPEAGGPEVTYEPPPTGGGGSGGGGSGGGGTHTCPPCPAPELLGGPSVFLFPPKPKDTLMISRTPEVTCVVVDVSHEDPEVKFNWYVDGVEVHNAKTKPREEQYNSTYRVVSVLTVLHQDWLNGKEYKCKVSNKALPAPIEKTISKAKGQPREPQVYTLPPSRDELTKNQVSLTCLVKGFYPSDIAVEWESNGQPENNYKTTPPVLDSDGSFFLYSKLTVDKSRWQQGNVFSCSVMHEALHNHYTQKSLSLSPG

SEQ ID NO: 229 - protein, 345 aa, synthetic construct
ETRECIYYNANWELERTNQSGLERCEGEQDKRYHCYASWRNSSGTIELVKKGCWIDDFNCYDRQECVATEENPQVYFCCCEGNFCNERFTHLPEAGGPEVTYEPPPTGGGGSGGGGSGGGGTHTCPPCPAPELLGGPSVFLFPPKPKDTLMISRTPEVTCVVVDVSHEDPEVKFNWYVDGVEVHNAKTKPREEQYNSTYRVVSVLTVLHQDWLNGKEYKCKVSNKALPAPIEKTISKAKGQPREPQVYTLPPSRDELTKNQVSLTCLVKGFYPSDIAVEWESNGQPENNYKTTPPVLDSDGSFFLYSKLTVDKSRWQQGNVFSCSVMHEALHNHYTQKSLSLSPG

SEQ ID NO: 230 - protein, 345 aa, synthetic construct
ETRECIYYNANWELERTNQSGLERCEGEQDKRWHCYASWRNSSGTIELVKKGCWLDDFNCYDRQECVATEENPQVYFCCCEGNFCNERFTHLPEAGGPEVTYEPPPTGGGGSGGGGSGGGGTHTCPPCPAPELLGGPSVFLFPPKPKDTLYISRTPEVTCVVVDVSHEDPEVKFNWYVDGVEVHNAKTKPREEQYNSTYRVVSVLTVLHQDWLNGKEYKCKVSNKALPAPIEKTISKAKGQPREPQVYTLPPSRDELTKNQVSLTCLVKGFYPSDIAVEWESNGQPENNYKTTPPVLDSDGSFFLYSKLTVDKSRWQQGNVFSCSVMHEALHNHYTQKSLSLSPG

SEQ ID NO: 231 - protein, 345 aa, synthetic construct
ETRECIYYNANWELERTNQSGLERCEGEQDKRWHCYASWRNSSGTIELVKKGCWLDDFNCYDRQECVATEENPQVYFCCCEGNFCNERFTHLPEAGGPEVTYEPPPTGGGGSGGGGSGGGGTHTCPPCPAPELLGGPSVFLFPPKPKDTLYITREPEVTCVVVDVSHEDPEVKFNWYVDGVEVHNAKTKPREEQYNSTYRVVSVLTVLHQDWLNGKEYKCKVSNKALPAPIEKTISKAKGQPREPQVYTLPPSRDELTKNQVSLTCLVKGFYPSDIAVEWESNGQPENNYKTTPPVLDSDGSFFLYSKLTVDKSRWQQGNVFSCSVMHEALHNHYTQKSLSLSPG

SEQ ID NO: 232 - protein, 350 aa, synthetic construct
ETRECIYYNANWELERTNQSGLERCEGEQDKRWHCYASWRNSSGTIELVKKGCWLDDFNCYDRQECVATEENPQVYFCCCEGNFCNERFTHLPEAGGPEVTYEPPPTGGGGSGGGGSGGGGSGGGGTHTCPPCPAPELLGGPSVFLFPPKPKDTLMISRTPEVTCVVVDVSHEDPEVKFNWYVDGVEVHNAKTKPREEQYNSTYRVVSVLTVLHQDWLNGKEYKCKVSNKALPAPIEKTISKAKGQPREPQVYTLPPSRDELTKNQVSLTCLVKGFYPSDIAVEWESNGQPENNYKTTPPVLDSDGSFFLYSKLTVDKSRWQQGNVFSCSVMHEALHNHYTQKSLSLSPG

SEQ ID NO: 233 - protein, 350 aa, synthetic construct
ETRECIYYNANWELERTNQSGLERCEGEQDKRWHCYASWRNSSGTIELVKKGCWLDDFNCYDRQECVATEENPQVYFCCCEGNFCNERFTHLPEAGGPEVTYEPPPTGGGGSGGGGSGGGGSGGGGTHTCPPCPAPELLGGPSVFLFPPKPKDTLYISRTPEVTCVVVDVSHEDPEVKFNWYVDGVEVHNAKTKPREEQYNSTYRVVSVLTVLHQDWLNGKEYKCKVSNKALPAPIEKTISKAKGQPREPQVYTLPPSRDELTKNQVSLTCLVKGFYPSDIAVEWESNGQPENNYKTTPPVLDSDGSFFLYSKLTVDKSRWQQGNVFSCSVMHEALHNHYTQKSLSLSPG

SEQ ID NO: 234 - protein, 350 aa, synthetic construct
ETRECIYYNANWELERTNQSGLERCEGEQDKRWHCYASWRNSSGTIELVKKGCWLDDFNCYDRQECVATEENPQVYFCCCEGNFCNERFTHLPEAGGPEVTYEPPPTGGGGSGGGGSGGGGSGGGGTHTCPPCPAPELLGGPSVFLFPPKPKDTLYITREPEVTCVVVDVSHEDPEVKFNWYVDGVEVHNAKTKPREEQYNSTYRVVSVLTVLHQDWLNGKEYKCKVSNKALPAPIEKTISKAKGQPREPQVYTLPPSRDELTKNQVSLTCLVKGFYPSDIAVEWESNGQPENNYKTTPPVLDSDGSFFLYSKLTVDKSRWQQGNVFSCSVMHEALHNHYTQKSLSLSPG

SEQ ID NO: 235 - protein, 350 aa, synthetic construct
ETRECIYYNANWELERTNQSGLERCEDEQDKRWHCYASWRNSSGTIELVKKGCWLDDFNCYDRQECVATEENPQVYFCCCEGNFCNERFTHLPEAGGPEVTYEPPPTGGGGSGGGGSGGGGSGGGGTHTCPPCPAPELLGGPSVFLFPPKPKDTLMISRTPEVTCVVVDVSHEDPEVKFNWYVDGVEVHNAKTKPREEQYNSTYRVVSVLTVLHQDWLNGKEYKCKVSNKALPAPIEKTISKAKGQPREPQVYTLPPSRDELTKNQVSLTCLVKGFYPSDIAVEWESNGQPENNYKTTPPVLDSDGSFFLYSKLTVDKSRWQQGNVFSCSVMHEALHNHYTQKSLSLSPG

SEQ ID NO: 236 - protein, 350 aa, synthetic construct
ETRECIYYNANWELERTNQSGLERCEEEQDKRWHCYASWRNSSGTIELVKKGCWLDDFNCYDRQECVATEENPQVYFCCCEGNFCNERFTHLPEAGGPEVTYEPPPTGGGGSGGGGSGGGGSGGGGTHTCPPCPAPELLGGPSVFLFPPKPKDTLMISRTPEVTCVVVDVSHEDPEVKFNWYVDGVEVHNAKTKPREEQYNSTYRVVSVLTVLHQDWLNGKEYKCKVSNKALPAPIEKTISKAKGQPREPQVYTLPPSRDELTKNQVSLTCLVKGFYPSDIAVEWESNGQPENNYKTTPPVLDSDGSFFLYSKLTVDKSRWQQGNVFSCSVMHEALHNHYTQKSLSLSPG

SEQ ID NO: 237 - protein, 350 aa, synthetic construct
ETRECIYYNANWELERTNQSGLERCENEQDKRWHCYASWRNSSGTIELVKKGCWLDDFNCYDRQECVATEENPQVYFCCCEGNFCNERFTHLPEAGGPEVTYEPPPTGGGGSGGGGSGGGGSGGGGTHTCPPCPAPELLGGPSVFLFPPKPKDTLMISRTPEVTCVVVDVSHEDPEVKFNWYVDGVEVHNAKTKPREEQYNSTYRVVSVLTVLHQDWLNGKEYKCKVSNKALPAPIEKTISKAKGQPREPQVYTLPPSRDELTKNQVSLTCLVKGFYPSDIAVEWESNGQPENNYKTTPPVLDSDGSFFLYSKLTVDKSRWQQGNVFSCSVMHEALHNHYTQKSLSLSPG

SEQ ID NO: 238 - protein, 350 aa, synthetic construct
ETRECIYYNANWELERTNQSGLERCEQEQDKRWHCYASWRNSSGTIELVKKGCWLDDFNCYDRQECVATEENPQVYFCCCEGNFCNERFTHLPEAGGPEVTYEPPPTGGGGSGGGGSGGGGSGGGGTHTCPPCPAPELLGGPSVFLFPPKPKDTLMISRTPEVTCVVVDVSHEDPEVKFNWYVDGVEVHNAKTKPREEQYNSTYRVVSVLTVLHQDWLNGKEYKCKVSNKALPAPIEKTISKAKGQPREPQVYTLPPSRDELTKNQVSLTCLVKGFYPSDIAVEWESNGQPENNYKTTPPVLDSDGSFFLYSKLTVDKSRWQQGNVFSCSVMHEALHNHYTQKSLSLSPG

SEQ ID NO: 239 - protein, 350 aa, synthetic construct
ETRECIYYNANWELERTNQSGLERCETEQDKRWHCYASWRNSSGTIELVKKGCWLDDFNCYDRQECVATEENPQVYFCCCEGNFCNERFTHLPEAGGPEVTYEPPPTGGGGSGGGGSGGGGSGGGGTHTCPPCPAPELLGGPSVFLFPPKPKDTLMISRTPEVTCVVVDVSHEDPEVKFNWYVDGVEVHNAKTKPREEQYNSTYRVVSVLTVLHQDWLNGKEYKCKVSNKALPAPIEKTISKAKGQPREPQVYTLPPSRDELTKNQVSLTCLVKGFYPSDIAVEWESNGQPENNYKTTPPVLDSDGSFFLYSKLTVDKSRWQQGNVFSCSVMHEALHNHYTQKSLSLSPG

SEQ ID NO: 240 - protein, 350 aa, synthetic construct
ETRECIYYNANWELERTNQSGLERCEMEQDKRWHCYASWRNSSGTIELVKKGCWLDDFNCYDRQECVATEENPQVYFCCCEGNFCNERFTHLPEAGGPEVTYEPPPTGGGGSGGGGSGGGGSGGGGTHTCPPCPAPELLGGPSVFLFPPKPKDTLMISRTPEVTCVVVDVSHEDPEVKFNWYVDGVEVHNAKTKPREEQYNSTYRVVSVLTVLHQDWLNGKEYKCKVSNKALPAPIEKTISKAKGQPREPQVYTLPPSRDELTKNQVSLTCLVKGFYPSDIAVEWESNGQPENNYKTTPPVLDSDGSFFLYSKLTVDKSRWQQGNVFSCSVMHEALHNHYTQKSLSLSPG

SEQ ID NO: 241 - protein, 350 aa, synthetic construct
ETRECIYYNANWELERTNQSGLERCEDEQDKRYHCYASWRNSSGTIELVKKGCWLDDFNCYDRQECVATEENPQVYFCCCEGNFCNERFTHLPEAGGPEVTYEPPPTGGGGSGGGGSGGGGSGGGGTHTCPPCPAPELLGGPSVFLFPPKPKDTLMISRTPEVTCVVVDVSHEDPEVKFNWYVDGVEVHNAKTKPREEQYNSTYRVVSVLTVLHQDWLNGKEYKCKVSNKALPAPIEKTISKAKGQPREPQVYTLPPSRDELTKNQVSLTCLVKGFYPSDIAVEWESNGQPENNYKTTPPVLDSDGSFFLYSKLTVDKSRWQQGNVFSCSVMHEALHNHYTQKSLSLSPG

SEQ ID NO: 242 - protein, 350 aa, synthetic construct
ETRECIYYNANWELERTNQSGLERCEEEQDKRYHCYASWRNSSGTIELVKKGCWLDDFNCYDRQECVATEENPQVYFCCCEGNFCNERFTHLPEAGGPEVTYEPPPTGGGGSGGGGSGGGGSGGGGTHTCPPCPAPELLGGPSVFLFPPKPKDTLMISRTPEVTCVVVDVSHEDPEVKFNWYVDGVEVHNAKTKPREEQYNSTYRVVSVLTVLHQDWLNGKEYKCKVSNKALPAPIEKTISKAKGQPREPQVYTLPPSRDELTKNQVSLTCLVKGFYPSDIAVEWESNGQPENNYKTTPPVLDSDGSFFLYSKLTVDKSRWQQGNVFSCSVMHEALHNHYTQKSLSLSPG

SEQ ID NO: 243 - protein, 350 aa, synthetic construct
ETRECIYYNANWELERTNQSGLERCENEQDKRYHCYASWRNSSGTIELVKKGCWLDDFNCYDRQECVATEENPQVYFCCCEGNFCNERFTHLPEAGGPEVTYEPPPTGGGGSGGGGSGGGGSGGGGTHTCPPCPAPELLGGPSVFLFPPKPKDTLMISRTPEVTCVVVDVSHEDPEVKFNWYVDGVEVHNAKTKPREEQYNSTYRVVSVLTVLHQDWLNGKEYKCKVSNKALPAPIEKTISKAKGQPREPQVYTLPPSRDELTKNQVSLTCLVKGFYPSDIAVEWESNGQPENNYKTTPPVLDSDGSFFLYSKLTVDKSRWQQGNVFSCSVMHEALHNHYTQKSLSLSPG

SEQ ID NO: 244 - protein, 350 aa, synthetic construct
ETRECIYYNANWELERTNQSGLERCEQEQDKRYHCYASWRNSSGTIELVKKGCWLDDFNCYDRQECVATEENPQVYFCCCEGNFCNERFTHLPEAGGPEVTYEPPPTGGGGSGGGGSGGGGSGGGGTHTCPPCPAPELLGGPSVFLFPPKPKDTLMISRTPEVTCVVVDVSHEDPEVKFNWYVDGVEVHNAKTKPREEQYNSTYRVVSVLTVLHQDWLNGKEYKCKVSNKALPAPIEKTISKAKGQPREPQVYTLPPSRDELTKNQVSLTCLVKGFYPSDIAVEWESNGQPENNYKTTPPVLDSDGSFFLYSKLTVDKSRWQQGNVFSCSVMHEALHNHYTQKSLSLSPG

SEQ ID NO: 245 - protein, 350 aa, synthetic construct
ETRECIYYNANWEEERTNQSGLERCEGEQDKRWHCYASWRNSSGTIELVKKGCWLDDFNCYDRQECVATEENPQVYFCCCEGNFCNERFTHLPEAGGPEVTYEPPPTGGGGSGGGGSGGGGSGGGGTHTCPPCPAPELLGGPSVFLFPPKPKDTLMISRTPEVTCVVVDVSHEDPEVKFNWYVDGVEVHNAKTKPREEQYNSTYRVVSVLTVLHQDWLNGKEYKCKVSNKALPAPIEKTISKAKGQPREPQVYTLPPSRDELTKNQVSLTCLVKGFYPSDIAVEWESNGQPENNYKTTPPVLDSDGSFFLYSKLTVDKSRWQQGNVFSCSVMHEALHNHYTQKSLSLSPG

SEQ ID NO: 246 - protein, 350 aa, synthetic construct
ETRECIYYNANWEDERTNQSGLERCEGEQDKRWHCYASWRNSSGTIELVKKGCWLDDFNCYDRQECVATEENPQVYFCCCEGNFCNERFTHLPEAGGPEVTYEPPPTGGGGSGGGGSGGGGSGGGGTHTCPPCPAPELLGGPSVFLFPPKPKDTLMISRTPEVTCVVVDVSHEDPEVKFNWYVDGVEVHNAKTKPREEQYNSTYRVVSVLTVLHQDWLNGKEYKCKVSNKALPAPIEKTISKAKGQPREPQVYTLPPSRDELTKNQVSLTCLVKGFYPSDIAVEWESNGQPENNYKTTPPVLDSDGSFFLYSKLTVDKSRWQQGNVFSCSVMHEALHNHYTQKSLSLSPG

SEQ ID NO: 247 - protein, 350 aa, synthetic construct
ETRECIYYNANWENERTNQSGLERCEGEQDKRWHCYASWRNSSGTIELVKKGCWLDDFNCYDRQECVATEENPQVYFCCCEGNFCNERFTHLPEAGGPEVTYEPPPTGGGGSGGGGSGGGGSGGGGTHTCPPCPAPELLGGPSVFLFPPKPKDTLMISRTPEVTCVVVDVSHEDPEVKFNWYVDGVEVHNAKTKPREEQYNSTYRVVSVLTVLHQDWLNGKEYKCKVSNKALPAPIEKTISKAKGQPREPQVYTLPPSRDELTKNQVSLTCLVKGFYPSDIAVEWESNGQPENNYKTTPPVLDSDGSFFLYSKLTVDKSRWQQGNVFSCSVMHEALHNHYTQKSLSLSPG

SEQ ID NO: 248 - protein, 350 aa, synthetic construct
ETRECIYYNANWEQERTNQSGLERCEGEQDKRWHCYASWRNSSGTIELVKKGCWLDDFNCYDRQECVATEENPQVYFCCCEGNFCNERFTHLPEAGGPEVTYEPPPTGGGGSGGGGSGGGGSGGGGTHTCPPCPAPELLGGPSVFLFPPKPKDTLMISRTPEVTCVVVDVSHEDPEVKFNWYVDGVEVHNAKTKPREEQYNSTYRVVSVLTVLHQDWLNGKEYKCKVSNKALPAPIEKTISKAKGQPREPQVYTLPPSRDELTKNQVSLTCLVKGFYPSDIAVEWESNGQPENNYKTTPPVLDSDGSFFLYSKLTVDKSRWQQGNVFSCSVMHEALHNHYTQKSLSLSPG

SEQ ID NO: 249 - protein, 350 aa, synthetic construct
ETRECIYYNANWEQERTNQSGLERCEGEQDKRYHCYASWRNSSGTIELVKKGCWLDDFNCYDRQECVATEENPQVYFCCCEGNFCNERFTHLPEAGGPEVTYEPPPTGGGGSGGGGSGGGGSGGGGTHTCPPCPAPELLGGPSVFLFPPKPKDTLMISRTPEVTCVVVDVSHEDPEVKFNWYVDGVEVHNAKTKPREEQYNSTYRVVSVLTVLHQDWLNGKEYKCKVSNKALPAPIEKTISKAKGQPREPQVYTLPPSRDELTKNQVSLTCLVKGFYPSDIAVEWESNGQPENNYKTTPPVLDSDGSFFLYSKLTVDKSRWQQGNVFSCSVMHEALHNHYTQKSLSLSPG

SEQ ID NO: 250 - protein, 350 aa, synthetic construct
ETRECIYYNANWEDERTNQSGLERCEGEQDKRYHCYASWRNSSGTIELVKKGCWLDDFNCYDRQECVATEENPQVYFCCCEGNFCNERFTHLPEAGGPEVTYEPPPTGGGGSGGGGSGGGGSGGGGTHTCPPCPAPELLGGPSVFLFPPKPKDTLMISRTPEVTCVVVDVSHEDPEVKFNWYVDGVEVHNAKTKPREEQYNSTYRVVSVLTVLHQDWLNGKEYKCKVSNKALPAPIEKTISKAKGQPREPQVYTLPPSRDELTKNQVSLTCLVKGFYPSDIAVEWESNGQPENNYKTTPPVLDSDGSFFLYSKLTVDKSRWQQGNVFSCSVMHEALHNHYTQKSLSLSPG

SEQ ID NO: 251 - protein, 350 aa, synthetic construct
ETRECIYYNANWENERTNQSGLERCEGEQDKRYHCYASWRNSSGTIELVKKGCWLDDFNCYDRQECVATEENPQVYFCCCEGNFCNERFTHLPEAGGPEVTYEPPPTGGGGSGGGGSGGGGSGGGGTHTCPPCPAPELLGGPSVFLFPPKPKDTLMISRTPEVTCVVVDVSHEDPEVKFNWYVDGVEVHNAKTKPREEQYNSTYRVVSVLTVLHQDWLNGKEYKCKVSNKALPAPIEKTISKAKGQPREPQVYTLPPSRDELTKNQVSLTCLVKGFYPSDIAVEWESNGQPENNYKTTPPVLDSDGSFFLYSKLTVDKSRWQQGNVFSCSVMHEALHNHYTQKSLSLSPG

SEQ ID NO: 252 - protein, 224 aa, Homo sapiens
THTCPPCPAPELLGGPSVFLFPPKPKDTLMISRTPEVTCVVVDVSHEDPEVKFNWYVDGVEVHNAKTKPREEQYNSTYRVVSVLTVLHQDWLNGKEYKCKVSNKALPAPIEKTISKAKGQPREPQVYTLPPSREEMTKNQVSLTCLVKGFYPSDIAVEWESNGQPENNYKTTPPVLDSDGSFFLYSKLTVDKSRWQQGNVFSCSVMHEALHNHYTQKSLSLSPG

SEQ ID NO: 253 - protein, 224 aa, Homo sapiens
THTCPPCPAPELLGGPSVFLFPPKPKDTLMISRTPEVTCVVVDVSHEDPEVKFNWYVDGVEVHNAKTKPREEQYNSTYRVVSVLTVLHQDWLNGKEYKCKVSNKALPAPIEKTISKAKGQPREPQVYTLPPSRDELTKNQVSLTCLVKGFYPSDIAVEWESNGQPENNYKTTPPVLDSDGSFFLYSKLTVDKSRWQQGNVFSCSVMHEALHNHYTQKSLSLSPG

SEQ ID NO: 254 - protein, 224 aa, Homo sapiens
THTCPPCPAPELLGGPSVFLFPPKPKDTLYITREPEVTCVVVDVSHEDPEVKFNWYVDGVEVHNAKTKPREEQYNSTYRVVSVLTVLHQDWLNGKEYKCKVSNKALPAPIEKTISKAKGQPREPQVYTLPPSREEMTKNQVSLTCLVKGFYPSDIAVEWESNGQPENNYKTTPPVLDSDGSFFLYSKLTVDKSRWQQGNVFSCSVMHEALHNHYTQKSLSLSPG

SEQ ID NO: 255 - protein, 224 aa, Homo sapiens
THTCPPCPAPELLGGPSVFLFPPKPKDTLYITREPEVTCVVVDVSHEDPEVKFNWYVDGVEVHNAKTKPREEQYNSTYRVVSVLTVLHQDWLNGKEYKCKVSNKALPAPIEKTISKAKGQPREPQVYTLPPSRDELTKNQVSLTCLVKGFYPSDIAVEWESNGQPENNYKTTPPVLDSDGSFFLYSKLTVDKSRWQQGNVFSCSVMHEALHNHYTQKSLSLSPG

SEQ ID NO: 256 - protein, 224 aa, Homo sapiens
THTCPPCPAPELLGGPSVFLFPPKPKDTLYISRTPEVTCVVVDVSHEDPEVKFNWYVDGVEVHNAKTKPREEQYNSTYRVVSVLTVLHQDWLNGKEYKCKVSNKALPAPIEKTISKAKGQPREPQVYTLPPSRDELTKNQVSLTCLVKGFYPSDIAVEWESNGQPENNYKTTPPVLDSDGSFFLYSKLTVDKSRWQQGNVFSCSVMHEALHNHYTQKSLSLSPG

SEQ ID NO: 257 - protein, 224 aa, Homo sapiens
THTCPPCPAPELLGGPSVFLFPPKPKDTLYISRTPEVTCVVVDVSHEDPEVKFNWYVDGVEVHNAKTKPREEQYNSTYRVVSVLTVLHQDWLNGKEYKCKVSNKALPAPIEKTISKAKGQPREPQVYTLPPSREEMTKNQVSLTCLVKGFYPSDIAVEWESNGQPENNYKTTPPVLDSDGSFFLYSKLTVDKSRWQQGNVFSCSVMHEALHNHYTQKSLSLSPG

SEQ ID NO: 258 - protein, 217 aa, Homo sapiens
APELLGGPSVFLFPPKPKDTLMISRTPEVTCVVVDVSHEDPEVKFNWYVDGVEVHNAKTKPREEQYNSTYRVVSVLTVLHQDWLNGKEYKCKVSNKALPAPIEKTISKAKGQPREPQVYTLPPSRDELTKNQVSLTCLVKGFYPSDIAVEWESNGQPENNYKTTPPVLDSDGSFFLYSKLTVDKSRWQQGNVFSCSVMHEALHNHYTQKSLSLSPGK

SEQ ID NO: 259 - protein, 216 aa, Homo sapiens
APELLGGPSVFLFPPKPKDTLMISRTPEVTCVVVDVSHEDPEVKFNWYVDGVEVHNAKTKPREEQYNSTYRVVSVLTVLHQDWLNGKEYKCKVSNKALPAPIEKTISKAKGQPREPQVYTLPPSRDELTKNQVSLTCLVKGFYPSDIAVEWESNGQPENNYKTTPPVLDSDGSFFLYSKLTVDKSRWQQGNVFSCSVMHEALHNHYTQKSLSLSPG

SEQ ID NO: 260 - protein, 220 aa, Homo sapiens
PPCPAPELLGGPSVFLFPPKPKDTLMISRTPEVTCVVVDVSHEDPEVKFNWYVDGVEVHNAKTKPREEQYNSTYRVVSVLTVLHQDWLNGKEYKCKVSNKALPAPIEKTISKAKGQPREPQVYTLPPSRDELTKNQVSLTCLVKGFYPSDIAVEWESNGQPENNYKTTPPVLDSDGSFFLYSKLTVDKSRWQQGNVFSCSVMHEALHNHYTQKSLSLSPG

SEQ ID NO: 261 - protein, 226 aa, Homo sapiens
DKTHTCPPCPAPELLGGPSVFLFPPKPKDTLMISRTPEVTCVVVDVSHEDPEVKFNWYVDGVEVHNAKTKPREEQYNSTYRVVSVLTVLHQDWLNGKEYKCKVSNKALPAPIEKTISKAKGQPREPQVYTLPPSRDELTKNQVSLTCLVKGFYPSDIAVEWESNGQPENNYKTTPPVLDSDGSFFLYSKLTVDKSRWQQGNVFSCSVMHEALHNHYTQKSLSLSPG

SEQ ID NO: 262 - protein, 231 aa, Homo sapiens
EPKSSDKTHTCPPCPAPELLGGPSVFLFPPKPKDTLMISRTPEVTCVVVDVSHEDPEVKFNWYVDGVEVHNAKTKPREEQYNSTYRVVSVLTVLHQDWLNGKEYKCKVSNKALPAPIEKTISKAKGQPREPQVYTLPPSRDELTKNQVSLTCLVKGFYPSDIAVEWESNGQPENNYKTTPPVLDSDGSFFLYSKLTVDKSRWQQGNVFSCSVMHEALHNHYTQKSLSLSPG

SEQ ID NO: 263 - protein, 231 aa, Homo sapiens
EPKSSDKTHTSPPSPAPELLGGPSVFLFPPKPKDTLMISRTPEVTCVVVDVSHEDPEVKFNWYVDGVEVHNAKTKPREEQYNSTYRVVSVLTVLHQDWLNGKEYKCKVSNKALPAPIEKTISKAKGQPREPQVYTLPPSRDELTKNQVSLTCLVKGFYPSDIAVEWESNGQPENNYKTTPPVLDSDGSFFLYSKLTVDKSRWQQGNVFSCSVMHEALHNHYTQKSLSLSPG

SEQ ID NO: 264 - protein, 224 aa, Homo sapiens; identical to SEQ ID NO: 257

SEQ ID NO: 265 - protein, 224 aa, Homo sapiens
THTCPPCPAPELLGGPSVFLFPPKPKDTLMISRTPEVTCVVVDVSHEDPEVKFNWYVDGVEVHNAKTKPREEQYNSTYRVVSVLTVLHQDWLNGKEYKCKVSNKALPVPIEKTISKAKGQPREPQVYTLPPSRDELTKNQVSLTCLVKGFYPSDIAVEWESNGQPENNYKTTPPVLDSDGSFFLYSKLTVDKSRWQQGNVFSCSVMHEALHNHYTQKSLSLSPG

SEQ ID NO: 266 - protein, 224 aa, Homo sapiens
THTCPPCPAPELLGGPSVFLFPPKPKDTLMISRTPEVTCVVVDVSHEDPEVKFNWYVDGVEVHNAKTKPREEQYNSTYRVVSVLTVLHQDWLNGKEYKCKVSNKALPVPIEKTISKAKGQPREPQVYTLPPSREEMTKNQVSLTCLVKGFYPSDIAVEWESNGQPENNYKTTPPVLDSDGSFFLYSKLTVDKSRWQQGNVFSCSVMHEALHNHYTQKSLSLSPG

SEQ ID NO: 267 - protein, 216 aa, Homo sapiens
APPVAGPSVFLFPPKPKDTLMISRTPEVTCVVVDVSHEDPEVQFNWYVDGVEVHNAKTKPREEQFNSTFRVVSVLTVVHQDWLNGKEYKCKVSNKGLPAPIEKTISKTKGQPREPQVYTLPPSREEMTKNQVSLTCLVKGFYPSDISVEWESNGQPENNYKTTPPMLDSDGSFFLYSKLTVDKSRWQQGNVFSCSVMHEALHNHYTQKSLSLSPGK

SEQ ID NO: 268 - protein, 223 aa, Homo sapiens
VECPPCPAPPVAGPSVFLFPPKPKDTLMISRTPEVTCVVVDVSHEDPEVQFNWYVDGVEVHNAKTKPREEQFNSTFRVVSVLTVVHQDWLNGKEYKCKVSNKGLPAPIEKTISKTKGQPREPQVYTLPPSREEMTKNQVSLTCLVKGFYPSDIAVEWESNGQPENNYKTTPPMLDSDGSFFLYSKLTVDKSRWQQGNVFSCSVMHEALHNHYTQKSLSLSPGK

SEQ ID NO: 269 - protein, 228 aa, Homo sapiens
ERKCCVECPPCPAPPVAGPSVFLFPPKPKDTLMISRTPEVTCVVVDVSHEDPEVQFNWYVDGVEVHNAKTKPREEQFNSTFRVVSVLTVVHQDWLNGKEYKCKVSNKGLPAPIEKTISKTKGQPREPQVYTLPPSREEMTKNQVSLTCLVKGFYPSDISVEWESNGQPENNYKTTPPMLDSDGSFFLYSKLTVDKSRWQQGNVFSCSVMHEALHNHYTQKSLSLSPGK

SEQ ID NO: 270 - protein, 227 aa, Homo sapiens
ERKSSVECPPCPAPPVAGPSVFLFPPKPKDTLMISRTPEVTCVVVDVSHEDPEVQFNWYVDGVEVHNAKTKPREEQFNSTFRVVSVLTVVHQDWLNGKEYKCKVSNKGLPAPIEKTISKTKGQPREPQVYTLPPSREEMTKNQVSLTCLVKGFYPSDISVEWESNGQPENNYKTTPPMLDSDGSFFLYSKLTVDKSRWQQGNVFSCSVMHEALHNHYTQKSLSLSPG

SEQ ID NO: 271 - protein, 227 aa, Homo sapiens
ERKSSVESPPCPAPPVAGPSVFLFPPKPKDTLMISRTPEVTCVVVDVSHEDPEVQFNWYVDGVEVHNAKTKPREEQFNSTFRVVSVLTVVHQDWLNGKEYKCKVSNKGLPAPIEKTISKTKGQPREPQVYTLPPSREEMTKNQVSLTCLVKGFYPSDISVEWESNGQPENNYKTTPPMLDSDGSFFLYSKLTVDKSRWQQGNVFSCSVMHEALHNHYTQKSLSLSPG

SEQ ID NO: 272 - protein, 227 aa, Homo sapiens
ERKSSVESPPSPAPPVAGPSVFLFPPKPKDTLMISRTPEVTCVVVDVSHEDPEVQFNWYVDGVEVHNAKTKPREEQFNSTFRVVSVLTVVHQDWLNGKEYKCKVSNKGLPAPIEKTISKTKGQPREPQVYTLPPSREEMTKNQVSLTCLVKGFYPSDISVEWESNGQPENNYKTTPPMLDSDGSFFLYSKLTVDKSRWQQGNVFSCSVMHEALHNHYTQKSLSLSPG

SEQ ID NO: 273 - protein, 215 aa, Homo sapiens
APPVAGPSVFLFPPKPKDTLMISRTPEVTCVVVDVSHEDPEVQFNWYVDGVEVHNAKTKPREEQFNSTFRVVSVLTVVHQDWLNGKEYKCKVSNKGLPAPIEKTISKTKGQPREPQVYTLPPSREEMTKNQVSLTCLVKGFYPSDISVEWESNGQPENNYKTTPPMLDSDGSFFLYSKLTVDKSRWQQGNVFSCSVMHEALHNHYTQKSLSLSPG

SEQ ID NO: 274 - protein, 219 aa, Homo sapiens
PPCPAPPVAGPSVFLFPPKPKDTLMISRTPEVTCVVVDVSHEDPEVQFNWYVDGVEVHNAKTKPREEQFNSTFRVVSVLTVVHQDWLNGKEYKCKVSNKGLPAPIEKTISKTKGQPREPQVYTLPPSREEMTKNQVSLTCLVKGFYPSDISVEWESNGQPENNYKTTPPMLDSDGSFFLYSKLTVDKSRWQQGNVFSCSVMHEALHNHYTQKSLSLSPG

SEQ ID NO: 275 - protein, 222 aa, Homo sapiens
VECPPCPAPPVAGPSVFLFPPKPKDTLMISRTPEVTCVVVDVSHEDPEVQFNWYVDGVEVHNAKTKPREEQFNSTFRVVSVLTVVHQDWLNGKEYKCKVSNKGLPAPIEKTISKTKGQPREPQVYTLPPSREEMTKNQVSLTCLVKGFYPSDISVEWESNGQPENNYKTTPPMLDSDGSFFLYSKLTVDKSRWQQGNVFSCSVMHEALHNHYTQKSLSLSPG

SEQ ID NO: 276 - protein, 224 aa, Homo sapiens
PCPPCKCPAPNLLGGPSVFIFPPKIKDVLMISLSPIVTCVVVDVSEDDPDVQISWFVNNVEVHTAQTQTHREDYNSTLRVVSALPIQHQDWMSGKEFKCKVNNKDLPAPIERTISKPKGSVRAPQVYVLPPPEEEMTKKQVTLTCMVTDFMPEDIYVEWTNNGKTELNYKNTEPVLDSDGSYFMYSKLRVEKKNWVERNSYSCSVVHEGLHNHHTTKSFSRTPG

SEQ ID NO: 277 - protein, 217 aa, Homo sapiens
APELLGGPSVFLFPPKPKDTLMISRTPEVTCVVVDVSHEDPEVQFKWYVDGVEVHNAKTKPREEQYNSTFRVVSVLTVLHQDWLNGKEYKCKVSNKALPAPIEKTISKTKGQPREPQVYTLPPSREEMTKNQVSLTCLVKGFYPSDIAVEWESSGQPENNYNTTPPMLDSDGSFFLYSKLTVDKSRWQQGNIFSCSVMHEALHNRFTQKSLSLSPGK

SEQ ID NO: 278 - protein, 216 aa, Homo sapiens
APELLGGPSVFLFPPKPKDTLMISRTPEVTCVVVDVSHEDPEVQFKWYVDGVEVHNAKTKPREEQYNSTFRVVSVLTVLHQDWLNGKEYKCKVSNKALPAPIEKTISKTKGQPREPQVYTLPPSREEMTKNQVSLTCLVKGFYPSDIAVEWESSGQPENNYNTTPPMLDSDGSFFLYSKLTVDKSRWQQGNIFSCSVMHEALHNRFTQKSLSLSPG

SEQ ID NO: 279 - protein, 220 aa, Homo sapiens
PRCPAPELLGGPSVFLFPPKPKDTLMISRTPEVTCVVVDVSHEDPEVQFKWYVDGVEVHNAKTKPREEQYNSTFRVVSVLTVLHQDWLNGKEYKCKVSNKALPAPIEKTISKTKGQPREPQVYTLPPSREEMTKNQVSLTCLVKGFYPSDIAVEWESSGQPENNYNTTPPMLDSDGSFFLYSKLTVDKSRWQQGNIFSCSVMHEALHNRFTQKSLSLSPG

SEQ ID NO: 280 - protein, 226 aa, Homo sapiens
DTPPPCPRCPAPELLGGPSVFLFPPKPKDTLMISRTPEVTCVVVDVSHEDPEVQFKWYVDGVEVHNAKTKPREEQYNSTFRVVSVLTVLHQDWLNGKEYKCKVSNKALPAPIEKTISKTKGQPREPQVYTLPPSREEMTKNQVSLTCLVKGFYPSDIAVEWESSGQPENNYNTTPPMLDSDGSFFLYSKLTVDKSRWQQGNIFSCSVMHEALHNRFTQKSLSLSPG

SEQ ID NO: 281 - protein, 231 aa, Homo sapiens
EPKSSDTPPPCPRCPAPELLGGPSVFLFPPKPKDTLMISRTPEVTCVVVDVSHEDPEVQFKWYVDGVEVHNAKTKPREEQYNSTFRVVSVLTVLHQDWLNGKEYKCKVSNKALPAPIEKTISKTKGQPREPQVYTLPPSREEMTKNQVSLTCLVKGFYPSDIAVEWESSGQPENNYNTTPPMLDSDGSFFLYSKLTVDKSRWQQGNIFSCSVMHEALHNRFTQKSLSLSPG

SEQ ID NO: 282 - protein, 231 aa, Homo sapiens
EPKSSDTPPPSPRCPAPELLGGPSVFLFPPKPKDTLMISRTPEVTCVVVDVSHEDPEVQFKWYVDGVEVHNAKTKPREEQYNSTFRVVSVLTVLHQDWLNGKEYKCKVSNKALPAPIEKTISKTKGQPREPQVYTLPPSREEMTKNQVSLTCLVKGFYPSDIAVEWESSGQPENNYNTTPPMLDSDGSFFLYSKLTVDKSRWQQGNIFSCSVMHEALHNRFTQKSLSLSPG

SEQ ID NO: 283 - protein, 231 aa, Homo sapiens
EPKSSDTPPPSPRSPAPELLGGPSVFLFPPKPKDTLMISRTPEVTCVVVDVSHEDPEVQFKWYVDGVEVHNAKTKPREEQYNSTFRVVSVLTVLHQDWLNGKEYKCKVSNKALPAPIEKTISKTKGQPREPQVYTLPPSREEMTKNQVSLTCLVKGFYPSDIAVEWESSGQPENNYNTTPPMLDSDGSFFLYSKLTVDKSRWQQGNIFSCSVMHEALHNRFTQKSLSLSPG

SEQ ID NO: 284 - protein, 217 aa, Homo sapiens
APEFLGGPSVFLFPPKPKDTLMISRTPEVTCVVVDVSQEDPEVQFNWYVDGVEVHNAKTKPREEQFNSTYRVVSVLTVLHQDWLNGKEYKCKVSNKGLPSSIEKTISKAKGQPREPQVYTLPPSQEEMTKNQVSLTCLVKGFYPSDIAVEWESNGQPENNYKTTPPVLDSDGSFFLYSRLTVDKSRWQEGNVFSCSVMHEALHNHYTQKSLSLSLGK

SEQ ID NO: 285 - protein, 224 aa, Homo sapiens
GPPCPPCPAPEFLGGPSVFLFPPKPKDTLMISRTPEVTCVVVDVSQEDPEVQFNWYVDGVEVHNAKTKPREEQFNSTYRVVSVLTVLHQDWLNGKEYKCKVSNKGLPSSIEKTISKAKGQPREPQVYTLPPSQEEMTKNQVSLTCLVKGFYPSDIAVEWESNGQPENNYKTTPPVLDSDGSFFLYSRLTVDKSRWQEGNVFSCSVMHEALHNHYTQKSLSLSLG

SEQ ID NO: 286 - protein, 216 aa, Homo sapiens
APEFLGGPSVFLFPPKPKDTLMISRTPEVTCVVVDVSQEDPEVQFNWYVDGVEVHNAKTKPREEQFNSTYRVVSVLTVLHQDWLNGKEYKCKVSNKGLPSSIEKTISKAKGQPREPQVYTLPPSQEEMTKNQVSLTCLVKGFYPSDIAVEWESNGQPENNYKTTPPVLDSDGSFFLYSRLTVDKSRWQEGNVFSCSVMHEALHNHYTQKSLSLSLG

SEQ ID NO: 287 - protein, 220 aa, Homo sapiens
PSCPAPEFLGGPSVFLFPPKPKDTLMISRTPEVTCVVVDVSQEDPEVQFNWYVDGVEVHNAKTKPREEQFNSTYRVVSVLTVLHQDWLNGKEYKCKVSNKGLPSSIEKTISKAKGQPREPQVYTLPPSQEEMTKNQVSLTCLVKGFYPSDIAVEWESNGQPENNYKTTPPVLDSDGSFFLYSRLTVDKSRWQEGNVFSCSVMHEALHNHYTQKSLSLSLG

SEQ ID NO: 288 - protein, 228 aa, Homo sapiens
ESKYGPPCPSCPAPEFLGGPSVFLFPPKPKDTLMISRTPEVTCVVVDVSQEDPEVQFNWYVDGVEVHNAKTKPREEQFNSTYRVVSVLTVLHQDWLNGKEYKCKVSNKGLPSSIEKTISKAKGQPREPQVYTLPPSQEEMTKNQVSLTCLVKGFYPSDIAVEWESNGQPENNYKTTPPVLDSDGSFFLYSRLTVDKSRWQEGNVFSCSVMHEALHNHYTQKSLSLSLG

SEQ ID NO: 289 - protein, 228 aa, Homo sapiens
ESKYGPPCPPCPAPEFLGGPSVFLFPPKPKDTLMISRTPEVTCVVVDVSQEDPEVQFNWYVDGVEVHNAKTKPREEQFNSTYRVVSVLTVLHQDWLNGKEYKCKVSNKGLPSSIEKTISKAKGQPREPQVYTLPPSQEEMTKNQVSLTCLVKGFYPSDIAVEWESNGQPENNYKTTPPVLDSDGSFFLYSRLTVDKSRWQEGNVFSCSVMHEALHNHYTQKSLSLSLG

SEQ ID NO: 290 - protein, 228 aa, Homo sapiens
ESKYGPPCPPCPAPEFLGGPSVFLFPPKPKDTLMISRTPEVTCVVVDVSQEDPEVQFNWYVDGVEVHNAKTKPREEQFNSTYRVVSVLTVLHQDWLNGKEYKCKVSNKGLPSSIEKTISKAKGQPREPQVYTLPPSQEEMTKNQVSLTCLVKGFYPSDIAVEWESNGQPENNYKTTPPVLDSDGSFFLYSKLTVDKSRWQEGNVFSCSVMHEALHNHYTQKSLSLSLG

SEQ ID NO: 291 - protein, 228 aa, Homo sapiens
ESKYGPPSPSCPAPEFLGGPSVFLFPPKPKDTLMISRTPEVTCVVVDVSQEDPEVQFNWYVDGVEVHNAKTKPREEQFNSTYRVVSVLTVLHQDWLNGKEYKCKVSNKGLPSSIEKTISKAKGQPREPQVYTLPPSQEEMTKNQVSLTCLVKGFYPSDIAVEWESNGQPENNYKTTPPVLDSDGSFFLYSRLTVDKSRWQEGNVFSCSVMHEALHNHYTQKSLSLSLG

SEQ ID NO: 292 - protein, 228 aa, Homo sapiens
ESKYGPPSPSSPAPEFLGGPSVFLFPPKPKDTLMISRTPEVTCVVVDVSQEDPEVQFNWYVDGVEVHNAKTKPREEQFNSTYRVVSVLTVLHQDWLNGKEYKCKVSNKGLPSSIEKTISKAKGQPREPQVYTLPPSQEEMTKNQVSLTCLVKGFYPSDIAVEWESNGQPENNYKTTPPVLDSDGSFFLYSRLTVDKSRWQEGNVFSCSVMHEALHNHYTQKSLSLSLG

SEQ ID NO: 293 - DNA, 1035 bp, synthetic construct
  source 1..1035: mol_type = other DNA
gagaccagggagtgtatctactataacgccaattgggagctggagaggacaaaccagtccggactggagcggtgtgagggcgagcaggacaagagataccattgctacgctagctggcgcaattccagcggcaccatcgagctggtgaagaagggctgttggctggacgatttcaactgttacgatagacaggagtgcgtggccaccgaggagaatcctcaggtgtatttttgctgttgcgagggcaacttctgcaatgagaggttcacccacctgccagaggctggaggaccagaggtgacctatgagccacctccaacaggaggaggaggctctggaggaggaggctccggaggaggaggaacccatacatgtccaccttgcccagctccagagctgctgggaggcccttccgtgttcctgtttccacccaagccaaaggacaccctgatgatctctaggaccccagaggtgacatgcgtggtggtggacgtgtcccacgaggaccccgaggtgaagtttaactggtacgtggatggcgtggaggtgcataatgctaagacaaagccaagggaggagcagtacaactccacctatcgggtggtgagcgtgctgacagtgctgcaccaggattggctgaacggcaaggagtataagtgtaaggtgagcaataaggctctgcctgccccaatcgagaagaccatctctaaggctaagggccagcccagagagcctcaggtgtacacactgcctccatcccgcgacgagctgaccaagaaccaggtgagcctgacatgcctggtgaagggcttctatcccagcgacatcgccgtggagtgggagtctaatggccagcctgagaacaattacaagaccacaccccctgtgctggacagcgatggctctttctttctgtattctaagctgaccgtggataagtcccggtggcagcagggcaacgtgttttcttgttccgtgatgcatgaggccctgcacaatcattacacacagaagagcctgtctctgtcccctggc

SEQ ID NO: 294 - DNA, 1035 bp, synthetic construct
  source 1..1035: mol_type = other DNA
gagaccagggagtgtatctactataacgccaattgggagctggagaggacaaaccagtccggactggagcggtgtgagggcgagcaggacaagagataccattgctacgctagctggcgcaattccagcggcaccatcgagctggtgaagaagggctgttggctggacgatttcaactgttacgatagacaggagtgcgtggcccacgaggagaatcctcaggtgtatttttgctgttgcgagggcaacttctgcaatgagaggttcacccacctgccagaggctggaggaccagaggtgacctatgagccacctccaacaggaggaggaggctctggaggaggaggctccggaggaggaggaacccatacatgtccaccttgcccagctccagagctgctgggaggcccttccgtgttcctgtttccacccaagccaaaggacaccctgatgatctctaggaccccagaggtgacatgcgtggtggtggacgtgtcccacgaggaccccgaggtgaagtttaactggtacgtggatggcgtggaggtgcataatgctaagacaaagccaagggaggagcagtacaactccacctatcgggtggtgagcgtgctgacagtgctgcaccaggattggctgaacggcaaggagtataagtgtaaggtgagcaataaggctctgcctgccccaatcgagaagaccatctctaaggctaagggccagcccagagagcctcaggtgtacacactgcctccatcccgcgacgagctgaccaagaaccaggtgagcctgacatgcctggtgaagggcttctatcccagcgacatcgccgtggagtgggagtctaatggccagcctgagaacaattacaagaccacaccccctgtgctggacagcgatggctctttctttctgtattctaagctgaccgtggataagtcccggtggcagcagggcaacgtgttttcttgttccgtgatgcatgaggccctgcacaatcattacacacagaagagcctgtctctgtcccctggc

SEQ ID NO: 295 - DNA, 1035 bp, synthetic construct; identical to SEQ ID NO: 294
  source 1..1035: mol_type = other DNA

SEQ ID NO: 296 - DNA, 1035 bp, synthetic construct
  source 1..1035: mol_type = other DNA
gagaccagggagtgtatctactataacgccaattgggagctggagaggacaaaccagtccggactggagcggtgtgagggcgagcaggacaagagatggcattgctacgctagctggcgcaattccagcggcaccatcgagctggtgaagaagggctgttggctggacgatttcaactgttacgatagacaggagtgcgtggccaccgaggagaatcctcaggtgtatttttgctgttgcgagggcaacttctgcaatgagaggttcacccacctgccagaggctggaggaccagaggtgacctatgagccacctccaacaggaggaggaggctctggaggaggaggctccggaggaggaggaacccatacatgtccaccttgcccagctccagagctgctgggaggcccttccgtgttcctgtttccacccaagccaaaggacaccctgtacatcaccagggagccagaggtgacatgcgtggtggtggacgtgtcccacgaggaccccgaggtgaagtttaactggtacgtggatggcgtggaggtgcataatgctaagacaaagccaagggaggagcagtacaactccacctatcgggtggtgagcgtgctgacagtgctgcaccaggattggctgaacggcaaggagtataagtgtaaggtgagcaataaggctctgcctgccccaatcgagaagaccatctctaaggctaagggccagcccagagagcctcaggtgtacacactgcctccatcccgcgacgagctgaccaagaaccaggtgagcctgacatgcctggtgaagggcttctatcccagcgacatcgccgtggagtgggagtctaatggccagcctgagaacaattacaagaccacaccccctgtgctggacagcgatggctctttctttctgtattctaagctgaccgtggataagtcccggtggcagcagggcaacgtgttttcttgttccgtgatgcatgaggccctgcacaatcattacacacagaagagcctgtctctgtcccctggc

SEQ ID NO: 297 - DNA, 63 bp, synthetic construct
  source 1..63: mol_type = other DNA
gccaccatggactggacctggagaatcctgttcctggtggctgctgctaccggaacacacgct

SEQ ID NO: 298 - DNA, 1002 bp, synthetic construct
  source 1..1002: mol_type = other DNA
gagacaagagagtgcatctactacaacgccaactgggaactcgagcggaccaaccagtctggcctggaaagatgtgaaggcgagcaggacaagcggctgcactgttacgcctcttggagaaactcctccggcaccatcgagctggtcaagaaaggctgctgggacgacgacttcaactgctacgaccggcaagagtgcgtggccaccgaagagaatccccaggtgtacttctgctgctgcgagggcaacttctgcaacgagcggttcacccatctgcctgaagctggcggacctgaagtgacctatgagcctcctccaaccggcggaggcacacatacttgtcctccatgtccagctccagagctgctcggagggcccagtgtgttcctgtttcctccaaagcctaaggacaccctgatgatctctcggacccctgaagtgacctgcgtggtggtggatgtgtctcacgaggacccagaagtgaagttcaattggtacgtggacggcgtggaagtgcacaacgccaagaccaagcctagagaggaacagtacaactccacctacagagtggtgtccgtgctgaccgtgctgcaccaggattggctgaacggcaaagaatacaagtgcaaggtgtccaacaaggccctgcctgctcctatcgaaaagaccatctccaaggccaagggccagcctagggaaccccaggtgtacacattgcctccatctcgggacgagctgaccaagaaccaggtgtccctgacctgtctggtcaagggcttctacccctccgatatcgccgtggaatgggagtctaatggccagcctgagaacaactacaagaccacacctcctgtgctggactccgacggctcattcttcctgtactccaagctgacagtggacaagtccagatggcagcagggcaacgtgttctcctgctccgtgatgcacgaggccctgcacaatcactacacacagaagtccttaagcttatcccctggc

SEQ ID NO: 299 - DNA, 1002 bp, synthetic construct
  source 1..1002: mol_type = other DNA
gagaccagggagtgtatctactataacgccaattgggagctggagaggacaaaccagtccggactggagcggtgtgagggagagcaggacaagagactgcattgctacgctagctggcgcaattccagcggcaccatcgagctggtgaagaagggctgttggctggacgatttcaactgttacgatagacaggagtgcgtggccaccgaggagaatcctcaggtgtatttttgctgttgcgagggcaacttctgcaatgagaggttcacccacctgccagaggctggaggaccagaggtgacctatgagccacctccaacaggaggaggaacccatacatgtccaccttgcccagctccagagctgctgggaggcccttccgtgttcctgtttccacccaagccaaaggacaccctgatgatctctaggaccccagaggtgacatgcgtggtggtggacgtgtcccacgaggaccccgaggtgaagtttaactggtacgtggatggcgtggaggtgcataatgctaagacaaagccaagggaggagcagtacaactccacctatcgggtggtgagcgtgctgacagtgctgcaccaggattggctgaacggcaaggagtataagtgtaaggtgagcaataaggctctgcctgccccaatcgagaagaccatctctaaggctaagggccagcccagagagcctcaggtgtacacactgcctccatcccgcgacgagctgaccaagaaccaggtgagcctgacatgcctggtgaagggcttctatcccagcgacatcgccgtggagtgggagtctaatggccagcctgagaacaattacaagaccacaccccctgtgctggacagcgatggctctttctttctgtattctaagctgaccgtggataagtcccggtggcagcagggcaacgtgttttcttgttccgtgatgcatgaggccctgcacaatcattacacacagaagagcctgtctctgtcccctggc

SEQ ID NO: 300 - DNA, 1029 bp, synthetic construct
  source 1..1029: mol_type = other DNA
atcctgggccgcagcgagacacaggagtgtctgttctttaacgccaattgggagaaggataggaccaaccagacaggcgtggagccatgttatggcgacaaggataagaggcggcattgcttcgctacctggaagaacatctccggcagcatcgagatcgtgaagcagggctgttggctggacgatatcaattgttacgaccggacagattgcgtggagaagaaggactctcccgaggtgtatttttgctgttgcgagggcaacatgtgcaatgagaagttctcttactttcccgagatggaggtgacccagcctacatccaatccagtgaccccaaagccacctacaggaggaggaacccacacatgtccaccatgccctgctccagagctgctgggaggaccatccgtgttcctgtttcctccaaagcccaaggacaccctgatgatcagcagaacccccgaggtgacatgcgtggtggtggacgtgtctcacgaggaccccgaggtgaagtttaactggtacgtggatggcgtggaggtgcataatgccaagaccaagcctagagaggagcagtacaactccacctatcgcgtggtgagcgtgctgacagtgctgcatcaggattggctgaacggcaaggagtacaagtgtaaggtgtccaataaggctctgcccgtgcctatcgagaagaccatcagcaaggccaagggccagcctagggagccacaggtgtatacactgcccccttcccgggaggagatgaccaagaaccaggtgagcctgacatgcctggtgaagggcttctaccctagcgacatcgctgtggagtgggagtctaatggccagccagagaacaattataagaccacaccacccgtgctggacagcgatggctctttctttctgtactctaagctgaccgtggataagtcccgctggcagcagggcaacgtgttttcttgttccgtgatgcacgaggccctgcacaatcattacacacagaagagcctgtctctgtccccaggc

SEQ ID NO: 301 - DNA, 1035 bp, synthetic construct
  source 1..1035: mol_type = other DNA
gagaccagggagtgtatctactataacgccaattgggagctggagaggacaaaccagtccggactggagcggtgtgaggaggagcaggacaagagactgcattgctacgctagctggcgcaattccagcggcaccatcgagctggtgaagaagggctgttggctggacgatttcaactgttacgatagacaggagtgcgtggccaccgaggagaatcctcaggtgtatttttgctgttgcgagggcaacttctgcaatgagaggttcacccacctgccagaggctggaggaccagaggtgacctatgagccacctccaacaggaggaggaggctctggaggaggaggctccggaggaggaggaacccatacatgtccaccttgcccagctccagagctgctgggaggcccttccgtgttcctgtttccacccaagccaaaggacaccctgatgatctctaggaccccagaggtgacatgcgtggtggtggacgtgtcccacgaggaccccgaggtgaagtttaactggtacgtggatggcgtggaggtgcataatgctaagacaaagccaagggaggagcagtacaactccacctatcgggtggtgagcgtgctgacagtgctgcaccaggattggctgaacggcaaggagtataagtgtaaggtgagcaataaggctctgcctgccccaatcgagaagaccatctctaaggctaagggccagcccagagagcctcaggtgtacacactgcctccatcccgcgacgagctgaccaagaaccaggtgagcctgacatgcctggtgaagggcttctatcccagcgacatcgccgtggagtgggagtctaatggccagcctgagaacaattacaagaccacaccccctgtgctggacagcgatggctctttctttctgtattctaagctgaccgtggataagtcccggtggcagcagggcaacgtgttttcttgttccgtgatgcatgaggccctgcacaatcattacacacagaagagcctgtctctgtcccctggc

SEQ ID NO: 302 - DNA, 1035 bp, synthetic construct
  source 1..1035: mol_type = other DNA
gagaccagggagtgtatctactataacgccaattgggagctggagaggacaaaccagtccggactggagcggtgtgagggcgagcaggacaagagaaggcattgctacgctagctggcgcaattccagcggcaccatcgagctggtgaagaagggctgttggctggacgatttcaactgttacgatagacaggagtgcgtggccaccgaggagaatcctcaggtgtatttttgctgttgcgagggcaacttctgcaatgagaggttcacccacctgccagaggctggaggaccagaggtgacctatgagccacctccaacaggaggaggaggctctggaggaggaggctccggaggaggaggaacccatacatgtccaccttgcccagctccagagctgctgggaggcccttccgtgttcctgtttccacccaagccaaaggacaccctgatgatctctaggaccccagaggtgacatgcgtggtggtggacgtgtcccacgaggaccccgaggtgaagtttaactggtacgtggatggcgtggaggtgcataatgctaagacaaagccaagggaggagcagtacaactccacctatcgggtggtgagcgtgctgacagtgctgcaccaggattggctgaacggcaaggagtataagtgtaaggtgagcaataaggctctgcctgccccaatcgagaagaccatctctaaggctaagggccagcccagagagcctcaggtgtacacactgcctccatcccgcgacgagctgaccaagaaccaggtgagcctgacatgcctggtgaagggcttctatcccagcgacatcgccgtggagtgggagtctaatggccagcctgagaacaattacaagaccacaccccctgtgctggacagcgatggctctttctttctgtattctaagctgaccgtggataagtcccggtggcagcagggcaacgtgttttcttgttccgtgatgcatgaggccctgcacaatcattacacacagaagagcctgtctctgtcccctggc

SEQ ID NO: 303 - DNA, 1035 bp, synthetic construct
  source 1..1035: mol_type = other DNA
gagaccagggagtgtatctactataacgccaattgggagctggagaggacaaaccagtccggactggagcggtgtgagggcgagcaggacaagagactgcattgctacgctagctggcgcaattccagcggcaccatcgagctggtgaagaagggctgttggctggacgatttcaactgttacgatagacaggagtgcgtggcccacgaggagaatcctcaggtgtatttttgctgttgcgagggcaacttctgcaatgagaggttcacccacctgccagaggctggaggaccagaggtgacctatgagccacctccaacaggaggaggaggctctggaggaggaggctccggaggaggaggaacccatacatgtccaccttgcccagctccagagctgctgggaggcccttccgtgttcctgtttccacccaagccaaaggacaccctgatgatctctaggaccccagaggtgacatgcgtggtggtggacgtgtcccacgaggaccccgaggtgaagtttaactggtacgtggatggcgtggaggtgcataatgctaagacaaagccaagggaggagcagtacaactccacctatcgggtggtgagcgtgctgacagtgctgcaccaggattggctgaacggcaaggagtataagtgtaaggtgagcaataaggctctgcctgccccaatcgagaagaccatctctaaggctaagggccagcccagagagcctcaggtgtacacactgcctccatcccgcgacgagctgaccaagaaccaggtgagcctgacatgcctggtgaagggcttctatcccagcgacatcgccgtggagtgggagtctaatggccagcctgagaacaattacaagaccacaccccctgtgctggacagcgatggctctttctttctgtattctaagctgaccgtggataagtcccggtggcagcagggcaacgtgttttcttgttccgtgatgcatgaggccctgcacaatcattacacacagaagagcctgtctctgtcccctggc

SEQ ID NO: 304 - DNA, 1035 bp, synthetic construct
  source 1..1035: mol_type = other DNA
gagaccagggagtgtatctactataacgccaattgggagctggagaggacaaaccagtccggactggagcggtgtgagggcgagcaggacaagagactgcattgctacgctagctggcgcaattccagcggcaccatcgagctggtgaagaagggctgttggctggacgatttcaactgttacgatagacaggagtgcgtggcccaggaggagaatcctcaggtgtatttttgctgttgcgagggcaacttctgcaatgagaggttcacccacctgccagaggctggaggaccagaggtgacctatgagccacctccaacaggaggaggaggctctggaggaggaggctccggaggaggaggaacccatacatgtccaccttgcccagctccagagctgctgggaggcccttccgtgttcctgtttccacccaagccaaaggacaccctgatgatctctaggaccccagaggtgacatgcgtggtggtggacgtgtcccacgaggaccccgaggtgaagtttaactggtacgtggatggcgtggaggtgcataatgctaagacaaagccaagggaggagcagtacaactccacctatcgggtggtgagcgtgctgacagtgctgcaccaggattggctgaacggcaaggagtataagtgtaaggtgagcaataaggctctgcctgccccaatcgagaagaccatctctaaggctaagggccagcccagagagcctcaggtgtacacactgcctccatcccgcgacgagctgaccaagaaccaggtgagcctgacatgcctggtgaagggcttctatcccagcgacatcgccgtggagtgggagtctaatggccagcctgagaacaattacaagaccacaccccctgtgctggacagcgatggctctttctttctgtattctaagctgaccgtggataagtcccggtggcagcagggcaacgtgttttcttgttccgtgatgcatgaggccctgcacaatcattacacacagaagagcctgtctctgtcccctggc

SEQ ID NO: 305 - DNA, 1002 bp, synthetic construct
  source 1..1002: mol_type = other DNA
gagaccagggagtgtatctactataacgccaattgggagctggagaggacaaaccagtccggactggagcggtgtgaggaggagcaggacaagagactgcattgctacgctagctggcgcaattccagcggcaccatcgagctggtgaagaagggctgttggctggacgatttcaactgttacgatagacaggagtgcgtggccaccgaggagaatcctcaggtgtatttttgctgttgcgagggcaacttctgcaatgagaggttcacccacctgccagaggctggaggaccagaggtgacctatgagccacctccaacaggaggaggaacccatacatgtccaccttgcccagctccagagctgctgggaggcccttccgtgttcctgtttccacccaagccaaaggacaccctgatgatctctaggaccccagaggtgacatgcgtggtggtggacgtgtcccacgaggaccccgaggtgaagtttaactggtacgtggatggcgtggaggtgcataatgctaagacaaagccaagggaggagcagtacaactccacctatcgggtggtgagcgtgctgacagtgctgcaccaggattggctgaacggcaaggagtataagtgtaaggtgagcaataaggctctgcctgccccaatcgagaagaccatctctaaggctaagggccagcccagagagcctcaggtgtacacactgcctccatcccgcgacgagctgaccaagaaccaggtgagcctgacatgcctggtgaagggcttctatcccagcgacatcgccgtggagtgggagtctaatggccagcctgagaacaattacaagaccacaccccctgtgctggacagcgatggctctttctttctgtattctaagctgaccgtggataagtcccggtggcagcagggcaacgtgttttcttgttccgtgatgcatgaggccctgcacaatcattacacacagaagagcctgtctctgtcccctggc

SEQ ID NO: 306 - DNA, 1002 bp, synthetic construct
  source 1..1002: mol_type = other DNA
gagaccagggagtgtatctactataacgccaattgggagctggagaggacaaaccagtccggactggagcggtgtgagggagagcaggacaagagataccattgctacgctagctggcgcaattccagcggcaccatcgagctggtgaagaagggctgttggctggacgatttcaactgttacgatagacaggagtgcgtggccaccgaggagaatcctcaggtgtatttttgctgttgcgagggcaacttctgcaatgagaggttcacccacctgccagaggctggaggaccagaggtgacctatgagccacctccaacaggaggaggaacccatacatgtccaccttgcccagctccagagctgctgggaggcccttccgtgttcctgtttccacccaagccaaaggacaccctgatgatctctaggaccccagaggtgacatgcgtggtggtggacgtgtcccacgaggaccccgaggtgaagtttaactggtacgtggatggcgtggaggtgcataatgctaagacaaagccaagggaggagcagtacaactccacctatcgggtggtgagcgtgctgacagtgctgcaccaggattggctgaacggcaaggagtataagtgtaaggtgagcaataaggctctgcctgccccaatcgagaagaccatctctaaggctaagggccagcccagagagcctcaggtgtacacactgcctccatcccgcgacgagctgaccaagaaccaggtgagcctgacatgcctggtgaagggcttctatcccagcgacatcgccgtggagtgggagtctaatggccagcctgagaacaattacaagaccacaccccctgtgctggacagcgatggctctttctttctgtattctaagctgaccgtggataagtcccggtggcagcagggcaacgtgttttcttgttccgtgatgcatgaggccctgcacaatcattacacacagaagagcctgtctctgtcccctggc

SEQ ID NO: 307 - DNA, 1002 bp, synthetic construct
  source 1..1002: mol_type = other DNA
gagaccagggagtgtatctactataacgccaattgggagctggagaggacaaaccagtccggactggagcggtgtgagggagagcaggacaagagactgcattgctacgctagctggcgcaattccagcggcaccatcgagctggtgaagaagggctgttggctggacgatttcaactgttacgatagacaggagtgcgtggcccacgaggagaatcctcaggtgtatttttgctgttgcgagggcaacttctgcaatgagaggttcacccacctgccagaggctggaggaccagaggtgacctatgagccacctccaacaggaggaggaacccatacatgtccaccttgcccagctccagagctgctgggaggcccttccgtgttcctgtttccacccaagccaaaggacaccctgatgatctctaggaccccagaggtgacatgcgtggtggtggacgtgtcccacgaggaccccgaggtgaagtttaactggtacgtggatggcgtggaggtgcataatgctaagacaaagccaagggaggagcagtacaactccacctatcgggtggtgagcgtgctgacagtgctgcaccaggattggctgaacggcaaggagtataagtgtaaggtgagcaataaggctctgcctgccccaatcgagaagaccatctctaaggctaagggccagcccagagagcctcaggtgtacacactgcctccatcccgcgacgagctgaccaagaaccaggtgagcctgacatgcctggtgaagggcttctatcccagcgacatcgccgtggagtgggagtctaatggccagcctgagaacaattacaagaccacaccccctgtgctggacagcgatggctctttctttctgtattctaagctgaccgtggataagtcccggtggcagcagggcaacgtgttttcttgttccgtgatgcatgaggccctgcacaatcattacacacagaagagcctgtctctgtcccctggc

SEQ ID NO: 308 - DNA, 1002 bp, synthetic construct
  source 1..1002: mol_type = other DNA
gagaccagggagtgtatctactataacgccaattgggagctggagaggacaaaccagtccggactggagcggtgtgagggagagcaggacaagagactgcattgctacgctagctggcgcaattccagcggcaccatcgagctggtgaagaagggctgttggctggacgatttcaactgttacgatagacaggagtgcgtggcccaggaggagaatcctcaggtgtatttttgctgttgcgagggcaacttctgcaatgagaggttcacccacctgccagaggctggaggaccagaggtgacctatgagccacctccaacaggaggaggaacccatacatgtccaccttgcccagctccagagctgctgggaggcccttccgtgttcctgtttccacccaagccaaaggacaccctgatgatctctaggaccccagaggtgacatgcgtggtggtggacgtgtcccacgaggaccccgaggtgaagtttaactggtacgtggatggcgtggaggtgcataatgctaagacaaagccaagggaggagcagtacaactccacctatcgggtggtgagcgtgctgacagtgctgcaccaggattggctgaacggcaaggagtataagtgtaaggtgagcaataaggctctgcctgccccaatcgagaagaccatctctaaggctaagggccagcccagagagcctcaggtgtacacactgcctccatcccgcgacgagctgaccaagaaccaggtgagcctgacatgcctggtgaagggcttctatcccagcgacatcgccgtggagtgggagtctaatggccagcctgagaacaattacaagaccacaccccctgtgctggacagcgatggctctttctttctgtattctaagctgaccgtggataagtcccggtggcagcagggcaacgtgttttcttgttccgtgatgcatgaggccctgcacaatcattacacacagaagagcctgtctctgtcccctggc

SEQ ID NO: 309 - DNA, 1002 bp, synthetic construct
  source 1..1002: mol_type = other DNA
gagaccagggagtgtatctactataacgccaattgggagctggagaggacaaaccagtccggactggagcggtgtgagggagagcaggacaagagataccattgctacgctagctggcgcaattccagcggcaccatcgagctggtgaagaagggctgttggctggacgatttcaactgttacgatagacaggagtgcgtggcccacgaggagaatcctcaggtgtatttttgctgttgcgagggcaacttctgcaatgagaggttcacccacctgccagaggctggaggaccagaggtgacctatgagccacctccaacaggaggaggaacccatacatgtccaccttgcccagctccagagctgctgggaggcccttccgtgttcctgtttccacccaagccaaaggacaccctgatgatctctaggaccccagaggtgacatgcgtggtggtggacgtgtcccacgaggaccccgaggtgaagtttaactggtacgtggatggcgtggaggtgcataatgctaagacaaagccaagggaggagcagtacaactccacctatcgggtggtgagcgtgctgacagtgctgcaccaggattggctgaacggcaaggagtataagtgtaaggtgagcaataaggctctgcctgccccaatcgagaagaccatctctaaggctaagggccagcccagagagcctcaggtgtacacactgcctccatcccgcgacgagctgaccaagaaccaggtgagcctgacatgcctggtgaagggcttctatcccagcgacatcgccgtggagtgggagtctaatggccagcctgagaacaattacaagaccacaccccctgtgctggacagcgatggctctttctttctgtattctaagctgaccgtggataagtcccggtggcagcagggcaacgtgttttcttgttccgtgatgcatgaggccctgcacaatcattacacacagaagagcctgtctctgtcccctggc

SEQ ID NO: 310 - DNA, 1023 bp, synthetic construct
  source 1..1023: mol_type = other DNA
gagaccagggagtgtatctactataacgccaattgggagctggagaggacaaaccagtccggactggagcggtgtgagggcgagcaggacaagagataccattgctacgctagctggcgcaattccagcggcaccatcgagctggtgaagaagggctgttggctggacgatttcaactgttacgatagacaggagtgcgtggcccacgaggagaatcctcaggtgtatttttgctgttgcgagggcaacttctgcaatgagaggttcacccacctgccagaggctggaggaccagaggtgacctatgagccacctccaacaggaggaggaggctctggaggaggaggctccacccatacatgtccaccttgcccagctccagagctgctgggaggcccttccgtgttcctgtttccacccaagccaaaggacaccctgatgatctctaggaccccagaggtgacatgcgtggtggtggacgtgtcccacgaggaccccgaggtgaagtttaactggtacgtggatggcgtggaggtgcataatgctaagacaaagccaagggaggagcagtacaactccacctatcgggtggtgagcgtgctgacagtgctgcaccaggattggctgaacggcaaggagtataagtgtaaggtgagcaataaggctctgcctgccccaatcgagaagaccatctctaaggctaagggccagcccagagagcctcaggtgtacacactgcctccatcccgcgacgagctgaccaagaaccaggtgagcctgacatgcctggtgaagggcttctatcccagcgacatcgccgtggagtgggagtctaatggccagcctgagaacaattacaagaccacaccccctgtgctggacagcgatggctctttctttctgtattctaagctgaccgtggataagtcccggtggcagcagggcaacgtgttttcttgttccgtgatgcatgaggccctgcacaatcattacacacagaagagcctgtctctgtcccctggc

SEQ ID NO: 311 - DNA, 1002 bp, synthetic construct
  source 1..1002: mol_type = other DNA
gagaccagggagtgtatctactataacgccaattgggagctggagaggacaaaccagtccggactggagcggtgtgagggagagcaggacaagagataccattgctacgctagctggcgcaattccagcggcaccatcgagctggtgaagaagggctgttggctggacgatttcaactgttacgatagacaggagtgcgtggcccaggaggagaatcctcaggtgtatttttgctgttgcgagggcaacttctgcaatgagaggttcacccacctgccagaggctggaggaccagaggtgacctatgagccacctccaacaggaggaggaacccatacatgtccaccttgcccagctccagagctgctgggaggcccttccgtgttcctgtttccacccaagccaaaggacaccctgatgatctctaggaccccagaggtgacatgcgtggtggtggacgtgtcccacgaggaccccgaggtgaagtttaactggtacgtggatggcgtggaggtgcataatgctaagacaaagccaagggaggagcagtacaactccacctatcgggtggtgagcgtgctgacagtgctgcaccaggattggctgaacggcaaggagtataagtgtaaggtgagcaataaggctctgcctgccccaatcgagaagaccatctctaaggctaagggccagcccagagagcctcaggtgtacacactgcctccatcccgcgacgagctgaccaagaaccaggtgagcctgacatgcctggtgaagggcttctatcccagcgacatcgccgtggagtgggagtctaatggccagcctgagaacaattacaagaccacaccccctgtgctggacagcgatggctctttctttctgtattctaagctgaccgtggataagtcccggtggcagcagggcaacgtgttttcttgttccgtgatgcatgaggccctgcacaatcattacacacagaagagcctgtctctgtcccctggc

SEQ ID NO: 312 - DNA, 1023 bp, synthetic construct
  source 1..1023: mol_type = other DNA
gagaccagggagtgtatctactataacgccaattgggagctggagaggacaaaccagtccggactggagcggtgtgagggcgagcaggacaagagataccattgctacgctagctggcgcaattccagcggcaccatcgagctggtgaagaagggctgttggctggacgatttcaactgttacgatagacaggagtgcgtggcccaggaggagaatcctcaggtgtatttttgctgttgcgagggcaacttctgcaatgagaggttcacccacctgccagaggctggaggaccagaggtgacctatgagccacctccaacaggaggaggaggctctggaggaggaggctccacccatacatgtccaccttgcccagctccagagctgctgggaggcccttccgtgttcctgtttccacccaagccaaaggacaccctgatgatctctaggaccccagaggtgacatgcgtggtggtggacgtgtcccacgaggaccccgaggtgaagtttaactggtacgtggatggcgtggaggtgcataatgctaagacaaagccaagggaggagcagtacaactccacctatcgggtggtgagcgtgctgacagtgctgcaccaggattggctgaacggcaaggagtataagtgtaaggtgagcaataaggctctgcctgccccaatcgagaagaccatctctaaggctaagggccagcccagagagcctcaggtgtacacactgcctccatcccgcgacgagctgaccaagaaccaggtgagcctgacatgcctggtgaagggcttctatcccagcgacatcgccgtggagtgggagtctaatggccagcctgagaacaattacaagaccacaccccctgtgctggacagcgatggctctttctttctgtattctaagctgaccgtggataagtcccggtggcagcagggcaacgtgttttcttgttccgtgatgcatgaggccctgcacaatcattacacacagaagagcctgtctctgtcccctggc

SEQ ID NO: 313 - DNA, 1035 bp, synthetic construct
  source 1..1035: mol_type = other DNA
gagaccagggagtgtatctactataacgccaattgggagctggagaggacaaaccagtccggactggagcggtgtgagggcgagcaggacaagagataccattgctacgctagctggcgcaattccagcggcaccatcgagctggtgaagaagggctgttggctggacgatttcaactgttacgatagacaggagtgcgtggcccaggaggagaatcctcaggtgtatttttgctgttgcgagggcaacttctgcaatgagaggttcacccacctgccagaggctggaggaccagaggtgacctatgagccacctccaacaggaggaggaggctctggaggaggaggctccggaggaggaggaacccatacatgtccaccttgcccagctccagagctgctgggaggcccttccgtgttcctgtttccacccaagccaaaggacaccctgatgatctctaggaccccagaggtgacatgcgtggtggtggacgtgtcccacgaggaccccgaggtgaagtttaactggtacgtggatggcgtggaggtgcataatgctaagacaaagccaagggaggagcagtacaactccacctatcgggtggtgagcgtgctgacagtgctgcaccaggattggctgaacggcaaggagtataagtgtaaggtgagcaataaggctctgcctgccccaatcgagaagaccatctctaaggctaagggccagcccagagagcctcaggtgtacacactgcctccatcccgcgacgagctgaccaagaaccaggtgagcctgacatgcctggtgaagggcttctatcccagcgacatcgccgtggagtgggagtctaatggccagcctgagaacaattacaagaccacaccccctgtgctggacagcgatggctctttctttctgtattctaagctgaccgtggataagtcccggtggcagcagggcaacgtgttttcttgttccgtgatgcatgaggccctgcacaatcattacacacagaagagcctgtctctgtcccctggc

SEQ ID NO: 314 - DNA, 1002 bp, synthetic construct
  source 1..1002: mol_type = other DNA
gagaccagggagtgtatctactataacgccaattgggagctggagaggacaaaccagtccggactggagcggtgtgagggagagcaggacaagagataccattgctacgctagctggcgcaattccagcggcaccatcgagctggtgaagaagggctgttggctggacgatttcaactgttacgatagacaggagtgcgtggccgaggaggagaatcctcaggtgtatttttgctgttgcgagggcaacttctgcaatgagaggttcacccacctgccagaggctggaggaccagaggtgacctatgagccacctccaacaggaggaggaacccatacatgtccaccttgcccagctccagagctgctgggaggcccttccgtgttcctgtttccacccaagccaaaggacaccctgatgatctctaggaccccagaggtgacatgcgtggtggtggacgtgtcccacgaggaccccgaggtgaagtttaactggtacgtggatggcgtggaggtgcataatgctaagacaaagccaagggaggagcagtacaactccacctatcgggtggtgagcgtgctgacagtgctgcaccaggattggctgaacggcaaggagtataagtgtaaggtgagcaataaggctctgcctgccccaatcgagaagaccatctctaaggctaagggccagcccagagagcctcaggtgtacacactgcctccatcccgcgacgagctgaccaagaaccaggtgagcctgacatgcctggtgaagggcttctatcccagcgacatcgccgtggagtgggagtctaatggccagcctgagaacaattacaagaccacaccccctgtgctggacagcgatggctctttctttctgtattctaagctgaccgtggataagtcccggtggcagcagggcaacgtgttttcttgttccgtgatgcatgaggccctgcacaatcattacacacagaagagcctgtctctgtcccctggc

SEQ ID NO: 315 - DNA, 1023 bp, synthetic construct
  source 1..1023: mol_type = other DNA
gagaccagggagtgtatctactataacgccaattgggagctggagaggacaaaccagtccggactggagcggtgtgagggcgagcaggacaagagataccattgctacgctagctggcgcaattccagcggcaccatcgagctggtgaagaagggctgttggctggacgatttcaactgttacgatagacaggagtgcgtggccgaggaggagaatcctcaggtgtatttttgctgttgcgagggcaacttctgcaatgagaggttcacccacctgccagaggctggaggaccagaggtgacctatgagccacctccaacaggaggaggaggctctggaggaggaggctccacccatacatgtccaccttgcccagctccagagctgctgggaggcccttccgtgttcctgtttccacccaagccaaaggacaccctgatgatctctaggaccccagaggtgacatgcgtggtggtggacgtgtcccacgaggaccccgaggtgaagtttaactggtacgtggatggcgtggaggtgcataatgctaagacaaagccaagggaggagcagtacaactccacctatcgggtggtgagcgtgctgacagtgctgcaccaggattggctgaacggcaaggagtataagtgtaaggtgagcaataaggctctgcctgccccaatcgagaagaccatctctaaggctaagggccagcccagagagcctcaggtgtacacactgcctccatcccgcgacgagctgaccaagaaccaggtgagcctgacatgcctggtgaagggcttctatcccagcgacatcgccgtggagtgggagtctaatggccagcctgagaacaattacaagaccacaccccctgtgctggacagcgatggctctttctttctgtattctaagctgaccgtggataagtcccggtggcagcagggcaacgtgttttcttgttccgtgatgcatgaggccctgcacaatcattacacacagaagagcctgtctctgtcccctggc

SEQ ID NO: 316 - DNA, 1035 bp, synthetic construct
  source 1..1035: mol_type = other DNA
gagaccagggagtgtatctactataacgccaattgggagctggagaggacaaaccagtccggactggagcggtgtgagggcgagcaggacaagagataccattgctacgctagctggcgcaattccagcggcaccatcgagctggtgaagaagggctgttggctggacgatttcaactgttacgatagacaggagtgcgtggccgaggaggagaatcctcaggtgtatttttgctgttgcgagggcaacttctgcaatgagaggttcacccacctgccagaggctggaggaccagaggtgacctatgagccacctccaacaggaggaggaggctctggaggaggaggctccggaggaggaggaacccatacatgtccaccttgcccagctccagagctgctgggaggcccttccgtgttcctgtttccacccaagccaaaggacaccctgatgatctctaggaccccagaggtgacatgcgtggtggtggacgtgtcccacgaggaccccgaggtgaagtttaactggtacgtggatggcgtggaggtgcataatgctaagacaaagccaagggaggagcagtacaactccacctatcgggtggtgagcgtgctgacagtgctgcaccaggattggctgaacggcaaggagtataagtgtaaggtgagcaataaggctctgcctgccccaatcgagaagaccatctctaaggctaagggccagcccagagagcctcaggtgtacacactgcctccatcccgcgacgagctgaccaagaaccaggtgagcctgacatgcctggtgaagggcttctatcccagcgacatcgccgtggagtgggagtctaatggccagcctgagaacaattacaagaccacaccccctgtgctggacagcgatggctctttctttctgtattctaagctgaccgtggataagtcccggtggcagcagggcaacgtgttttcttgttccgtgatgcatgaggccctgcacaatcattacacacagaagagcctgtctctgtcccctggc

SEQ ID NO: 317 - DNA, 1002 bp, synthetic construct
  source 1..1002: mol_type = other DNA
gagaccagggagtgtatctactataacgccaattgggagctggagaggacaaaccagtccggactggagcggtgtgaggacgagcaggacaagagataccattgctacgctagctggcgcaattccagcggcaccatcgagctggtgaagaagggctgttggctggacgatttcaactgttacgatagacaggagtgcgtggccaccgaggagaatcctcaggtgtatttttgctgttgcgagggcaacttctgcaatgagaggttcacccacctgccagaggctggaggaccagaggtgacctatgagccacctccaacaggaggaggaacccatacatgtccaccttgcccagctccagagctgctgggaggcccttccgtgttcctgtttccacccaagccaaaggacaccctgatgatctctaggaccccagaggtgacatgcgtggtggtggacgtgtcccacgaggaccccgaggtgaagtttaactggtacgtggatggcgtggaggtgcataatgctaagacaaagccaagggaggagcagtacaactccacctatcgggtggtgagcgtgctgacagtgctgcaccaggattggctgaacggcaaggagtataagtgtaaggtgagcaataaggctctgcctgccccaatcgagaagaccatctctaaggctaagggccagcccagagagcctcaggtgtacacactgcctccatcccgcgacgagctgaccaagaaccaggtgagcctgacatgcctggtgaagggcttctatcccagcgacatcgccgtggagtgggagtctaatggccagcctgagaacaattacaagaccacaccccctgtgctggacagcgatggctctttctttctgtattctaagctgaccgtggataagtcccggtggcagcagggcaacgtgttttcttgttccgtgatgcatgaggccctgcacaatcattacacacagaagagcctgtctctgtcccctggc

SEQ ID NO: 318 - DNA, 1023 bp, synthetic construct
  source 1..1023: mol_type = other DNA
gagaccagggagtgtatctactataacgccaattgggagctggagaggacaaaccagtccggactggagcggtgtgaggacgagcaggacaagagataccattgctacgctagctggcgcaattccagcggcaccatcgagctggtgaagaagggctgttggctggacgatttcaactgttacgatagacaggagtgcgtggccaccgaggagaatcctcaggtgtatttttgctgttgcgagggcaacttctgcaatgagaggttcacccacctgccagaggctggaggaccagaggtgacctatgagccacctccaacaggaggaggaggctctggaggaggaggctccacccatacatgtccaccttgcccagctccagagctgctgggaggcccttccgtgttcctgtttccacccaagccaaaggacaccctgatgatctctaggaccccagaggtgacatgcgtggtggtggacgtgtcccacgaggaccccgaggtgaagtttaactggtacgtggatggcgtggaggtgcataatgctaagacaaagccaagggaggagcagtacaactccacctatcgggtggtgagcgtgctgacagtgctgcaccaggattggctgaacggcaaggagtataagtgtaaggtgagcaataaggctctgcctgccccaatcgagaagaccatctctaaggctaagggccagcccagagagcctcaggtgtacacactgcctccatcccgcgacgagctgaccaagaaccaggtgagcctgacatgcctggtgaagggcttctatcccagcgacatcgccgtggagtgggagtctaatggccagcctgagaacaattacaagaccacaccccctgtgctggacagcgatggctctttctttctgtattctaagctgaccgtggataagtcccggtggcagcagggcaacgtgttttcttgttccgtgatgcatgaggccctgcacaatcattacacacagaagagcctgtctctgtcccctggc

SEQ ID NO: 319 - DNA, 1035 bp, synthetic construct
  source 1..1035: mol_type = other DNA
gagaccagggagtgtatctactataacgccaattgggagctggagaggacaaaccagtccggactggagcggtgtgaggacgagcaggacaagagataccattgctacgctagctggcgcaattccagcggcaccatcgagctggtgaagaagggctgttggctggacgatttcaactgttacgatagacaggagtgcgtggccaccgaggagaatcctcaggtgtatttttgctgttgcgagggcaacttctgcaatgagaggttcacccacctgccagaggctggaggaccagaggtgacctatgagccacctccaacaggaggaggaggctctggaggaggaggctccggaggaggaggaacccatacatgtccaccttgcccagctccagagctgctgggaggcccttccgtgttcctgtttccacccaagccaaaggacaccctgatgatctctaggaccccagaggtgacatgcgtggtggtggacgtgtcccacgaggaccccgaggtgaagtttaactggtacgtggatggcgtggaggtgcataatgctaagacaaagccaagggaggagcagtacaactccacctatcgggtggtgagcgtgctgacagtgctgcaccaggattggctgaacggcaaggagtataagtgtaaggtgagcaataaggctctgcctgccccaatcgagaagaccatctctaaggctaagggccagcccagagagcctcaggtgtacacactgcctccatcccgcgacgagctgaccaagaaccaggtgagcctgacatgcctggtgaagggcttctatcccagcgacatcgccgtggagtgggagtctaatggccagcctgagaacaattacaagaccacaccccctgtgctggacagcgatggctctttctttctgtattctaagctgaccgtggataagtcccggtggcagcagggcaacgtgttttcttgttccgtgatgcatgaggccctgcacaatcattacacacagaagagcctgtctctgtcccctggc

SEQ ID NO: 320 - DNA, 1002 bp, synthetic construct
  source 1..1002: mol_type = other DNA
gagaccagggagtgtatctactataacgccaattgggagctggagaggacaaaccagtccggactggagcggtgtgaggaggagcaggacaagagataccattgctacgctagctggcgcaattccagcggcaccatcgagctggtgaagaagggctgttggctggacgatttcaactgttacgatagacaggagtgcgtggccaccgaggagaatcctcaggtgtatttttgctgttgcgagggcaacttctgcaatgagaggttcacccacctgccagaggctggaggaccagaggtgacctatgagccacctccaacaggaggaggaacccatacatgtccaccttgcccagctccagagctgctgggaggcccttccgtgttcctgtttccacccaagccaaaggacaccctgatgatctctaggaccccagaggtgacatgcgtggtggtggacgtgtcccacgaggaccccgaggtgaagtttaactggtacgtggatggcgtggaggtgcataatgctaagacaaagccaagggaggagcagtacaactccacctatcgggtggtgagcgtgctgacagtgctgcaccaggattggctgaacggcaaggagtataagtgtaaggtgagcaataaggctctgcctgccccaatcgagaagaccatctctaaggctaagggccagcccagagagcctcaggtgtacacactgcctccatcccgcgacgagctgaccaagaaccaggtgagcctgacatgcctggtgaagggcttctatcccagcgacatcgccgtggagtgggagtctaatggccagcctgagaacaattacaagaccacaccccctgtgctggacagcgatggctctttctttctgtattctaagctgaccgtggataagtcccggtggcagcagggcaacgtgttttcttgttccgtgatgcatgaggccctgcacaatcattacacacagaagagcctgtctctgtcccctggc

SEQ ID NO: 321 - DNA, 1023 bp, synthetic construct
  source 1..1023: mol_type = other DNA
gagaccagggagtgtatctactataacgccaattgggagctggagaggacaaaccagtccggactggagcggtgtgaggaggagcaggacaagagataccattgctacgctagctggcgcaattccagcggcaccatcgagctggtgaagaagggctgttggctggacgatttcaactgttacgatagacaggagtgcgtggccaccgaggagaatcctcaggtgtatttttgctgttgcgagggcaacttctgcaatgagaggttcacccacctgccagaggctggaggaccagaggtgacctatgagccacctccaacaggaggaggaggctctggaggaggaggctccacccatacatgtccaccttgcccagctccagagctgctgggaggcccttccgtgttcctgtttccacccaagccaaaggacaccctgatgatctctaggaccccagaggtgacatgcgtggtggtggacgtgtcccacgaggaccccgaggtgaagtttaactggtacgtggatggcgtggaggtgcataatgctaagacaaagccaagggaggagcagtacaactccacctatcgggtggtgagcgtgctgacagtgctgcaccaggattggctgaacggcaaggagtataagtgtaaggtgagcaataaggctctgcctgccccaatcgagaagaccatctctaaggctaagggccagcccagagagcctcaggtgtacacactgcctccatcccgcgacgagctgaccaagaaccaggtgagcctgacatgcctggtgaagggcttctatcccagcgacatcgccgtggagtgggagtctaatggccagcctgagaacaattacaagaccacaccccctgtgctggacagcgatggctctttctttctgtattctaagctgaccgtggataagtcccggtggcagcagggcaacgtgttttcttgttccgtgatgcatgaggccctgcacaatcattacacacagaagagcctgtctctgtcccctggc

SEQ ID NO: 322 - DNA, 1035 bp, synthetic construct
  source 1..1035: mol_type = other DNA
gagaccagggagtgtatctactataacgccaattgggagctggagaggacaaaccagtccggactggagcggtgtgaggaggagcaggacaagagataccattgctacgctagctggcgcaattccagcggcaccatcgagctggtgaagaagggctgttggctggacgatttcaactgttacgatagacaggagtgcgtggccaccgaggagaatcctcaggtgtatttttgctgttgcgagggcaacttctgcaatgagaggttcacccacctgccagaggctggaggaccagaggtgacctatgagccacctccaacaggaggaggaggctctggaggaggaggctccggaggaggaggaacccatacatgtccaccttgcccagctccagagctgctgggaggcccttccgtgttcctgtttccacccaagccaaaggacaccctgatgatctctaggaccccagaggtgacatgcgtggtggtggacgtgtcccacgaggaccccgaggtgaagtttaactggtacgtggatggcgtggaggtgcataatgctaagacaaagccaagggaggagcagtacaactccacctatcgggtggtgagcgtgctgacagtgctgcaccaggattggctgaacggcaaggagtataagtgtaaggtgagcaataaggctctgcctgccccaatcgagaagaccatctctaaggctaagggccagcccagagagcctcaggtgtacacactgcctccatcccgcgacgagctgaccaagaaccaggtgagcctgacatgcctggtgaagggcttctatcccagcgacatcgccgtggagtgggagtctaatggccagcctgagaacaattacaagaccacaccccctgtgctggacagcgatggctctttctttctgtattctaagctgaccgtggataagtcccggtggcagcagggcaacgtgttttcttgttccgtgatgcatgaggccctgcacaatcattacacacagaagagcctgtctctgtcccctggc

SEQ ID NO: 323 - DNA, 1002 bp, synthetic construct
  source 1..1002: mol_type = other DNA
gagaccagggagtgtatctactataacgccaattgggagctggagaggacaaaccagtccggactggagcggtgtgagggagagcaggacaagagattccattgctacgctagctggcgcaattccagcggcaccatcgagctggtgaagaagggctgttggctggacgatttcaactgttacgatagacaggagtgcgtggcccaggaggagaatcctcaggtgtatttttgctgttgcgagggcaacttctgcaatgagaggttcacccacctgccagaggctggaggaccagaggtgacctatgagccacctccaacaggaggaggaacccatacatgtccaccttgcccagctccagagctgctgggaggcccttccgtgttcctgtttccacccaagccaaaggacaccctgatgatctctaggaccccagaggtgacatgcgtggtggtggacgtgtcccacgaggaccccgaggtgaagtttaactggtacgtggatggcgtggaggtgcataatgctaagacaaagccaagggaggagcagtacaactccacctatcgggtggtgagcgtgctgacagtgctgcaccaggattggctgaacggcaaggagtataagtgtaaggtgagcaataaggctctgcctgccccaatcgagaagaccatctctaaggctaagggccagcccagagagcctcaggtgtacacactgcctccatcccgcgacgagctgaccaagaaccaggtgagcctgacatgcctggtgaagggcttctatcccagcgacatcgccgtggagtgggagtctaatggccagcctgagaacaattacaagaccacaccccctgtgctggacagcgatggctctttctttctgtattctaagctgaccgtggataagtcccggtggcagcagggcaacgtgttttcttgttccgtgatgcatgaggccctgcacaatcattacacacagaagagcctgtctctgtcccctggc

SEQ ID NO: 324 - DNA, 1023 bp, synthetic construct
  source 1..1023: mol_type = other DNA
gagaccagggagtgtatctactataacgccaattgggagctggagaggacaaaccagtccggactggagcggtgtgagggcgagcaggacaagagattccattgctacgctagctggcgcaattccagcggcaccatcgagctggtgaagaagggctgttggctggacgatttcaactgttacgatagacaggagtgcgtggcccaggaggagaatcctcaggtgtatttttgctgttgcgagggcaacttctgcaatgagaggttcacccacctgccagaggctggaggaccagaggtgacctatgagccacctccaacaggaggaggaggctctggaggaggaggctccacccatacatgtccaccttgcccagctccagagctgctgggaggcccttccgtgttcctgtttccacccaagccaaaggacaccctgatgatctctaggaccccagaggtgacatgcgtggtggtggacgtgtcccacgaggaccccgaggtgaagtttaactggtacgtggatggcgtggaggtgcataatgctaagacaaagccaagggaggagcagtacaactccacctatcgggtggtgagcgtgctgacagtgctgcaccaggattggctgaacggcaaggagtataagtgtaaggtgagcaataaggctctgcctgccccaatcgagaagaccatctctaaggctaagggccagcccagagagcctcaggtgtacacactgcctccatcccgcgacgagctgaccaagaaccaggtgagcctgacatgcctggtgaagggcttctatcccagcgacatcgccgtggagtgggagtctaatggccagcctgagaacaattacaagaccacaccccctgtgctggacagcgatggctctttctttctgtattctaagctgaccgtggataagtcccggtggcagcagggcaacgtgttttcttgttccgtgatgcatgaggccctgcacaatcattacacacagaagagcctgtctctgtcccctggc

SEQ ID NO: 325 - DNA, 1035 bp, synthetic construct
  source 1..1035: mol_type = other DNA
gagaccagggagtgtatctactataacgccaattgggagctggagaggacaaaccagtccggactggagcggtgtgagggcgagcaggacaagagattccattgctacgctagctggcgcaattccagcggcaccatcgagctggtgaagaagggctgttggctggacgatttcaactgttacgatagacaggagtgcgtggcccaggaggagaatcctcaggtgtatttttgctgttgcgagggcaacttctgcaatgagaggttcacccacctgccagaggctggaggaccagaggtgacctatgagccacctccaacaggaggaggaggctctggaggaggaggctccggaggaggaggaacccatacatgtccaccttgcccagctccagagctgctgggaggcccttccgtgttcctgtttccacccaagccaaaggacaccctgatgatctctaggaccccagaggtgacatgcgtggtggtggacgtgtcccacgaggaccccgaggtgaagtttaactggtacgtggatggcgtggaggtgcataatgctaagacaaagccaagggaggagcagtacaactccacctatcgggtggtgagcgtgctgacagtgctgcaccaggattggctgaacggcaaggagtataagtgtaaggtgagcaataaggctctgcctgccccaatcgagaagaccatctctaaggctaagggccagcccagagagcctcaggtgtacacactgcctccatcccgcgacgagctgaccaagaaccaggtgagcctgacatgcctggtgaagggcttctatcccagcgacatcgccgtggagtgggagtctaatggccagcctgagaacaattacaagaccacaccccctgtgctggacagcgatggctctttctttctgtattctaagctgaccgtggataagtcccggtggcagcagggcaacgtgttttcttgttccgtgatgcatgaggccctgcacaatcattacacacagaagagcctgtctctgtcccctggc

SEQ ID NO: 326 - DNA, 1002 bp, synthetic construct
  source 1..1002: mol_type = other DNA
gagaccagggagtgtatctactataacgccaattgggagctggagaggacaaaccagtccggactggagcggtgtgagggagagcaggacaagagactgcattgctacgctagctggcgcaattccagcggcaccatcgagctggtgaagaagggctgttggctggacgatttcaactgttacgatagacaggagtgcgtggccgaggaggagaatcctcaggtgtatttttgctgttgcgagggcaacttctgcaatgagaggttcacccacctgccagaggctggaggaccagaggtgacctatgagccacctccaacaggaggaggaacccatacatgtccaccttgcccagctccagagctgctgggaggcccttccgtgttcctgtttccacccaagccaaaggacaccctgatgatctctaggaccccagaggtgacatgcgtggtggtggacgtgtcccacgaggaccccgaggtgaagtttaactggtacgtggatggcgtggaggtgcataatgctaagacaaagccaagggaggagcagtacaactccacctatcgggtggtgagcgtgctgacagtgctgcaccaggattggctgaacggcaaggagtataagtgtaaggtgagcaataaggctctgcctgccccaatcgagaagaccatctctaaggctaagggccagcccagagagcctcaggtgtacacactgcctccatcccgcgacgagctgaccaagaaccaggtgagcctgacatgcctggtgaagggcttctatcccagcgacatcgccgtggagtgggagtctaatggccagcctgagaacaattacaagaccacaccccctgtgctggacagcgatggctctttctttctgtattctaagctgaccgtggataagtcccggtggcagcagggcaacgtgttttcttgttccgtgatgcatgaggccctgcacaatcattacacacagaagagcctgtctctgtcccctggc

SEQ ID NO: 327 - DNA, 1023 bp, synthetic construct
  source 1..1023: mol_type = other DNA
gagaccagggagtgtatctactataacgccaattgggagctggagaggacaaaccagtccggactggagcggtgtgagggcgagcaggacaagagactgcattgctacgctagctggcgcaattccagcggcaccatcgagctggtgaagaagggctgttggctggacgatttcaactgttacgatagacaggagtgcgtggccgaggaggagaatcctcaggtgtatttttgctgttgcgagggcaacttctgcaatgagaggttcacccacctgccagaggctggaggaccagaggtgacctatgagccacctccaacaggaggaggaggctctggaggaggaggctccacccatacatgtccaccttgcccagctccagagctgctgggaggcccttccgtgttcctgtttccacccaagccaaaggacaccctgatgatctctaggaccccagaggtgacatgcgtggtggtggacgtgtcccacgaggaccccgaggtgaagtttaactggtacgtggatggcgtggaggtgcataatgctaagacaaagccaagggaggagcagtacaactccacctatcgggtggtgagcgtgctgacagtgctgcaccaggattggctgaacggcaaggagtataagtgtaaggtgagcaataaggctctgcctgccccaatcgagaagaccatctctaaggctaagggccagcccagagagcctcaggtgtacacactgcctccatcccgcgacgagctgaccaagaaccaggtgagcctgacatgcctggtgaagggcttctatcccagcgacatcgccgtggagtgggagtctaatggccagcctgagaacaattacaagaccacaccccctgtgctggacagcgatggctctttctttctgtattctaagctgaccgtggataagtcccggtggcagcagggcaacgtgttttcttgttccgtgatgcatgaggccctgcacaatcattacacacagaagagcctgtctctgtcccctggc

SEQ ID NO: 328 - DNA, 1035 bp, synthetic construct
  source 1..1035: mol_type = other DNA
gagaccagggagtgtatctactataacgccaattgggagctggagaggacaaaccagtccggactggagcggtgtgagggcgagcaggacaagagactgcattgctacgctagctggcgcaattccagcggcaccatcgagctggtgaagaagggctgttggctggacgatttcaactgttacgatagacaggagtgcgtggccgaggaggagaatcctcaggtgtatttttgctgttgcgagggcaacttctgcaatgagaggttcacccacctgccagaggctggaggaccagaggtgacctatgagccacctccaacaggaggaggaggctctggaggaggaggctccggaggaggaggaacccatacatgtccaccttgcccagctccagagctgctgggaggcccttccgtgttcctgtttccacccaagccaaaggacaccctgatgatctctaggaccccagaggtgacatgcgtggtggtggacgtgtcccacgaggaccccgaggtgaagtttaactggtacgtggatggcgtggaggtgcataatgctaagacaaagccaagggaggagcagtacaactccacctatcgggtggtgagcgtgctgacagtgctgcaccaggattggctgaacggcaaggagtataagtgtaaggtgagcaataaggctctgcctgccccaatcgagaagaccatctctaaggctaagggccagcccagagagcctcaggtgtacacactgcctccatcccgcgacgagctgaccaagaaccaggtgagcctgacatgcctggtgaagggcttctatcccagcgacatcgccgtggagtgggagtctaatggccagcctgagaacaattacaagaccacaccccctgtgctggacagcgatggctctttctttctgtattctaagctgaccgtggataagtcccggtggcagcagggcaacgtgttttcttgttccgtgatgcatgaggccctgcacaatcattacacacagaagagcctgtctctgtcccctggc

SEQ ID NO: 329 - DNA, 1002 bp, synthetic construct
  source 1..1002: mol_type = other DNA
gagaccagggagtgtatctactataacgccaattgggagctggagaggacaaaccagtccggactggagcggtgtgagggagagcaggacaagagattccattgctacgctagctggcgcaattccagcggcaccatcgagctggtgaagaagggctgttggctggacgatttcaactgttacgatagacaggagtgcgtggccaccgaggagaatcctcaggtgtatttttgctgttgcgagggcaacttctgcaatgagaggttcacccacctgccagaggctggaggaccagaggtgacctatgagccacctccaacaggaggaggaacccatacatgtccaccttgcccagctccagagctgctgggaggcccttccgtgttcctgtttccacccaagccaaaggacaccctgatgatctctaggaccccagaggtgacatgcgtggtggtggacgtgtcccacgaggaccccgaggtgaagtttaactggtacgtggatggcgtggaggtgcataatgctaagacaaagccaagggaggagcagtacaactccacctatcgggtggtgagcgtgctgacagtgctgcaccaggattggctgaacggcaaggagtataagtgtaaggtgagcaataaggctctgcctgccccaatcgagaagaccatctctaaggctaagggccagcccagagagcctcaggtgtacacactgcctccatcccgcgacgagctgaccaagaaccaggtgagcctgacatgcctggtgaagggcttctatcccagcgacatcgccgtggagtgggagtctaatggccagcctgagaacaattacaagaccacaccccctgtgctggacagcgatggctctttctttctgtattctaagctgaccgtggataagtcccggtggcagcagggcaacgtgttttcttgttccgtgatgcatgaggccctgcacaatcattacacacagaagagcctgtctctgtcccctggc

SEQ ID NO: 330 - DNA, 1023 bp, synthetic construct
  source 1..1023: mol_type = other DNA
gagaccagggagtgtatctactataacgccaattgggagctggagaggacaaaccagtccggactggagcggtgtgagggcgagcaggacaagagattccattgctacgctagctggcgcaattccagcggcaccatcgagctggtgaagaagggctgttggctggacgatttcaactgttacgatagacaggagtgcgtggccaccgaggagaatcctcaggtgtatttttgctgttgcgagggcaacttctgcaatgagaggttcacccacctgccagaggctggaggaccagaggtgacctatgagccacctccaacaggaggaggaggctctggaggaggaggctccacccatacatgtccaccttgcccagctccagagctgctgggaggcccttccgtgttcctgtttccacccaagccaaaggacaccctgatgatctctaggaccccagaggtgacatgcgtggtggtggacgtgtcccacgaggaccccgaggtgaagtttaactggtacgtggatggcgtggaggtgcataatgctaagacaaagccaagggaggagcagtacaactccacctatcgggtggtgagcgtgctgacagtgctgcaccaggattggctgaacggcaaggagtataagtgtaaggtgagcaataaggctctgcctgccccaatcgagaagaccatctctaaggctaagggccagcccagagagcctcaggtgtacacactgcctccatcccgcgacgagctgaccaagaaccaggtgagcctgacatgcctggtgaagggcttctatcccagcgacatcgccgtggagtgggagtctaatggccagcctgagaacaattacaagaccacaccccctgtgctggacagcgatggctctttctttctgtattctaagctgaccgtggataagtcccggtggcagcagggcaacgtgttttcttgttccgtgatgcatgaggccctgcacaatcattacacacagaagagcctgtctctgtcccctggc

SEQ ID NO: 331 - DNA, 1035 bp, synthetic construct
  source 1..1035: mol_type = other DNA
gagaccagggagtgtatctactataacgccaattgggagctggagaggacaaaccagtccggactggagcggtgtgagggcgagcaggacaagagattccattgctacgctagctggcgcaattccagcggcaccatcgagctggtgaagaagggctgttggctggacgatttcaactgttacgatagacaggagtgcgtggccaccgaggagaatcctcaggtgtatttttgctgttgcgagggcaacttctgcaatgagaggttcacccacctgccagaggctggaggaccagaggtgacctatgagccacctccaacaggaggaggaggctctggaggaggaggctccggaggaggaggaacccatacatgtccaccttgcccagctccagagctgctgggaggcccttccgtgttcctgtttccacccaagccaaaggacaccctgatgatctctaggaccccagaggtgacatgcgtggtggtggacgtgtcccacgaggaccccgaggtgaagtttaactggtacgtggatggcgtggaggtgcataatgctaagacaaagccaagggaggagcagtacaactccacctatcgggtggtgagcgtgctgacagtgctgcaccaggattggctgaacggcaaggagtataagtgtaaggtgagcaataaggctctgcctgccccaatcgagaagaccatctctaaggctaagggccagcccagagagcctcaggtgtacacactgcctccatcccgcgacgagctgaccaagaaccaggtgagcctgacatgcctggtgaagggcttctatcccagcgacatcgccgtggagtgggagtctaatggccagcctgagaacaattacaagaccacaccccctgtgctggacagcgatggctctttctttctgtattctaagctgaccgtggataagtcccggtggcagcagggcaacgtgttttcttgttccgtgatgcatgaggccctgcacaatcattacacacagaagagcctgtctctgtcccctggc

SEQ ID NO: 332 - DNA, 1002 bp, synthetic construct
  source 1..1002: mol_type = other DNA
gagaccagggagtgtatctactataacgccaattgggagctggagaggacaaaccagtccggactggagcggtgtgagggagagcaggacaagagacagcattgctacgctagctggcgcaattccagcggcaccatcgagctggtgaagaagggctgttggctggacgatttcaactgttacgatagacaggagtgcgtggccaccgaggagaatcctcaggtgtatttttgctgttgcgagggcaacttctgcaatgagaggttcacccacctgccagaggctggaggaccagaggtgacctatgagccacctccaacaggaggaggaacccatacatgtccaccttgcccagctccagagctgctgggaggcccttccgtgttcctgtttccacccaagccaaaggacaccctgatgatctctaggaccccagaggtgacatgcgtggtggtggacgtgtcccacgaggaccccgaggtgaagtttaactggtacgtggatggcgtggaggtgcataatgctaagacaaagccaagggaggagcagtacaactccacctatcgggtggtgagcgtgctgacagtgctgcaccaggattggctgaacggcaaggagtataagtgtaaggtgagcaataaggctctgcctgccccaatcgagaagaccatctctaaggctaagggccagcccagagagcctcaggtgtacacactgcctccatcccgcgacgagctgaccaagaaccaggtgagcctgacatgcctggtgaagggcttctatcccagcgacatcgccgtggagtgggagtctaatggccagcctgagaacaattacaagaccacaccccctgtgctggacagcgatggctctttctttctgtattctaagctgaccgtggataagtcccggtggcagcagggcaacgtgttttcttgttccgtgatgcatgaggccctgcacaatcattacacacagaagagcctgtctctgtcccctggc

SEQ ID NO: 333 - DNA, 1023 bp, synthetic construct
  source 1..1023: mol_type = other DNA
gagaccagggagtgtatctactataacgccaattgggagctggagaggacaaaccagtccggactggagcggtgtgagggcgagcaggacaagagacagcattgctacgctagctggcgcaattccagcggcaccatcgagctggtgaagaagggctgttggctggacgatttcaactgttacgatagacaggagtgcgtggccaccgaggagaatcctcaggtgtatttttgctgttgcgagggcaacttctgcaatgagaggttcacccacctgccagaggctggaggaccagaggtgacctatgagccacctccaacaggaggaggaggctctggaggaggaggctccacccatacatgtccaccttgcccagctccagagctgctgggaggcccttccgtgttcctgtttccacccaagccaaaggacaccctgatgatctctaggaccccagaggtgacatgcgtggtggtggacgtgtcccacgaggaccccgaggtgaagtttaactggtacgtggatggcgtggaggtgcataatgctaagacaaagccaagggaggagcagtacaactccacctatcgggtggtgagcgtgctgacagtgctgcaccaggattggctgaacggcaaggagtataagtgtaaggtgagcaataaggctctgcctgccccaatcgagaagaccatctctaaggctaagggccagcccagagagcctcaggtgtacacactgcctccatcccgcgacgagctgaccaagaaccaggtgagcctgacatgcctggtgaagggcttctatcccagcgacatcgccgtggagtgggagtctaatggccagcctgagaacaattacaagaccacaccccctgtgctggacagcgatggctctttctttctgtattctaagctgaccgtggataagtcccggtggcagcagggcaacgtgttttcttgttccgtgatgcatgaggccctgcacaatcattacacacagaagagcctgtctctgtcccctggc

SEQ ID NO: 334 - DNA, 1023 bp, synthetic construct
  source 1..1023: mol_type = other DNA
gagaccagggagtgtatctactataacgccaattgggagctggagaggacaaaccagtccggactggagcggtgtgagggcgagcaggacaagagataccattgctacgctagctggcgcaattccagcggcaccatcgagctggtgaagaagggctgttggctggacgatttcaactgttacgatagacaggagtgcgtggccaccgaggagaatcctcaggtgtatttttgctgttgcgagggcaacttctgcaatgagaggttcacccacctgccagaggctggaggaccagaggtgacctatgagccacctccaacaggaggaggaggctctggaggaggaggctccacccatacatgtccaccttgcccagctccagagctgctgggaggcccttccgtgttcctgtttccacccaagccaaaggacaccctgatgatctctaggaccccagaggtgacatgcgtggtggtggacgtgtcccacgaggaccccgaggtgaagtttaactggtacgtggatggcgtggaggtgcataatgctaagacaaagccaagggaggagcagtacaactccacctatcgggtggtgagcgtgctgacagtgctgcaccaggattggctgaacggcaaggagtataagtgtaaggtgagcaataaggctctgcctgccccaatcgagaagaccatctctaaggctaagggccagcccagagagcctcaggtgtacacactgcctccatcccgcgacgagctgaccaagaaccaggtgagcctgacatgcctggtgaagggcttctatcccagcgacatcgccgtggagtgggagtctaatggccagcctgagaacaattacaagaccacaccccctgtgctggacagcgatggctctttctttctgtattctaagctgaccgtggataagtcccggtggcagcagggcaacgtgttttcttgttccgtgatgcatgaggccctgcacaatcattacacacagaagagcctgtctctgtcccctggc

SEQ ID NO: 335 - DNA, 1035 bp, synthetic construct
  source 1..1035: mol_type = other DNA
gagaccagggagtgtatctactataacgccaattgggagctggagaggacaaaccagtccggactggagcggtgtgagggcgagcaggacaagagatggcattgctacgctagctggcgcaattccagcggcaccatcgagctggtgaagaagggctgttggctggacgatttcaactgttacgatagacaggagtgcgtggccaccgaggagaatcctcaggtgtatttttgctgttgcgagggcaacttctgcaatgagaggttcacccacctgccagaggctggaggaccagaggtgacctatgagccacctccaacaggaggaggaggctctggaggaggaggctccggaggaggaggaacccatacatgtccaccttgcccagctccagagctgctgggaggcccttccgtgttcctgtttccacccaagccaaaggacaccctgatgatctctaggaccccagaggtgacatgcgtggtggtggacgtgtcccacgaggaccccgaggtgaagtttaactggtacgtggatggcgtggaggtgcataatgctaagacaaagccaagggaggagcagtacaactccacctatcgggtggtgagcgtgctgacagtgctgcaccaggattggctgaacggcaaggagtataagtgtaaggtgagcaataaggctctgcctgccccaatcgagaagaccatctctaaggctaagggccagcccagagagcctcaggtgtacacactgcctccatcccgcgacgagctgaccaagaaccaggtgagcctgacatgcctggtgaagggcttctatcccagcgacatcgccgtggagtgggagtctaatggccagcctgagaacaattacaagaccacaccccctgtgctggacagcgatggctctttctttctgtattctaagctgaccgtggataagtcccggtggcagcagggcaacgtgttttcttgttccgtgatgcatgaggccctgcacaatcattacacacagaagagcctgtctctgtcccctggc

SEQ ID NO: 336 - DNA, 1035 bp, synthetic construct
  source 1..1035: mol_type = other DNA
gagaccagggagtgtatctactataacgccaattgggagctggagaggacaaaccagtccggactggagcggtgtgagggcgagcaggacaagagagagcattgctacgctagctggcgcaattccagcggcaccatcgagctggtgaagaagggctgttggctggacgatttcaactgttacgatagacaggagtgcgtggccaccgaggagaatcctcaggtgtatttttgctgttgcgagggcaacttctgcaatgagaggttcacccacctgccagaggctggaggaccagaggtgacctatgagccacctccaacaggaggaggaggctctggaggaggaggctccggaggaggaggaacccatacatgtccaccttgcccagctccagagctgctgggaggcccttccgtgttcctgtttccacccaagccaaaggacaccctgatgatctctaggaccccagaggtgacatgcgtggtggtggacgtgtcccacgaggaccccgaggtgaagtttaactggtacgtggatggcgtggaggtgcataatgctaagacaaagccaagggaggagcagtacaactccacctatcgggtggtgagcgtgctgacagtgctgcaccaggattggctgaacggcaaggagtataagtgtaaggtgagcaataaggctctgcctgccccaatcgagaagaccatctctaaggctaagggccagcccagagagcctcaggtgtacacactgcctccatcccgcgacgagctgaccaagaaccaggtgagcctgacatgcctggtgaagggcttctatcccagcgacatcgccgtggagtgggagtctaatggccagcctgagaacaattacaagaccacaccccctgtgctggacagcgatggctctttctttctgtattctaagctgaccgtggataagtcccggtggcagcagggcaacgtgttttcttgttccgtgatgcatgaggccctgcacaatcattacacacagaagagcctgtctctgtcccctggc

SEQ ID NO: 337 - DNA, 1035 bp, synthetic construct
  source 1..1035: mol_type = other DNA
gagaccagggagtgtatctactataacgccaattgggagctggagaggacaaaccagtccggactggagcggtgtgagggcgagcaggacaagagaaagcattgctacgctagctggcgcaattccagcggcaccatcgagctggtgaagaagggctgttggctggacgatttcaactgttacgatagacaggagtgcgtggccaccgaggagaatcctcaggtgtatttttgctgttgcgagggcaacttctgcaatgagaggttcacccacctgccagaggctggaggaccagaggtgacctatgagccacctccaacaggaggaggaggctctggaggaggaggctccggaggaggaggaacccatacatgtccaccttgcccagctccagagctgctgggaggcccttccgtgttcctgtttccacccaagccaaaggacaccctgatgatctctaggaccccagaggtgacatgcgtggtggtggacgtgtcccacgaggaccccgaggtgaagtttaactggtacgtggatggcgtggaggtgcataatgctaagacaaagccaagggaggagcagtacaactccacctatcgggtggtgagcgtgctgacagtgctgcaccaggattggctgaacggcaaggagtataagtgtaaggtgagcaataaggctctgcctgccccaatcgagaagaccatctctaaggctaagggccagcccagagagcctcaggtgtacacactgcctccatcccgcgacgagctgaccaagaaccaggtgagcctgacatgcctggtgaagggcttctatcccagcgacatcgccgtggagtgggagtctaatggccagcctgagaacaattacaagaccacaccccctgtgctggacagcgatggctctttctttctgtattctaagctgaccgtggataagtcccggtggcagcagggcaacgtgttttcttgttccgtgatgcatgaggccctgcacaatcattacacacagaagagcctgtctctgtcccctggc

SEQ ID NO: 338 - DNA, 1035 bp, synthetic construct
  source 1..1035: mol_type = other DNA
gagaccagggagtgtatctactataacgccaattgggagctggagaggacaaaccagtccggactggagcggtgtgagggcgagcaggacaagagaatgcattgctacgctagctggcgcaattccagcggcaccatcgagctggtgaagaagggctgttggctggacgatttcaactgttacgatagacaggagtgcgtggccaccgaggagaatcctcaggtgtatttttgctgttgcgagggcaacttctgcaatgagaggttcacccacctgccagaggctggaggaccagaggtgacctatgagccacctccaacaggaggaggaggctctggaggaggaggctccggaggaggaggaacccatacatgtccaccttgcccagctccagagctgctgggaggcccttccgtgttcctgtttccacccaagccaaaggacaccctgatgatctctaggaccccagaggtgacatgcgtggtggtggacgtgtcccacgaggaccccgaggtgaagtttaactggtacgtggatggcgtggaggtgcataatgctaagacaaagccaagggaggagcagtacaactccacctatcgggtggtgagcgtgctgacagtgctgcaccaggattggctgaacggcaaggagtataagtgtaaggtgagcaataaggctctgcctgccccaatcgagaagaccatctctaaggctaagggccagcccagagagcctcaggtgtacacactgcctccatcccgcgacgagctgaccaagaaccaggtgagcctgacatgcctggtgaagggcttctatcccagcgacatcgccgtggagtgggagtctaatggccagcctgagaacaattacaagaccacaccccctgtgctggacagcgatggctctttctttctgtattctaagctgaccgtggataagtcccggtggcagcagggcaacgtgttttcttgttccgtgatgcatgaggccctgcacaatcattacacacagaagagcctgtctctgtcccctggc

SEQ ID NO: 339 - DNA, 1035 bp, synthetic construct; identical to SEQ ID NO: 319
  source 1..1035: mol_type = other DNA

SEQ ID NO: 340 - DNA, 1035 bp, synthetic construct
  source 1..1035: mol_type = other DNA
gagaccagggagtgtatctactataacgccaattgggagctggagaggacaaaccagtccggactggagcggtgtgagaacgagcaggacaagagataccattgctacgctagctggcgcaattccagcggcaccatcgagctggtgaagaagggctgttggctggacgatttcaactgttacgatagacaggagtgcgtggccaccgaggagaatcctcaggtgtatttttgctgttgcgagggcaacttctgcaatgagaggttcacccacctgccagaggctggaggaccagaggtgacctatgagccacctccaacaggaggaggaggctctggaggaggaggctccggaggaggaggaacccatacatgtccaccttgcccagctccagagctgctgggaggcccttccgtgttcctgtttccacccaagccaaaggacaccctgatgatctctaggaccccagaggtgacatgcgtggtggtggacgtgtcccacgaggaccccgaggtgaagtttaactggtacgtggatggcgtggaggtgcataatgctaagacaaagccaagggaggagcagtacaactccacctatcgggtggtgagcgtgctgacagtgctgcaccaggattggctgaacggcaaggagtataagtgtaaggtgagcaataaggctctgcctgccccaatcgagaagaccatctctaaggctaagggccagcccagagagcctcaggtgtacacactgcctccatcccgcgacgagctgaccaagaaccaggtgagcctgacatgcctggtgaagggcttctatcccagcgacatcgccgtggagtgggagtctaatggccagcctgagaacaattacaagaccacaccccctgtgctggacagcgatggctctttctttctgtattctaagctgaccgtggataagtcccggtggcagcagggcaacgtgttttcttgttccgtgatgcatgaggccctgcacaatcattacacacagaagagcctgtctctgtcccctggc

SEQ ID NO: 341 - DNA, 1035 bp, synthetic construct
  source 1..1035: mol_type = other DNA
gagaccagggagtgtatctactataacgccaattgggagctggagaggacaaaccagtccggactggagcggtgtgagcaggagcaggacaagagataccattgctacgctagctggcgcaattccagcggcaccatcgagctggtgaagaagggctgttggctggacgatttcaactgttacgatagacaggagtgcgtggccaccgaggagaatcctcaggtgtatttttgctgttgcgagggcaacttctgcaatgagaggttcacccacctgccagaggctggaggaccagaggtgacctatgagccacctccaacaggaggaggaggctctggaggaggaggctccggaggaggaggaacccatacatgtccaccttgcccagctccagagctgctgggaggcccttccgtgttcctgtttccacccaagccaaaggacaccctgatgatctctaggaccccagaggtgacatgcgtggtggtggacgtgtcccacgaggaccccgaggtgaagtttaactggtacgtggatggcgtggaggtgcataatgctaagacaaagccaagggaggagcagtacaactccacctatcgggtggtgagcgtgctgacagtgctgcaccaggattggctgaacggcaaggagtataagtgtaaggtgagcaataaggctctgcctgccccaatcgagaagaccatctctaaggctaagggccagcccagagagcctcaggtgtacacactgcctccatcccgcgacgagctgaccaagaaccaggtgagcctgacatgcctggtgaagggcttctatcccagcgacatcgccgtggagtgggagtctaatggccagcctgagaacaattacaagaccacaccccctgtgctggacagcgatggctctttctttctgtattctaagctgaccgtggataagtcccggtggcagcagggcaacgtgttttcttgttccgtgatgcatgaggccctgcacaatcattacacacagaagagcctgtctctgtcccctggc

SEQ ID NO: 342 - DNA, 1035 bp, synthetic construct
  source 1..1035: mol_type = other DNA
gagaccagggagtgtatctactataacgccaattgggagctggagaggacaaaccagtccggactggagcggtgtgagaaggagcaggacaagagataccattgctacgctagctggcgcaattccagcggcaccatcgagctggtgaagaagggctgttggctggacgatttcaactgttacgatagacaggagtgcgtggccaccgaggagaatcctcaggtgtatttttgctgttgcgagggcaacttctgcaatgagaggttcacccacctgccagaggctggaggaccagaggtgacctatgagccacctccaacaggaggaggaggctctggaggaggaggctccggaggaggaggaacccatacatgtccaccttgcccagctccagagctgctgggaggcccttccgtgttcctgtttccacccaagccaaaggacaccctgatgatctctaggaccccagaggtgacatgcgtggtggtggacgtgtcccacgaggaccccgaggtgaagtttaactggtacgtggatggcgtggaggtgcataatgctaagacaaagccaagggaggagcagtacaactccacctatcgggtggtgagcgtgctgacagtgctgcaccaggattggctgaacggcaaggagtataagtgtaaggtgagcaataaggctctgcctgccccaatcgagaagaccatctctaaggctaagggccagcccagagagcctcaggtgtacacactgcctccatcccgcgacgagctgaccaagaaccaggtgagcctgacatgcctggtgaagggcttctatcccagcgacatcgccgtggagtgggagtctaatggccagcctgagaacaattacaagaccacaccccctgtgctggacagcgatggctctttctttctgtattctaagctgaccgtggataagtcccggtggcagcagggcaacgtgttttcttgttccgtgatgcatgaggccctgcacaatcattacacacagaagagcctgtctctgtcccctggc

SEQ ID NO: 343 - DNA, 1035 bp, synthetic construct
  source 1..1035: mol_type = other DNA
gagaccagggagtgtatctactataacgccaattgggagctggagaggacaaaccagtccggactggagcggtgtgagaccgagcaggacaagagataccattgctacgctagctggcgcaattccagcggcaccatcgagctggtgaagaagggctgttggctggacgatttcaactgttacgatagacaggagtgcgtggccaccgaggagaatcctcaggtgtatttttgctgttgcgagggcaacttctgcaatgagaggttcacccacctgccagaggctggaggaccagaggtgacctatgagccacctccaacaggaggaggaggctctggaggaggaggctccggaggaggaggaacccatacatgtccaccttgcccagctccagagctgctgggaggcccttccgtgttcctgtttccacccaagccaaaggacaccctgatgatctctaggaccccagaggtgacatgcgtggtggtggacgtgtcccacgaggaccccgaggtgaagtttaactggtacgtggatggcgtggaggtgcataatgctaagacaaagccaagggaggagcagtacaactccacctatcgggtggtgagcgtgctgacagtgctgcaccaggattggctgaacggcaaggagtataagtgtaaggtgagcaataaggctctgcctgccccaatcgagaagaccatctctaaggctaagggccagcccagagagcctcaggtgtacacactgcctccatcccgcgacgagctgaccaagaaccaggtgagcctgacatgcctggtgaagggcttctatcccagcgacatcgccgtggagtgggagtctaatggccagcctgagaacaattacaagaccacaccccctgtgctggacagcgatggctctttctttctgtattctaagctgaccgtggataagtcccggtggcagcagggcaacgtgttttcttgttccgtgatgcatgaggccctgcacaatcattacacacagaagagcctgtctctgtcccctggc

SEQ ID NO: 344 - DNA, 1035 bp, synthetic construct
  source 1..1035: mol_type = other DNA
gagaccagggagtgtatctactataacgccaattgggagctggagaggacaaaccagtccggactggagcggtgtgagatggagcaggacaagagataccattgctacgctagctggcgcaattccagcggcaccatcgagctggtgaagaagggctgttggctggacgatttcaactgttacgatagacaggagtgcgtggccaccgaggagaatcctcaggtgtatttttgctgttgcgagggcaacttctgcaatgagaggttcacccacctgccagaggctggaggaccagaggtgacctatgagccacctccaacaggaggaggaggctctggaggaggaggctccggaggaggaggaacccatacatgtccaccttgcccagctccagagctgctgggaggcccttccgtgttcctgtttccacccaagccaaaggacaccctgatgatctctaggaccccagaggtgacatgcgtggtggtggacgtgtcccacgaggaccccgaggtgaagtttaactggtacgtggatggcgtggaggtgcataatgctaagacaaagccaagggaggagcagtacaactccacctatcgggtggtgagcgtgctgacagtgctgcaccaggattggctgaacggcaaggagtataagtgtaaggtgagcaataaggctctgcctgccccaatcgagaagaccatctctaaggctaagggccagcccagagagcctcaggtgtacacactgcctccatcccgcgacgagctgaccaagaaccaggtgagcctgacatgcctggtgaagggcttctatcccagcgacatcgccgtggagtgggagtctaatggccagcctgagaacaattacaagaccacaccccctgtgctggacagcgatggctctttctttctgtattctaagctgaccgtggataagtcccggtggcagcagggcaacgtgttttcttgttccgtgatgcatgaggccctgcacaatcattacacacagaagagcctgtctctgtcccctggc

SEQ ID NO: 345 - DNA, 1035 bp, synthetic construct
  source 1..1035: mol_type = other DNA
gagaccagggagtgtatctactataacgccaattgggagctggagaggacaaaccagtccggactggagcggtgtgagggcgagcaggacaagagataccattgctacgctagctggcgcaattccagcggcaccatcgagctggtgaagaagggctgttggctggacgatttcaactgttacgatagacaggagtgcgtggccagggaggagaatcctcaggtgtatttttgctgttgcgagggcaacttctgcaatgagaggttcacccacctgccagaggctggaggaccagaggtgacctatgagccacctccaacaggaggaggaggctctggaggaggaggctccggaggaggaggaacccatacatgtccaccttgcccagctccagagctgctgggaggcccttccgtgttcctgtttccacccaagccaaaggacaccctgatgatctctaggaccccagaggtgacatgcgtggtggtggacgtgtcccacgaggaccccgaggtgaagtttaactggtacgtggatggcgtggaggtgcataatgctaagacaaagccaagggaggagcagtacaactccacctatcgggtggtgagcgtgctgacagtgctgcaccaggattggctgaacggcaaggagtataagtgtaaggtgagcaataaggctctgcctgccccaatcgagaagaccatctctaaggctaagggccagcccagagagcctcaggtgtacacactgcctccatcccgcgacgagctgaccaagaaccaggtgagcctgacatgcctggtgaagggcttctatcccagcgacatcgccgtggagtgggagtctaatggccagcctgagaacaattacaagaccacaccccctgtgctggacagcgatggctctttctttctgtattctaagctgaccgtggataagtcccggtggcagcagggcaacgtgttttcttgttccgtgatgcatgaggccctgcacaatcattacacacagaagagcctgtctctgtcccctggc

SEQ ID NO: 346 - DNA, 1035 bp, synthetic construct
  source 1..1035: mol_type = other DNA
gagaccagggagtgtatctactataacgccaattgggagctggagaggacaaaccagtccggactggagcggtgtgagggcgagcaggacaagagataccattgctacgctagctggcgcaattccagcggcaccatcgagctggtgaagaagggctgttggctggacgatttcaactgttacgatagacaggagtgcgtggcctacgaggagaatcctcaggtgtatttttgctgttgcgagggcaacttctgcaatgagaggttcacccacctgccagaggctggaggaccagaggtgacctatgagccacctccaacaggaggaggaggctctggaggaggaggctccggaggaggaggaacccatacatgtccaccttgcccagctccagagctgctgggaggcccttccgtgttcctgtttccacccaagccaaaggacaccctgatgatctctaggaccccagaggtgacatgcgtggtggtggacgtgtcccacgaggaccccgaggtgaagtttaactggtacgtggatggcgtggaggtgcataatgctaagacaaagccaagggaggagcagtacaactccacctatcgggtggtgagcgtgctgacagtgctgcaccaggattggctgaacggcaaggagtataagtgtaaggtgagcaataaggctctgcctgccccaatcgagaagaccatctctaaggctaagggccagcccagagagcctcaggtgtacacactgcctccatcccgcgacgagctgaccaagaaccaggtgagcctgacatgcctggtgaagggcttctatcccagcgacatcgccgtggagtgggagtctaatggccagcctgagaacaattacaagaccacaccccctgtgctggacagcgatggctctttctttctgtattctaagctgaccgtggataagtcccggtggcagcagggcaacgtgttttcttgttccgtgatgcatgaggccctgcacaatcattacacacagaagagcctgtctctgtcccctggc

SEQ ID NO: 347 - DNA, 1035 bp, synthetic construct
  source 1..1035: mol_type = other DNA
gagaccagggagtgtatctactataacgccaattgggagctggagaggacaaaccagtccggactggagcggtgtgagggcgagcaggacaagagataccattgctacgctagctggcgcaattccagcggcaccatcgagctggtgaagaagggctgttggctggacgatttcaactgttacgatagacaggagtgcgtggcctgggaggagaatcctcaggtgtatttttgctgttgcgagggcaacttctgcaatgagaggttcacccacctgccagaggctggaggaccagaggtgacctatgagccacctccaacaggaggaggaggctctggaggaggaggctccggaggaggaggaacccatacatgtccaccttgcccagctccagagctgctgggaggcccttccgtgttcctgtttccacccaagccaaaggacaccctgatgatctctaggaccccagaggtgacatgcgtggtggtggacgtgtcccacgaggaccccgaggtgaagtttaactggtacgtggatggcgtggaggtgcataatgctaagacaaagccaagggaggagcagtacaactccacctatcgggtggtgagcgtgctgacagtgctgcaccaggattggctgaacggcaaggagtataagtgtaaggtgagcaataaggctctgcctgccccaatcgagaagaccatctctaaggctaagggccagcccagagagcctcaggtgtacacactgcctccatcccgcgacgagctgaccaagaaccaggtgagcctgacatgcctggtgaagggcttctatcccagcgacatcgccgtggagtgggagtctaatggccagcctgagaacaattacaagaccacaccccctgtgctggacagcgatggctctttctttctgtattctaagctgaccgtggataagtcccggtggcagcagggcaacgtgttttcttgttccgtgatgcatgaggccctgcacaatcattacacacagaagagcctgtctctgtcccctggc

SEQ ID NO: 348 - DNA, 1035 bp, synthetic construct
  source 1..1035: mol_type = other DNA
gagaccagggagtgtatctactataacgccaattgggaggaggagaggacaaaccagtccggactggagcggtgtgagggcgagcaggacaagagataccattgctacgctagctggcgcaattccagcggcaccatcgagctggtgaagaagggctgttggctggacgatttcaactgttacgatagacaggagtgcgtggccaccgaggagaatcctcaggtgtatttttgctgttgcgagggcaacttctgcaatgagaggttcacccacctgccagaggctggaggaccagaggtgacctatgagccacctccaacaggaggaggaggctctggaggaggaggctccggaggaggaggaacccatacatgtccaccttgcccagctccagagctgctgggaggcccttccgtgttcctgtttccacccaagccaaaggacaccctgatgatctctaggaccccagaggtgacatgcgtggtggtggacgtgtcccacgaggaccccgaggtgaagtttaactggtacgtggatggcgtggaggtgcataatgctaagacaaagccaagggaggagcagtacaactccacctatcgggtggtgagcgtgctgacagtgctgcaccaggattggctgaacggcaaggagtataagtgtaaggtgagcaataaggctctgcctgccccaatcgagaagaccatctctaaggctaagggccagcccagagagcctcaggtgtacacactgcctccatcccgcgacgagctgaccaagaaccaggtgagcctgacatgcctggtgaagggcttctatcccagcgacatcgccgtggagtgggagtctaatggccagcctgagaacaattacaagaccacaccccctgtgctggacagcgatggctctttctttctgtattctaagctgaccgtggataagtcccggtggcagcagggcaacgtgttttcttgttccgtgatgcatgaggccctgcacaatcattacacacagaagagcctgtctctgtcccctggc

SEQ ID NO: 349 - DNA, 1035 bp, synthetic construct
  source 1..1035: mol_type = other DNA
gagaccagggagtgtatctactataacgccaattgggagcacgagaggacaaaccagtccggactggagcggtgtgagggcgagcaggacaagagataccattgctacgctagctggcgcaattccagcggcaccatcgagctggtgaagaagggctgttggctggacgatttcaactgttacgatagacaggagtgcgtggccaccgaggagaatcctcaggtgtatttttgctgttgcgagggcaacttctgcaatgagaggttcacccacctgccagaggctggaggaccagaggtgacctatgagccacctccaacaggaggaggaggctctggaggaggaggctccggaggaggaggaacccatacatgtccaccttgcccagctccagagctgctgggaggcccttccgtgttcctgtttccacccaagccaaaggacaccctgatgatctctaggaccccagaggtgacatgcgtggtggtggacgtgtcccacgaggaccccgaggtgaagtttaactggtacgtggatggcgtggaggtgcataatgctaagacaaagccaagggaggagcagtacaactccacctatcgggtggtgagcgtgctgacagtgctgcaccaggattggctgaacggcaaggagtataagtgtaaggtgagcaataaggctctgcctgccccaatcgagaagaccatctctaaggctaagggccagcccagagagcctcaggtgtacacactgcctccatcccgcgacgagctgaccaagaaccaggtgagcctgacatgcctggtgaagggcttctatcccagcgacatcgccgtggagtgggagtctaatggccagcctgagaacaattacaagaccacaccccctgtgctggacagcgatggctctttctttctgtattctaagctgaccgtggataagtcccggtggcagcagggcaacgtgttttcttgttccgtgatgcatgaggccctgcacaatcattacacacagaagagcctgtctctgtcccctggc

SEQ ID NO: 350 - DNA, 1035 bp, synthetic construct
  source 1..1035: mol_type = other DNA
gagaccagggagtgtatctactataacgccaattgggagtccgagaggacaaaccagtccggactggagcggtgtgagggcgagcaggacaagagataccattgctacgctagctggcgcaattccagcggcaccatcgagctggtgaagaagggctgttggctggacgatttcaactgttacgatagacaggagtgcgtggccaccgaggagaatcctcaggtgtatttttgctgttgcgagggcaacttctgcaatgagaggttcacccacctgccagaggctggaggaccagaggtgacctatgagccacctccaacaggaggaggaggctctggaggaggaggctccggaggaggaggaacccatacatgtccaccttgcccagctccagagctgctgggaggcccttccgtgttcctgtttccacccaagccaaaggacaccctgatgatctctaggaccccagaggtgacatgcgtggtggtggacgtgtcccacgaggaccccgaggtgaagtttaactggtacgtggatggcgtggaggtgcataatgctaagacaaagccaagggaggagcagtacaactccacctatcgggtggtgagcgtgctgacagtgctgcaccaggattggctgaacggcaaggagtataagtgtaaggtgagcaataaggctctgcctgccccaatcgagaagaccatctctaaggctaagggccagcccagagagcctcaggtgtacacactgcctccatcccgcgacgagctgaccaagaaccaggtgagcctgacatgcctggtgaagggcttctatcccagcgacatcgccgtggagtgggagtctaatggccagcctgagaacaattacaagaccacaccccctgtgctggacagcgatggctctttctttctgtattctaagctgaccgtggataagtcccggtggcagcagggcaacgtgttttcttgttccgtgatgcatgaggccctgcacaatcattacacacagaagagcctgtctctgtcccctggc

SEQ ID NO: 351 - DNA, 1035 bp, synthetic construct
  source 1..1035: mol_type = other DNA
gagaccagggagtgtatctactataacgccaattgggagctggagaggacaaaccagtccggactggagcggtgtgagggcgagcaggacaagagataccattgctacgctagctggcgcaattccagcggcaccatcgagctggtgaagaagggctgttggtacgacgatttcaactgttacgatagacaggagtgcgtggccaccgaggagaatcctcaggtgtatttttgctgttgcgagggcaacttctgcaatgagaggttcacccacctgccagaggctggaggaccagaggtgacctatgagccacctccaacaggaggaggaggctctggaggaggaggctccggaggaggaggaacccatacatgtccaccttgcccagctccagagctgctgggaggcccttccgtgttcctgtttccacccaagccaaaggacaccctgatgatctctaggaccccagaggtgacatgcgtggtggtggacgtgtcccacgaggaccccgaggtgaagtttaactggtacgtggatggcgtggaggtgcataatgctaagacaaagccaagggaggagcagtacaactccacctatcgggtggtgagcgtgctgacagtgctgcaccaggattggctgaacggcaaggagtataagtgtaaggtgagcaataaggctctgcctgccccaatcgagaagaccatctctaaggctaagggccagcccagagagcctcaggtgtacacactgcctccatcccgcgacgagctgaccaagaaccaggtgagcctgacatgcctggtgaagggcttctatcccagcgacatcgccgtggagtgggagtctaatggccagcctgagaacaattacaagaccacaccccctgtgctggacagcgatggctctttctttctgtattctaagctgaccgtggataagtcccggtggcagcagggcaacgtgttttcttgttccgtgatgcatgaggccctgcacaatcattacacacagaagagcctgtctctgtcccctggc

SEQ ID NO: 352 - DNA, 1035 bp, synthetic construct
  source 1..1035: mol_type = other DNA
gagaccagggagtgtatctactataacgccaattgggagctggagaggacaaaccagtccggactggagcggtgtgagggcgagcaggacaagagataccattgctacgctagctggcgcaattccagcggcaccatcgagctggtgaagaagggctgttggcaggacgatttcaactgttacgatagacaggagtgcgtggccaccgaggagaatcctcaggtgtatttttgctgttgcgagggcaacttctgcaatgagaggttcacccacctgccagaggctggaggaccagaggtgacctatgagccacctccaacaggaggaggaggctctggaggaggaggctccggaggaggaggaacccatacatgtccaccttgcccagctccagagctgctgggaggcccttccgtgttcctgtttccacccaagccaaaggacaccctgatgatctctaggaccccagaggtgacatgcgtggtggtggacgtgtcccacgaggaccccgaggtgaagtttaactggtacgtggatggcgtggaggtgcataatgctaagacaaagccaagggaggagcagtacaactccacctatcgggtggtgagcgtgctgacagtgctgcaccaggattggctgaacggcaaggagtataagtgtaaggtgagcaataaggctctgcctgccccaatcgagaagaccatctctaaggctaagggccagcccagagagcctcaggtgtacacactgcctccatcccgcgacgagctgaccaagaaccaggtgagcctgacatgcctggtgaagggcttctatcccagcgacatcgccgtggagtgggagtctaatggccagcctgagaacaattacaagaccacaccccctgtgctggacagcgatggctctttctttctgtattctaagctgaccgtggataagtcccggtggcagcagggcaacgtgttttcttgttccgtgatgcatgaggccctgcacaatcattacacacagaagagcctgtctctgtcccctggc

SEQ ID NO: 353 - DNA, 1035 bp, synthetic construct
  source 1..1035: mol_type = other DNA
gagaccagggagtgtatctactataacgccaattgggagctggagaggacaaaccagtccggactggagcggtgtgagggcgagcaggacaagagataccattgctacgctagctggcgcaattccagcggcaccatcgagctggtgaagaagggctgttggatggacgatttcaactgttacgatagacaggagtgcgtggccaccgaggagaatcctcaggtgtatttttgctgttgcgagggcaacttctgcaatgagaggttcacccacctgccagaggctggaggaccagaggtgacctatgagccacctccaacaggaggaggaggctctggaggaggaggctccggaggaggaggaacccatacatgtccaccttgcccagctccagagctgctgggaggcccttccgtgttcctgtttccacccaagccaaaggacaccctgatgatctctaggaccccagaggtgacatgcgtggtggtggacgtgtcccacgaggaccccgaggtgaagtttaactggtacgtggatggcgtggaggtgcataatgctaagacaaagccaagggaggagcagtacaactccacctatcgggtggtgagcgtgctgacagtgctgcaccaggattggctgaacggcaaggagtataagtgtaaggtgagcaataaggctctgcctgccccaatcgagaagaccatctctaaggctaagggccagcccagagagcctcaggtgtacacactgcctccatcccgcgacgagctgaccaagaaccaggtgagcctgacatgcctggtgaagggcttctatcccagcgacatcgccgtggagtgggagtctaatggccagcctgagaacaattacaagaccacaccccctgtgctggacagcgatggctctttctttctgtattctaagctgaccgtggataagtcccggtggcagcagggcaacgtgttttcttgttccgtgatgcatgaggccctgcacaatcattacacacagaagagcctgtctctgtcccctggc

SEQ ID NO: 354 - DNA, 1035 bp, synthetic construct
  source 1..1035: mol_type = other DNA
gagaccagggagtgtatctactataacgccaattgggagctggagaggacaaaccagtccggactggagcggtgtgagggcgagcaggacaagagataccattgctacgctagctggcgcaattccagcggcaccatcgagctggtgaagaagggctgttggatcgacgatttcaactgttacgatagacaggagtgcgtggccaccgaggagaatcctcaggtgtatttttgctgttgcgagggcaacttctgcaatgagaggttcacccacctgccagaggctggaggaccagaggtgacctatgagccacctccaacaggaggaggaggctctggaggaggaggctccggaggaggaggaacccatacatgtccaccttgcccagctccagagctgctgggaggcccttccgtgttcctgtttccacccaagccaaaggacaccctgatgatctctaggaccccagaggtgacatgcgtggtggtggacgtgtcccacgaggaccccgaggtgaagtttaactggtacgtggatggcgtggaggtgcataatgctaagacaaagccaagggaggagcagtacaactccacctatcgggtggtgagcgtgctgacagtgctgcaccaggattggctgaacggcaaggagtataagtgtaaggtgagcaataaggctctgcctgccccaatcgagaagaccatctctaaggctaagggccagcccagagagcctcaggtgtacacactgcctccatcccgcgacgagctgaccaagaaccaggtgagcctgacatgcctggtgaagggcttctatcccagcgacatcgccgtggagtgggagtctaatggccagcctgagaacaattacaagaccacaccccctgtgctggacagcgatggctctttctttctgtattctaagctgaccgtggataagtcccggtggcagcagggcaacgtgttttcttgttccgtgatgcatgaggccctgcacaatcattacacacagaagagcctgtctctgtcccctggc

SEQ ID NO: 355 - DNA, 1035 bp, synthetic construct
  source 1..1035: mol_type = other DNA
gagaccagggagtgtatctactataacgccaattgggagctggagaggacaaaccagtccggactggagcggtgtgagggcgagcaggacaagagatggcattgctacgctagctggcgcaattccagcggcaccatcgagctggtgaagaagggctgttggctggacgatttcaactgttacgatagacaggagtgcgtggccaccgaggagaatcctcaggtgtatttttgctgttgcgagggcaacttctgcaatgagaggttcacccacctgccagaggctggaggaccagaggtgacctatgagccacctccaacaggaggaggaggctctggaggaggaggctccggaggaggaggaacccatacatgtccaccttgcccagctccagagctgctgggaggcccttccgtgttcctgtttccacccaagccaaaggacaccctgtacatctctaggaccccagaggtgacatgcgtggtggtggacgtgtcccacgaggaccccgaggtgaagtttaactggtacgtggatggcgtggaggtgcataatgctaagacaaagccaagggaggagcagtacaactccacctatcgggtggtgagcgtgctgacagtgctgcaccaggattggctgaacggcaaggagtataagtgtaaggtgagcaataaggctctgcctgccccaatcgagaagaccatctctaaggctaagggccagcccagagagcctcaggtgtacacactgcctccatcccgcgacgagctgaccaagaaccaggtgagcctgacatgcctggtgaagggcttctatcccagcgacatcgccgtggagtgggagtctaatggccagcctgagaacaattacaagaccacaccccctgtgctggacagcgatggctctttctttctgtattctaagctgaccgtggataagtcccggtggcagcagggcaacgtgttttcttgttccgtgatgcatgaggccctgcacaatcattacacacagaagagcctgtctctgtcccctggc

SEQ ID NO: 356 - DNA, 1050 bp, synthetic construct
  source 1..1050: mol_type = other DNA
gagaccagggagtgtatctactataacgccaattgggagctggagaggacaaaccagtccggactggagcggtgtgagggcgagcaggacaagagatggcattgctacgctagctggcgcaattccagcggcaccatcgagctggtgaagaagggctgttggctggacgatttcaactgttacgatagacaggagtgcgtggccaccgaggagaatcctcaggtgtatttttgctgttgcgagggcaacttctgcaatgagaggttcacccacctgccagaggctggaggaccagaggtgacctatgagccacctccaacaggaggcggcggctccggcggaggaggctctggaggaggaggctccggaggaggaggaacccatacatgtccaccttgcccagctccagagctgctgggaggcccttccgtgttcctgtttccacccaagccaaaggacaccctgatgatctctaggaccccagaggtgacatgcgtggtggtggacgtgtcccacgaggaccccgaggtgaagtttaactggtacgtggatggcgtggaggtgcataatgctaagacaaagccaagggaggagcagtacaactccacctatcgggtggtgagcgtgctgacagtgctgcaccaggattggctgaacggcaaggagtataagtgtaaggtgagcaataaggctctgcctgccccaatcgagaagaccatctctaaggctaagggccagcccagagagcctcaggtgtacacactgcctccatcccgcgacgagctgaccaagaaccaggtgagcctgacatgcctggtgaagggcttctatcccagcgacatcgccgtggagtgggagtctaatggccagcctgagaacaattacaagaccacaccccctgtgctggacagcgatggctctttctttctgtattctaagctgaccgtggataagtcccggtggcagcagggcaacgtgttttcttgttccgtgatgcatgaggccctgcacaatcattacacacagaagagcctgtctctgtcccctggc

SEQ ID NO: 357 - DNA, 1050 bp, synthetic construct
  source 1..1050: mol_type = other DNA
gagaccagggagtgtatctactataacgccaattgggagctggagaggacaaaccagtccggactggagcggtgtgagggcgagcaggacaagagatggcattgctacgctagctggcgcaattccagcggcaccatcgagctggtgaagaagggctgttggctggacgatttcaactgttacgatagacaggagtgcgtggccaccgaggagaatcctcaggtgtatttttgctgttgcgagggcaacttctgcaatgagaggttcacccacctgccagaggctggaggaccagaggtgacctatgagccacctccaacaggaggcggcggctccggcggaggaggctctggaggaggaggctccggaggaggaggaacccatacatgtccaccttgcccagctccagagctgctgggaggcccttccgtgttcctgtttccacccaagccaaaggacaccctgtacatctctaggaccccagaggtgacatgcgtggtggtggacgtgtcccacgaggaccccgaggtgaagtttaactggtacgtggatggcgtggaggtgcataatgctaagacaaagccaagggaggagcagtacaactccacctatcgggtggtgagcgtgctgacagtgctgcaccaggattggctgaacggcaaggagtataagtgtaaggtgagcaataaggctctgcctgccccaatcgagaagaccatctctaaggctaagggccagcccagagagcctcaggtgtacacactgcctccatcccgcgacgagctgaccaagaaccaggtgagcctgacatgcctggtgaagggcttctatcccagcgacatcgccgtggagtgggagtctaatggccagcctgagaacaattacaagaccacaccccctgtgctggacagcgatggctctttctttctgtattctaagctgaccgtggataagtcccggtggcagcagggcaacgtgttttcttgttccgtgatgcatgaggccctgcacaatcattacacacagaagagcctgtctctgtcccctggc

SEQ ID NO: 358 - DNA, 1050 bp, synthetic construct
  source 1..1050: mol_type = other DNA
gagaccagggagtgtatctactataacgccaattgggagctggagaggacaaaccagtccggactggagcggtgtgagggcgagcaggacaagagatggcattgctacgctagctggcgcaattccagcggcaccatcgagctggtgaagaagggctgttggctggacgatttcaactgttacgatagacaggagtgcgtggccaccgaggagaatcctcaggtgtatttttgctgttgcgagggcaacttctgcaatgagaggttcacccacctgccagaggctggaggaccagaggtgacctatgagccacctccaacaggaggcggcggctccggcggaggaggctctggaggaggaggctccggaggaggaggaacccatacatgtccaccttgcccagctccagagctgctgggaggcccttccgtgttcctgtttccacccaagccaaaggacaccctgtacatcaccagggagccagaggtgacatgcgtggtggtggacgtgtcccacgaggaccccgaggtgaagtttaactggtacgtggatggcgtggaggtgcataatgctaagacaaagccaagggaggagcagtacaactccacctatcgggtggtgagcgtgctgacagtgctgcaccaggattggctgaacggcaaggagtataagtgtaaggtgagcaataaggctctgcctgccccaatcgagaagaccatctctaaggctaagggccagcccagagagcctcaggtgtacacactgcctccatcccgcgacgagctgaccaagaaccaggtgagcctgacatgcctggtgaagggcttctatcccagcgacatcgccgtggagtgggagtctaatggccagcctgagaacaattacaagaccacaccccctgtgctggacagcgatggctctttctttctgtattctaagctgaccgtggataagtcccggtggcagcagggcaacgtgttttcttgttccgtgatgcatgaggccctgcacaatcattacacacagaagagcctgtctctgtcccctggc

SEQ ID NO: 359 - DNA, 1050 bp, synthetic construct
  source 1..1050: mol_type = other DNA
gagaccagggagtgtatctactataacgccaattgggagctggagaggacaaaccagtccggactggagcggtgtgaggacgagcaggacaagagatggcattgctacgctagctggcgcaattccagcggcaccatcgagctggtgaagaagggctgttggctggacgatttcaactgttacgatagacaggagtgcgtggccaccgaggagaatcctcaggtgtatttttgctgttgcgagggcaacttctgcaatgagaggttcacccacctgccagaggctggaggaccagaggtgacctatgagccacctccaacaggaggcggcggctccggcggaggaggctctggaggaggaggctccggaggaggaggaacccatacatgtccaccttgcccagctccagagctgctgggaggcccttccgtgttcctgtttccacccaagccaaaggacaccctgatgatctctaggaccccagaggtgacatgcgtggtggtggacgtgtcccacgaggaccccgaggtgaagtttaactggtacgtggatggcgtggaggtgcataatgctaagacaaagccaagggaggagcagtacaactccacctatcgggtggtgagcgtgctgacagtgctgcaccaggattggctgaacggcaaggagtataagtgtaaggtgagcaataaggctctgcctgccccaatcgagaagaccatctctaaggctaagggccagcccagagagcctcaggtgtacacactgcctccatcccgcgacgagctgaccaagaaccaggtgagcctgacatgcctggtgaagggcttctatcccagcgacatcgccgtggagtgggagtctaatggccagcctgagaacaattacaagaccacaccccctgtgctggacagcgatggctctttctttctgtattctaagctgaccgtggataagtcccggtggcagcagggcaacgtgttttcttgttccgtgatgcatgaggccctgcacaatcattacacacagaagagcctgtctctgtcccctggc

SEQ ID NO: 360 - DNA, 1050 bp, synthetic construct
  source 1..1050: mol_type = other DNA
gagaccagggagtgtatctactataacgccaattgggagctggagaggacaaaccagtccggactggagcggtgtgaggaggagcaggacaagagatggcattgctacgctagctggcgcaattccagcggcaccatcgagctggtgaagaagggctgttggctggacgatttcaactgttacgatagacaggagtgcgtggccaccgaggagaatcctcaggtgtatttttgctgttgcgagggcaacttctgcaatgagaggttcacccacctgccagaggctggaggaccagaggtgacctatgagccacctccaacaggaggcggcggctccggcggaggaggctctggaggaggaggctccggaggaggaggaacccatacatgtccaccttgcccagctccagagctgctgggaggcccttccgtgttcctgtttccacccaagccaaaggacaccctgatgatctctaggaccccagaggtgacatgcgtggtggtggacgtgtcccacgaggaccccgaggtgaagtttaactggtacgtggatggcgtggaggtgcataatgctaagacaaagccaagggaggagcagtacaactccacctatcgggtggtgagcgtgctgacagtgctgcaccaggattggctgaacggcaaggagtataagtgtaaggtgagcaataaggctctgcctgccccaatcgagaagaccatctctaaggctaagggccagcccagagagcctcaggtgtacacactgcctccatcccgcgacgagctgaccaagaaccaggtgagcctgacatgcctggtgaagggcttctatcccagcgacatcgccgtggagtgggagtctaatggccagcctgagaacaattacaagaccacaccccctgtgctggacagcgatggctctttctttctgtattctaagctgaccgtggataagtcccggtggcagcagggcaacgtgttttcttgttccgtgatgcatgaggccctgcacaatcattacacacagaagagcctgtctctgtcccctggc

SEQ ID NO: 361 - DNA, 1050 bp, synthetic construct
  source 1..1050: mol_type = other DNA
gagaccagggagtgtatctactataacgccaattgggagctggagaggacaaaccagtccggactggagcggtgtgagaacgagcaggacaagagatggcattgctacgctagctggcgcaattccagcggcaccatcgagctggtgaagaagggctgttggctggacgatttcaactgttacgatagacaggagtgcgtggccaccgaggagaatcctcaggtgtatttttgctgttgcgagggcaacttctgcaatgagaggttcacccacctgccagaggctggaggaccagaggtgacctatgagccacctccaacaggaggcggcggctccggcggaggaggctctggaggaggaggctccggaggaggaggaacccatacatgtccaccttgcccagctccagagctgctgggaggcccttccgtgttcctgtttccacccaagccaaaggacaccctgatgatctctaggaccccagaggtgacatgcgtggtggtggacgtgtcccacgaggaccccgaggtgaagtttaactggtacgtggatggcgtggaggtgcataatgctaagacaaagccaagggaggagcagtacaactccacctatcgggtggtgagcgtgctgacagtgctgcaccaggattggctgaacggcaaggagtataagtgtaaggtgagcaataaggctctgcctgccccaatcgagaagaccatctctaaggctaagggccagcccagagagcctcaggtgtacacactgcctccatcccgcgacgagctgaccaagaaccaggtgagcctgacatgcctggtgaagggcttctatcccagcgacatcgccgtggagtgggagtctaatggccagcctgagaacaattacaagaccacaccccctgtgctggacagcgatggctctttctttctgtattctaagctgaccgtggataagtcccggtggcagcagggcaacgtgttttcttgttccgtgatgcatgaggccctgcacaatcattacacacagaagagcctgtctctgtcccctggc

SEQ ID NO: 362 - DNA, 1050 bp, synthetic construct
  source 1..1050: mol_type = other DNA
gagaccagggagtgtatctactataacgccaattgggagctggagaggacaaaccagtccggactggagcggtgtgagcaggagcaggacaagagatggcattgctacgctagctggcgcaattccagcggcaccatcgagctggtgaagaagggctgttggctggacgatttcaactgttacgatagacaggagtgcgtggccaccgaggagaatcctcaggtgtatttttgctgttgcgagggcaacttctgcaatgagaggttcacccacctgccagaggctggaggaccagaggtgacctatgagccacctccaacaggaggcggcggctccggcggaggaggctctggaggaggaggctccggaggaggaggaacccatacatgtccaccttgcccagctccagagctgctgggaggcccttccgtgttcctgtttccacccaagccaaaggacaccctgatgatctctaggaccccagaggtgacatgcgtggtggtggacgtgtcccacgaggaccccgaggtgaagtttaactggtacgtggatggcgtggaggtgcataatgctaagacaaagccaagggaggagcagtacaactccacctatcgggtggtgagcgtgctgacagtgctgcaccaggattggctgaacggcaaggagtataagtgtaaggtgagcaataaggctctgcctgccccaatcgagaagaccatctctaaggctaagggccagcccagagagcctcaggtgtacacactgcctccatcccgcgacgagctgaccaagaaccaggtgagcctgacatgcctggtgaagggcttctatcccagcgacatcgccgtggagtgggagtctaatggccagcctgagaacaattacaagaccacaccccctgtgctggacagcgatggctctttctttctgtattctaagctgaccgtggataagtcccggtggcagcagggcaacgtgttttcttgttccgtgatgcatgaggccctgcacaatcattacacacagaagagcctgtctctgtcccctggc

SEQ ID NO: 363 - DNA, 1050 bp, synthetic construct
  source 1..1050: mol_type = other DNA
gagaccagggagtgtatctactataacgccaattgggagctggagaggacaaaccagtccggactggagcggtgtgagaccgagcaggacaagagatggcattgctacgctagctggcgcaattccagcggcaccatcgagctggtgaagaagggctgttggctggacgatttcaactgttacgatagacaggagtgcgtggccaccgaggagaatcctcaggtgtatttttgctgttgcgagggcaacttctgcaatgagaggttcacccacctgccagaggctggaggaccagaggtgacctatgagccacctccaacaggaggcggcggctccggcggaggaggctctggaggaggaggctccggaggaggaggaacccatacatgtccaccttgcccagctccagagctgctgggaggcccttccgtgttcctgtttccacccaagccaaaggacaccctgatgatctctaggaccccagaggtgacatgcgtggtggtggacgtgtcccacgaggaccccgaggtgaagtttaactggtacgtggatggcgtggaggtgcataatgctaagacaaagccaagggaggagcagtacaactccacctatcgggtggtgagcgtgctgacagtgctgcaccaggattggctgaacggcaaggagtataagtgtaaggtgagcaataaggctctgcctgccccaatcgagaagaccatctctaaggctaagggccagcccagagagcctcaggtgtacacactgcctccatcccgcgacgagctgaccaagaaccaggtgagcctgacatgcctggtgaagggcttctatcccagcgacatcgccgtggagtgggagtctaatggccagcctgagaacaattacaagaccacaccccctgtgctggacagcgatggctctttctttctgtattctaagctgaccgtggataagtcccggtggcagcagggcaacgtgttttcttgttccgtgatgcatgaggccctgcacaatcattacacacagaagagcctgtctctgtcccctggc

SEQ ID NO: 364 - DNA, 1050 bp, synthetic construct
  source 1..1050: mol_type = other DNA
gagaccagggagtgtatctactataacgccaattgggagctggagaggacaaaccagtccggactggagcggtgtgagatggagcaggacaagagatggcattgctacgctagctggcgcaattccagcggcaccatcgagctggtgaagaagggctgttggctggacgatttcaactgttacgatagacaggagtgcgtggccaccgaggagaatcctcaggtgtatttttgctgttgcgagggcaacttctgcaatgagaggttcacccacctgccagaggctggaggaccagaggtgacctatgagccacctccaacaggaggcggcggctccggcggaggaggctctggaggaggaggctccggaggaggaggaacccatacatgtccaccttgcccagctccagagctgctgggaggcccttccgtgttcctgtttccacccaagccaaaggacaccctgatgatctctaggaccccagaggtgacatgcgtggtggtggacgtgtcccacgaggaccccgaggtgaagtttaactggtacgtggatggcgtggaggtgcataatgctaagacaaagccaagggaggagcagtacaactccacctatcgggtggtgagcgtgctgacagtgctgcaccaggattggctgaacggcaaggagtataagtgtaaggtgagcaataaggctctgcctgccccaatcgagaagaccatctctaaggctaagggccagcccagagagcctcaggtgtacacactgcctccatcccgcgacgagctgaccaagaaccaggtgagcctgacatgcctggtgaagggcttctatcccagcgacatcgccgtggagtgggagtctaatggccagcctgagaacaattacaagaccacaccccctgtgctggacagcgatggctctttctttctgtattctaagctgaccgtggataagtcccggtggcagcagggcaacgtgttttcttgttccgtgatgcatgaggccctgcacaatcattacacacagaagagcctgtctctgtcccctggc

SEQ ID NO: 365 - DNA, 1050 bp, synthetic construct
  source 1..1050: mol_type = other DNA
gagaccagggagtgtatctactataacgccaattgggagctggagaggacaaaccagtccggactggagcggtgtgaggacgagcaggacaagagataccattgctacgctagctggcgcaattccagcggcaccatcgagctggtgaagaagggctgttggctggacgatttcaactgttacgatagacaggagtgcgtggccaccgaggagaatcctcaggtgtatttttgctgttgcgagggcaacttctgcaatgagaggttcacccacctgccagaggctggaggaccagaggtgacctatgagccacctccaacaggcggcggcggctccggaggaggaggctctggaggaggaggctccggaggaggaggaacccatacatgtccaccttgcccagctccagagctgctgggaggcccttccgtgttcctgtttccacccaagccaaaggacaccctgatgatctctaggaccccagaggtgacatgcgtggtggtggacgtgtcccacgaggaccccgaggtgaagtttaactggtacgtggatggcgtggaggtgcataatgctaagacaaagccaagggaggagcagtacaactccacctatcgggtggtgagcgtgctgacagtgctgcaccaggattggctgaacggcaaggagtataagtgtaaggtgagcaataaggctctgcctgccccaatcgagaagaccatctctaaggctaagggccagcccagagagcctcaggtgtacacactgcctccatcccgcgacgagctgaccaagaaccaggtgagcctgacatgcctggtgaagggcttctatcccagcgacatcgccgtggagtgggagtctaatggccagcctgagaacaattacaagaccacaccccctgtgctggacagcgatggctctttctttctgtattctaagctgaccgtggataagtcccggtggcagcagggcaacgtgttttcttgttccgtgatgcatgaggccctgcacaatcattacacacagaagagcctgtctctgtcccctggc

SEQ ID NO: 366 - DNA, 1050 bp, synthetic construct
  source 1..1050: mol_type = other DNA
gagaccagggagtgtatctactataacgccaattgggagctggagaggacaaaccagtccggactggagcggtgtgaggaggagcaggacaagagataccattgctacgctagctggcgcaattccagcggcaccatcgagctggtgaagaagggctgttggctggacgatttcaactgttacgatagacaggagtgcgtggccaccgaggagaatcctcaggtgtatttttgctgttgcgagggcaacttctgcaatgagaggttcacccacctgccagaggctggaggaccagaggtgacctatgagccacctccaacaggaggaggcggctccggcggcggaggctctggaggaggaggctccggaggaggaggaacccatacatgtccaccttgcccagctccagagctgctgggaggcccttccgtgttcctgtttccacccaagccaaaggacaccctgatgatctctaggaccccagaggtgacatgcgtggtggtggacgtgtcccacgaggaccccgaggtgaagtttaactggtacgtggatggcgtggaggtgcataatgctaagacaaagccaagggaggagcagtacaactccacctatcgggtggtgagcgtgctgacagtgctgcaccaggattggctgaacggcaaggagtataagtgtaaggtgagcaataaggctctgcctgccccaatcgagaagaccatctctaaggctaagggccagcccagagagcctcaggtgtacacactgcctccatcccgcgacgagctgaccaagaaccaggtgagcctgacatgcctggtgaagggcttctatcccagcgacatcgccgtggagtgggagtctaatggccagcctgagaacaattacaagaccacaccccctgtgctggacagcgatggctctttctttctgtattctaagctgaccgtggataagtcccggtggcagcagggcaacgtgttttcttgttccgtgatgcatgaggccctgcacaatcattacacacagaagagcctgtctctgtcccctggc

SEQ ID NO: 367 - DNA, 1050 bp, synthetic construct
  source 1..1050: mol_type = other DNA
gagaccagggagtgtatctactataacgccaattgggagctggagaggacaaaccagtccggactggagcggtgtgagaacgagcaggacaagagataccattgctacgctagctggcgcaattccagcggcaccatcgagctggtgaagaagggctgttggctggacgatttcaactgttacgatagacaggagtgcgtggccaccgaggagaatcctcaggtgtatttttgctgttgcgagggcaacttctgcaatgagaggttcacccacctgccagaggctggaggaccagaggtgacctatgagccacctccaacaggcggcggcggctccggaggaggaggctctggaggaggaggctccggaggaggaggaacccatacatgtccaccttgcccagctccagagctgctgggaggcccttccgtgttcctgtttccacccaagccaaaggacaccctgatgatctctaggaccccagaggtgacatgcgtggtggtggacgtgtcccacgaggaccccgaggtgaagtttaactggtacgtggatggcgtggaggtgcataatgctaagacaaagccaagggaggagcagtacaactccacctatcgggtggtgagcgtgctgacagtgctgcaccaggattggctgaacggcaaggagtataagtgtaaggtgagcaataaggctctgcctgccccaatcgagaagaccatctctaaggctaagggccagcccagagagcctcaggtgtacacactgcctccatcccgcgacgagctgaccaagaaccaggtgagcctgacatgcctggtgaagggcttctatcccagcgacatcgccgtggagtgggagtctaatggccagcctgagaacaattacaagaccacaccccctgtgctggacagcgatggctctttctttctgtattctaagctgaccgtggataagtcccggtggcagcagggcaacgtgttttcttgttccgtgatgcatgaggccctgcacaatcattacacacagaagagcctgtctctgtcccctggc

SEQ ID NO: 368 - DNA, 1050 bp, synthetic construct
  source 1..1050: mol_type = other DNA
gagaccagggagtgtatctactataacgccaattgggagctggagaggacaaaccagtccggactggagcggtgtgagcaggagcaggacaagagataccattgctacgctagctggcgcaattccagcggcaccatcgagctggtgaagaagggctgttggctggacgatttcaactgttacgatagacaggagtgcgtggccaccgaggagaatcctcaggtgtatttttgctgttgcgagggcaacttctgcaatgagaggttcacccacctgccagaggctggaggaccagaggtgacctatgagccacctccaacaggaggaggcggctccggcggcggaggctctggaggaggaggctccggaggaggaggaacccatacatgtccaccttgcccagctccagagctgctgggaggcccttccgtgttcctgtttccacccaagccaaaggacaccctgatgatctctaggaccccagaggtgacatgcgtggtggtggacgtgtcccacgaggaccccgaggtgaagtttaactggtacgtggatggcgtggaggtgcataatgctaagacaaagccaagggaggagcagtacaactccacctatcgggtggtgagcgtgctgacagtgctgcaccaggattggctgaacggcaaggagtataagtgtaaggtgagcaataaggctctgcctgccccaatcgagaagaccatctctaaggctaagggccagcccagagagcctcaggtgtacacactgcctccatcccgcgacgagctgaccaagaaccaggtgagcctgacatgcctggtgaagggcttctatcccagcgacatcgccgtggagtgggagtctaatggccagcctgagaacaattacaagaccacaccccctgtgctggacagcgatggctctttctttctgtattctaagctgaccgtggataagtcccggtggcagcagggcaacgtgttttcttgttccgtgatgcatgaggccctgcacaatcattacacacagaagagcctgtctctgtcccctggc

SEQ ID NO: 369 - DNA, 1050 bp, synthetic construct
  source 1..1050: mol_type = other DNA
gagaccagggagtgtatctactataacgccaattgggaggaggagaggacaaaccagtccggactggagcggtgtgagggcgagcaggacaagagatggcattgctacgctagctggcgcaattccagcggcaccatcgagctggtgaagaagggctgttggctggacgatttcaactgttacgatagacaggagtgcgtggccaccgaggagaatcctcaggtgtatttttgctgttgcgagggcaacttctgcaatgagaggttcacccacctgccagaggctggaggaccagaggtgacctatgagccacctccaacaggcggcggcggctccggaggaggaggctctggaggaggaggctccggaggaggaggaacccatacatgtccaccttgcccagctccagagctgctgggaggcccttccgtgttcctgtttccacccaagccaaaggacaccctgatgatctctaggaccccagaggtgacatgcgtggtggtggacgtgtcccacgaggaccccgaggtgaagtttaactggtacgtggatggcgtggaggtgcataatgctaagacaaagccaagggaggagcagtacaactccacctatcgggtggtgagcgtgctgacagtgctgcaccaggattggctgaacggcaaggagtataagtgtaaggtgagcaataaggctctgcctgccccaatcgagaagaccatctctaaggctaagggccagcccagagagcctcaggtgtacacactgcctccatcccgcgacgagctgaccaagaaccaggtgagcctgacatgcctggtgaagggcttctatcccagcgacatcgccgtggagtgggagtctaatggccagcctgagaacaattacaagaccacaccccctgtgctggacagcgatggctctttctttctgtattctaagctgaccgtggataagtcccggtggcagcagggcaacgtgttttcttgttccgtgatgcatgaggccctgcacaatcattacacacagaagagcctgtctctgtcccctggc

SEQ ID NO: 370 - DNA, 1050 bp, synthetic construct
  source 1..1050: mol_type = other DNA
gagaccagggagtgtatctactataacgccaattgggaggacgagaggacaaaccagtccggactggagcggtgtgagggcgagcaggacaagagatggcattgctacgctagctggcgcaattccagcggcaccatcgagctggtgaagaagggctgttggctggacgatttcaactgttacgatagacaggagtgcgtggccaccgaggagaatcctcaggtgtatttttgctgttgcgagggcaacttctgcaatgagaggttcacccacctgccagaggctggaggaccagaggtgacctatgagccacctccaacaggcggcggcggctccggaggaggaggctctggaggaggaggctccggaggaggaggaacccatacatgtccaccttgcccagctccagagctgctgggaggcccttccgtgttcctgtttccacccaagccaaaggacaccctgatgatctctaggaccccagaggtgacatgcgtggtggtggacgtgtcccacgaggaccccgaggtgaagtttaactggtacgtggatggcgtggaggtgcataatgctaagacaaagccaagggaggagcagtacaactccacctatcgggtggtgagcgtgctgacagtgctgcaccaggattggctgaacggcaaggagtataagtgtaaggtgagcaataaggctctgcctgccccaatcgagaagaccatctctaaggctaagggccagcccagagagcctcaggtgtacacactgcctccatcccgcgacgagctgaccaagaaccaggtgagcctgacatgcctggtgaagggcttctatcccagcgacatcgccgtggagtgggagtctaatggccagcctgagaacaattacaagaccacaccccctgtgctggacagcgatggctctttctttctgtattctaagctgaccgtggataagtcccggtggcagcagggcaacgtgttttcttgttccgtgatgcatgaggccctgcacaatcattacacacagaagagcctgtctctgtcccctggc

SEQ ID NO: 371 - DNA, 1050 bp, synthetic construct
  source 1..1050: mol_type = other DNA
gagaccagggagtgtatctactataacgccaattgggagaacgagaggacaaaccagtccggactggagcggtgtgagggcgagcaggacaagagatggcattgctacgctagctggcgcaattccagcggcaccatcgagctggtgaagaagggctgttggctggacgatttcaactgttacgatagacaggagtgcgtggccaccgaggagaatcctcaggtgtatttttgctgttgcgagggcaacttctgcaatgagaggttcacccacctgccagaggctggaggaccagaggtgacctatgagccacctccaacaggcggcggcggctccggaggaggaggctctggaggaggaggctccggaggaggaggaacccatacatgtccaccttgcccagctccagagctgctgggaggcccttccgtgttcctgtttccacccaagccaaaggacaccctgatgatctctaggaccccagaggtgacatgcgtggtggtggacgtgtcccacgaggaccccgaggtgaagtttaactggtacgtggatggcgtggaggtgcataatgctaagacaaagccaagggaggagcagtacaactccacctatcgggtggtgagcgtgctgacagtgctgcaccaggattggctgaacggcaaggagtataagtgtaaggtgagcaataaggctctgcctgccccaatcgagaagaccatctctaaggctaagggccagcccagagagcctcaggtgtacacactgcctccatcccgcgacgagctgaccaagaaccaggtgagcctgacatgcctggtgaagggcttctatcccagcgacatcgccgtggagtgggagtctaatggccagcctgagaacaattacaagaccacaccccctgtgctggacagcgatggctctttctttctgtattctaagctgaccgtggataagtcccggtggcagcagggcaacgtgttttcttgttccgtgatgcatgaggccctgcacaatcattacacacagaagagcctgtctctgtcccctggc

SEQ ID NO: 372 - DNA, 1050 bp, synthetic construct
  source 1..1050: mol_type = other DNA
gagaccagggagtgtatctactataacgccaattgggagcaggagaggacaaaccagtccggactggagcggtgtgagggcgagcaggacaagagatggcattgctacgctagctggcgcaattccagcggcaccatcgagctggtgaagaagggctgttggctggacgatttcaactgttacgatagacaggagtgcgtggccaccgaggagaatcctcaggtgtatttttgctgttgcgagggcaacttctgcaatgagaggttcacccacctgccagaggctggaggaccagaggtgacctatgagccacctccaacaggcggcggcggctccggaggaggaggctctggaggaggaggctccggaggaggaggaacccatacatgtccaccttgcccagctccagagctgctgggaggcccttccgtgttcctgtttccacccaagccaaaggacaccctgatgatctctaggaccccagaggtgacatgcgtggtggtggacgtgtcccacgaggaccccgaggtgaagtttaactggtacgtggatggcgtggaggtgcataatgctaagacaaagccaagggaggagcagtacaactccacctatcgggtggtgagcgtgctgacagtgctgcaccaggattggctgaacggcaaggagtataagtgtaaggtgagcaataaggctctgcctgccccaatcgagaagaccatctctaaggctaagggccagcccagagagcctcaggtgtacacactgcctccatcccgcgacgagctgaccaagaaccaggtgagcctgacatgcctggtgaagggcttctatcccagcgacatcgccgtggagtgggagtctaatggccagcctgagaacaattacaagaccacaccccctgtgctggacagcgatggctctttctttctgtattctaagctgaccgtggataagtcccggtggcagcagggcaacgtgttttcttgttccgtgatgcatgaggccctgcacaatcattacacacagaagagcctgtctctgtcccctggc

SEQ ID NO: 373 - DNA, 1050 bp, synthetic construct
  source 1..1050: mol_type = other DNA
gagaccagggagtgtatctactataacgccaattgggagcaggagaggacaaaccagtccggactggagcggtgtgagggcgagcaggacaagagataccattgctacgctagctggcgcaattccagcggcaccatcgagctggtgaagaagggctgttggctggacgatttcaactgttacgatagacaggagtgcgtggccaccgaggagaatcctcaggtgtatttttgctgttgcgagggcaacttctgcaatgagaggttcacccacctgccagaggctggaggaccagaggtgacctatgagccacctccaacaggaggaggcggctccggcggcggaggctctggaggaggaggctccggaggaggaggaacccatacatgtccaccttgcccagctccagagctgctgggaggcccttccgtgttcctgtttccacccaagccaaaggacaccctgatgatctctaggaccccagaggtgacatgcgtggtggtggacgtgtcccacgaggaccccgaggtgaagtttaactggtacgtggatggcgtggaggtgcataatgctaagacaaagccaagggaggagcagtacaactccacctatcgggtggtgagcgtgctgacagtgctgcaccaggattggctgaacggcaaggagtataagtgtaaggtgagcaataaggctctgcctgccccaatcgagaagaccatctctaaggctaagggccagcccagagagcctcaggtgtacacactgcctccatcccgcgacgagctgaccaagaaccaggtgagcctgacatgcctggtgaagggcttctatcccagcgacatcgccgtggagtgggagtctaatggccagcctgagaacaattacaagaccacaccccctgtgctggacagcgatggctctttctttctgtattctaagctgaccgtggataagtcccggtggcagcagggcaacgtgttttcttgttccgtgatgcatgaggccctgcacaatcattacacacagaagagcctgtctctgtcccctggc

SEQ ID NO: 374 - DNA, 1050 bp, synthetic construct
  source 1..1050: mol_type = other DNA
gagaccagggagtgtatctactataacgccaattgggaggacgagaggacaaaccagtccggactggagcggtgtgagggcgagcaggacaagagataccattgctacgctagctggcgcaattccagcggcaccatcgagctggtgaagaagggctgttggctggacgatttcaactgttacgatagacaggagtgcgtggccaccgaggagaatcctcaggtgtatttttgctgttgcgagggcaacttctgcaatgagaggttcacccacctgccagaggctggaggaccagaggtgacctatgagccacctccaacaggaggaggcggctccggcggcggaggctctggaggaggaggctccggaggaggaggaacccatacatgtccaccttgcccagctccagagctgctgggaggcccttccgtgttcctgtttccacccaagccaaaggacaccctgatgatctctaggaccccagaggtgacatgcgtggtggtggacgtgtcccacgaggaccccgaggtgaagtttaactggtacgtggatggcgtggaggtgcataatgctaagacaaagccaagggaggagcagtacaactccacctatcgggtggtgagcgtgctgacagtgctgcaccaggattggctgaacggcaaggagtataagtgtaaggtgagcaataaggctctgcctgccccaatcgagaagaccatctctaaggctaagggccagcccagagagcctcaggtgtacacactgcctccatcccgcgacgagctgaccaagaaccaggtgagcctgacatgcctggtgaagggcttctatcccagcgacatcgccgtggagtgggagtctaatggccagcctgagaacaattacaagaccacaccccctgtgctggacagcgatggctctttctttctgtattctaagctgaccgtggataagtcccggtggcagcagggcaacgtgttttcttgttccgtgatgcatgaggccctgcacaatcattacacacagaagagcctgtctctgtcccctggc

SEQ ID NO: 375 - DNA, 1050 bp, synthetic construct
  source 1..1050: mol_type = other DNA
gagaccagggagtgtatctactataacgccaattgggagaacgagaggacaaaccagtccggactggagcggtgtgagggcgagcaggacaagagataccattgctacgctagctggcgcaattccagcggcaccatcgagctggtgaagaagggctgttggctggacgatttcaactgttacgatagacaggagtgcgtggccaccgaggagaatcctcaggtgtatttttgctgttgcgagggcaacttctgcaatgagaggttcacccacctgccagaggctggaggaccagaggtgacctatgagccacctccaacaggaggaggcggctccggcggcggaggctctggaggaggaggctccggaggaggaggaacccatacatgtccaccttgcccagctccagagctgctgggaggcccttccgtgttcctgtttccacccaagccaaaggacaccctgatgatctctaggaccccagaggtgacatgcgtggtggtggacgtgtcccacgaggaccccgaggtgaagtttaactggtacgtggatggcgtggaggtgcataatgctaagacaaagccaagggaggagcagtacaactccacctatcgggtggtgagcgtgctgacagtgctgcaccaggattggctgaacggcaaggagtataagtgtaaggtgagcaataaggctctgcctgccccaatcgagaagaccatctctaaggctaagggccagcccagagagcctcaggtgtacacactgcctccatcccgcgacgagctgaccaagaaccaggtgagcctgacatgcctggtgaagggcttctatcccagcgacatcgccgtggagtgggagtctaatggccagcctgagaacaattacaagaccacaccccctgtgctggacagcgatggctctttctttctgtattctaagctgaccgtggataagtcccggtggcagcagggcaacgtgttttcttgttccgtgatgcatgaggccctgcacaatcattacacacagaagagcctgtctctgtcccctggc

SEQ ID NO: 376 - protein, 464 aa, synthetic construct
MDWTWRILFLVAAATGTHAQVQLVQSGAEVKKPGASVKVSCKASGYTFTSSYINWVRQAPGQGLEWMGTINPVSGSTSYAQKFQGRVTMTRDTSISTAYMELSSLRSEDTAVYYCARGGWFDYWGQGTLVTVSSAKTTAPSVYPLAPVCGDTTGSSVTLGCLVKGYFPEPVTLTWNSGSLSSGVHTFPAVLQSDLYTLSSSVTVTSSTWPSQSITCNVAHPASSTKVDKKIEPRGPTIKPCPPCKCPAPNAAGGPSVFIFPPKIKDVLMISLSPIVTCVVVDVSEDDPDVQISWFVNNVEVHTAQTQTHREDYNSTLRVVSALPIQHQDWMSGKEFKCKVNNKDLPAPIERTISKPKGSVRAPQVYVLPPPEEEMTKKQVTLTCMVTDFMPEDIYVEWTNNGKTELNYKNTEPVLDSDGSYFMYSKLRVEKKNWVERNSYSCSVVHEGLHNHHTTKSFSRTPGK

SEQ ID NO: 377 - protein, 236 aa, synthetic construct
MVLQTQVFISLLLWISGAYGDIALTQPASVSGSPGQSITISCTGTSSDVGSYNYVNWYQQHPGKAPKLMIYGVSKRPSGVSNRFSGSKSGNTASLTISGLQAEDEADYYCGTFAGGSYYGVFGGGTKLTVLGQPKSTPTLTVFPPSSEELKENKATLVCLISNFSPSGVTVAWKANGTPITQGVDTSNPTKEGNKFMASSFLHLTSDQWRSHNSFTCQVTHEGDTVEKSLSPAECL